European Patent Application EP 4 606 910 A1, published August 27, 2025. Title: DIAGONOSTIC AND PROGNOSTIC METHODS AND COMPOSITIONS RELATING TO ULCERATIVE COLITIS. Applicant: The Royal College of Surgeons in Ireland. Application EP, filed February 21, 2024. The sequence listing filed with the application follows.

SEQUENCE LISTING (53 sequences)

SEQ ID NO: 1 - RNA, 2582 nt, Homo sapiens
  source 1..2582: mol_type = mRNA
agtagtgcagcccgtggagccgcggctttgcccgtctcctctgggtggccccagtgcgcgggctgacactcattcagccggggaaggtgaggcgagtagaggctggtgcggaacttgccgcccccagcagcgccggcgggctaagcccagggccgggcagacaaaagaggccgcccgcgtaggaaggcacggccggcggcggcggagcgcagcgatggccgggcgagggggcagcgcgctgctggctctgtgcggggcactggctgcctgcgggtggctcctgggcgccgaagcccaggagcccggggcgcccgcggcgggcatgaggcggcgccggcggctgcagcaagaggacggcatctccttcgagtaccaccgctaccccgagctgcgcgaggcgctcgtgtccgtgtggctgcagtgcaccgccatcagcaggatttacacggtggggcgcagcttcgagggccgggagctcctggtcatcgagctgtccgacaaccctggcgtccatgagcctggtgagcctgaatttaaatacattgggaatatgcatgggaatgaggctgttggacgagaactgctcattttcttggcccagtacctatgcaacgaataccagaaggggaacgagacaattgtcaacctgatccacagtacccgcattcacatcatgccttccctgaacccagatggctttgagaaggcagcgtctcagcctggtgaactcaaggactggtttgtgggtcgaagcaatgcccagggaatagatctgaaccggaactttccagacctggataggatagtgtacgtgaatgagaaagaaggtggtccaaataatcatctgttgaaaaatatgaagaaaattgtggatcaaaacacaaagcttgctcctgagaccaaggctgtcattcattggattatggatattccttttgtgctttctgccaatctccatggaggagaccttgtggccaattatccatatgatgagacgcggagtggtagtgctcacgaatacagctcctccccagatgacgccattttccaaagcttggcccgggcatactcttctttcaacccggccatgtctgaccccaatcggccaccatgtcgcaagaatgatgatgacagcagctttgtagatggaaccaccaacggtggtgcttggtacagcgtacctggagggatgcaagacttcaattaccttagcagcaactgttttgagatcaccgtggagcttagctgtgagaagttcccacctgaagagactctgaagacctactgggaggataacaaaaactccctcattagctaccttgagcagatacaccgaggagttaaaggatttgtccgagaccttcaaggtaacccaattgcgaatgccaccatctccgtggaaggaatagaccacgatgttacatccgcaaaggatggtgattactggagattgcttatacctggaaactataaacttacagcctcagctccaggctatctggcaataacaaagaaagtggcagttccttacagccctgctgctggggttgattttgaactggagtcattttctgaaaggaaagaagaggagaaggaagaattgatggaatggtggaaaatgatgtcagaaactttaaatttttaaaaaggcttctagttagctgctttaaatctatctatataatgtagtatgatgtaatgtggtcttttttttagattttgtgcagttaatacttaacattgatttattttttaatcatttaaatattaatcaactttccttaaaataaatagcctcttaggtaaaaatataagaacttgatatatttcattctcttatatagtattcattttcctacctatattacacaaaaaagtatagaaaagatttaagtaattttgccatcctaggcttaaatgcaatattcctggtattatttacaatgcagaattttttgagtaattctagctttcaaaaattagtgaagttcttttactgtaattggtgacaatgtcacataatgaatgctattgaaaaggttaacagatacagctcggagttgtgagcactctactgcaagacttaaatagttcagtataaattgtcgtttttttcttgtgctgactaactataagcatgatcttgttaatgcatttttgatgggaagaaaaggtacatgtttacaaagaggttttatgaaaagaataaaaattgacttcttgcttgtacatataggagcaatactattatattatgtagtccgttaacactacttaaaagtttagggttttctcttggttgtagagtggcccagaattgcattctgaatgaataaaggttaaaaaaaaatccccagtgcatgtatttcagttctctaagatttttggtctggcattgtggtcttatgatgaaaacatgtatcctcttaatggcggcttctcatatattcatcctgtacattttaaaatttgttaagcaactactgtgtgctaagcactgcatagcctctatgtatgttattgtggcaggcaaaaggttctgattttgggcacaacctttatataaataacacaaaaattaa

SEQ ID NO: 2 - RNA, 1295 nt, Homo sapiens
  source 1..1295: mol_type = mRNA
agactgtgcacgctcctgtccccactcacaggcccacgcagcgaggggggcccctcttctgtgtgcgtctggaaggtcgctgcccagggaggaaatgcctttaaccggcgtggggccgggcagctgcaggaggcagatcatccgggctctgtgcctcttgctacttctcctccacgccggctctgccaagaatatctggaaacgggcattgcctgcgaggctggccgagaaatcccgtgccgaggaggcgggcgcgcccggcggcccccggcagccccgagcagaccgctgcccgccgcctccgcggacgctgccccccggcgcctgccaggccgcgcgctgtcaggcggactccgagtgcccgcggcaccggcgctgctgctacaacggatgcgcctacgcctgcctagaagctgtgccgcccccgccagtcttagactggctggtgcagccgaaacctcgatggcttggtggcaatggctggctcctggatggccctgaggaggtgttacaagcagaggcgtgcagcaccacggaggatggggccgaacccctgctctgtccctcgggctatgagtgccacatcctgagcccaggtgacgtggccgaaggtatccccaaccgtgggcagtgcgtcaagcagcgccggcaagcagatgggcgaatcctacgacacaaactttacaaagaatatccagaaggtgactcaaagaatgtggcagaacctggaaggggacaacagaagcactttcagtaaagcaacggcaagcagctaggttgcaagaacattcctctactttctgctaagccttggaaacagttgggaaaagtagtttgaccctcacagttcacattcagctcagcagagcaagaccccagagatgcttagagacaggacacctggccatcaaacccagtttggcccagcctggttgggtgactttgtgggagccacttaacagctctgggtccctgttttaccatcctgggagcaaggccctgcagctccacgagacctttaccccgggaagaagccgccacccatgaaagcatttctgaagcccctttctaagacaaggctcagcatcttgatatttttgacagattcctcccaagtctggctctgggaggtatgtacccatctcaaatgttcccaagataaattcatccttcaggaaatggaaatgaacttgcttactaatgtgtgattcctagttgtagccaccggatgtgctgaggcctaaatgttagcaggtgggaggaggccacagaacaataaaaacaaccaaataaga

SEQ ID NO: 3 - RNA, 2593 nt, Homo sapiens
  source 1..2593: mol_type = mRNA
agagctggctggacccaaggaggtgaagagtcacttttcagccccaggaagggcaaagaagagagaaaatcagcctgtctgctctctccttggctcaacaaggcctctaacagtcttctgtcctctattctgcacacagcatatttgggaacgagaaacaaaagttttcccaaatgaagagaactcacttgtttattgtggggatttattttctgtcctcttgcagggcagaagaggggcttaatttccccacatatgatgggaaggaccgagtggtaagtctttccgagaagaacttcaagcaggttttaaagaaatatgacttgctttgcctctactaccatgagccggtgtcttcagataaggtcacgcaaaaacagttccaactgaaagaaatcgtgcttgagcttgtggcccaggtccttgaacataaagctataggctttgtgatggtggatgccaagaaagaagccaagcttgccaagaaactgggttttgatgaagaaggaagcctgtatattcttaagggtgatcgcacaatagagtttgatggcgagtttgcagctgatgtcttggtggagttcctcttggatctaattgaagacccagtggagatcatcagcagcaaactggaagtccaagccttcgaacgcattgaagactacatcaaactcattggctttttcaagagtgaggactcagaatactacaaggcttttgaagaagcagctgaacacttccagccttacatcaaattctttgccacctttgacaaaggggttgcaaagaaattatctttgaagatgaatgaggttgacttctatgagccatttatggatgagcccattgccatccccaacaaaccttacacagaagaggagctggtggagtttgtgaaggaacaccaaagacccactctacgtcgcctgcgcccagaagaaatgtttgaaacatgggaagatgatttgaatgggatccacattgtggcctttgcagagaagagtgatccagatggctacgaattcctggagatcctgaaacaggttgcccgggacaatactgacaaccccgatctgagcatcctgtggatcgacccggacgactttcctctgctcgttgcctactgggagaagactttcaagattgacctattcaggccacagattggggtggtgaatgtcacagatgctgacagtgtctggatggagattccagatgatgacgatcttccaactgctgaggagctggaggactggattgaggatgtgctttctggaaagataaacactgaagatgatgatgaagatgatgatgatgatgataattctgatgaagaggataatgatgacagtgatgacgatgatgatgaatagcccaactccaaacaattctgatgaaaacaaaatcacagcacccactaccatacagacagcacaaggtggcagcaagcaattctgccccacacccagccagctcctttcccttttccatcatctcttttcccactccctttgcgtcaggagcagcatcattcagcaaatgccttttcaaatgcagcaatcccacttagcagggacaggagaaaaattattcccatgttgactgtcttgactgtcacggaacagatcttgttctttgctggaccatcaagggtcatggcagtgcctgaacatggcagtctagggtgaacaatcccctaacacaagtttacttgtctttgattatgacagtaacaaaattgacagctttctaactcacaggcatagagtgaccttttaatcagagcccagggaagacacatgattaatgatttagctccctccatacctcgaacatcagttgggatccctcctccagccaagatgatccttcttagagaaggctcagccttggaagcaaacttataaatcatattctcatggctttgttaaacttatttcaagtgatggtcattcatatcactatgaacttggatattcaagcctttggatggctatggagagggcttgaaatgtgtacaggtgtcaccatcatttctagtatattaggaaactgggatgggaggttgatttgctctctaaacttccctctagttggcaagtctcacatattcatcagcaggagtggagggtgggggaaaactagaaagatgaaaacttttacatttttctgatgggttcatgtctctgattgggtcagctggcttcctagcctaagctgggatctgaataccccttctctgtagctgctagtgagccttcccatttagattaaagattgctttatccagcagtcaattaactctccagttatcagtactcccacaattggccagggcaacaataattggagttcatactgatgccctgaggcactgaaaaaaaaaaaaatcccaaagtgccttctgagctgtctaaaagttacattgtgcttggtagatttagtgttaagtgtgcagtataattttctaatttattttctcaatcttttagcacatgtgtaagacactgtgcaaattttttgaaaatagagcaatactttttgtggaatactagctaactaattctgtcattaaactcatattttgaaaata

SEQ ID NO: 4 - RNA, 3393 nt, Homo sapiens
  source 1..3393: mol_type = mRNA
aaacaatgcttctttttgacctttcccaaggagaagcgctacaaagcagccactgtgcttactgaacggcctccccctgtatcgcttaattgagaaggtatacaaatgctctcagtccagccagacaccaagccgaaaggttgtgctggctgcaaccgaaagatcaaggaccggtatcttctaaaggcactggacaaatactggcatgaagactgcctgaagtgtgcctgctgtgactgtcgcttgggagaggtgggctccaccctgtacactaaagctaatcttatcctttgtcgcagagactatctgaggctctttggtgtaacgggaaactgcgctgcctgtagtaagctcatccctgcctttgagatggtgatgcgtgccaaggacaatgtttaccacctggactgctttgcatgtcagctttgtaatcagagattttgtgttggagacaaatttttcctaaagaataacatgatcctttgccagacggactacgaggaaggtttaatgaaagaaggttatgcaccccaggttcgctgatctatcaacatcaccccattaagaatacaaagcactacattcttttatcttttttgctccacatgtacataagaattgacacaggaacctactgaatagcgtagatataggaaggcaggatggttatatggaataaaaggcggactgcatctgtatgtagtgaaattgccccagttcagagttgaatgtttattattaaagaaaaaagtaatgtacatatggctggatttttttgcttgctattcgtttttgtgtcacttggcatgagatgtttattttggactattgtatataatgtattgtaatatttgaagcacaaatgtaatacagttttattgtgttaccatttgtgttccatttgcttctttgtattgttgcatttagtacaatcagtgtttaaacttactgtatatttatgctttctgtatttaccagctattttaaatgagctgtaactttctagtaaagaattgaaaagcaaatctcactaatgatacacagatagataaagcaagtctatcaacattaaaaatactaaaaaataaagacacacacagagcattttagtgacatccactacttattgccgctatgagttagagtctatcagtgttcttgttataaccccctattttcagggggttaaaaatcagctttaaaaaaatacataaaaatttcatcttaaagcactttcattttataccaacgtgaaaagtgccatttttagaataactttaaagcttaacaggtttccttttaatatcctttttttgtgtgctctttacttacacaatggctttgttttgctttttcagccacaccccttatgtgaactagtgcctttgggtatcacgtaaaattttttccaaagggttactttaaaaatctgttaccacaattatgagatgatttttaagtgataaattaaacttcttcttgtataaattctgcccagatctctccacaagagctgagggtttcataactttatggcttaataaatgtatgacactgaaaagatttgagtgtgaatctactgaaatcactataatgcacattgaagctatgatggtatttgagtagtgaggttacttttgatcggagcaacataatgctcatagaatcttctagaagaagagaaacaaagggattgataaaatgctgagaactagtgattatatatttttctgtatttacctgacatttattttaatgttcaaaaagtaaacactttaagtttgatgtgttttactctctcattgttttaagtaattgccaactcagaatacatcattcttaggctgaaatttgtctttccattttttaaggtgaaatagtactaccttacgtgatagcatacaaagaagaaagctctagaaagagaaattatggagaatgattatttaaattacaattaaggaaatgagaatatgatcccctcttccgagttgcccacaaacttgcttctttgcttttgctccctgtaatagaactacttttcaacaaatctaattttgcacggcaccgttaaccatattttcactacagcaaacttagtgctatgggttttctttttctttgtttttttcttgatcacttgtataggaaacaatattttccagtgttatttgcatatatattttgtccttccaatatatgcattacagatgaaaattaaatgttatacctgaattcttgggttggggccaaaatattaagctgaaaataatgctggtgtggatttgttttaaaacaaagctttattatgaacatgcatgtgaatctggatattgcctcttatttttaagaaaatggttctgtgaaaagtgaatgatatgtatttttccaaatgcttcatggttaggagtcttcaagttccatgttccccagatttgagatatactaaagaaagaaattcaaaagtagctatttggggcccacaaaaataactattattttagccttagagccttacacttgtttcatgaagagaaaggacttgcataaccaaaataaacaaagcaagacaaattaaaaatatgtgggggagagatcagtgaaaagtggttttcttaatgcagccctgctggtccccattaacaattgcttgaaattcacatggatgtaaaattataattgtcaggatcttattcagatgatcttttaaggtttaactggttttgcttttgtttatctatatgtcaaaatacttgtaaattgggaacaaacttctctcagcttcttgaagttgttcaactatccttgccactggaagaccaaacaaggttttcactgctttttcttttacataatatgctgagaattatttcttatgctttttactacaaacaaaattactcacctggattaaagattaaggccttaatctgtttagattatctttaatctccatgaaatcgtgaaataagacaagaatagtgtttcagctgtaggccattttacagctaattgcccataaattgtagcatttattgacctgaagtactaagctaattgtcttgactactcaaagcccctgaattgttgtcaactttcccctttgtgttgtgtagccctaacgtcatttagcttgttgtctgatgcctccagtaggacacctccgatggagctttgatttctgagcagcgaaagctcccttcctaagatgcatctcgcataggctgcctatgatgaaggaccgtgcacctccactccaacagagtgctgagtttaaaagttgacctgtgtttgtaatttcactttcatcttgcttaataaatatctgctggattctttcattcacttttttacatttggatttatgtttttaataaaaggggtgttacacta

SEQ ID NO: 5 - RNA, 7353 nt, Homo sapiens
  source 1..7353: mol_type = mRNA
agtctgcgggcctccggggcagcggcgaggccggagcgtcgcggcggagaggacgagaccgggacaagaccagggcaggagggagccggccagccgcgagaaccccgcacgcccggcaagatgctgtcctggcggctgcagacgggccccgagaaggccgagctccaggagctcaacgcccggctctatgactacgtgtgtcgggtgcgggagctggagcgcgaaaacctactcctggaggaggagctgcgcggccggcgcgggcgagagggcctgtgggccgaggggcaggcccgctgcgccgaggaggcgcgcagcttgcggcagcagctggacgagctgagctgggccactgcgctggcggagggcgagcgggacgctctgcggcgcgagctgcgggagctgcagcgcctggatgcggaggagcgcgccgcccgcggccgcctggacgccgagctgggtgcgcagcagcgcgagctgcaggaggcgctgggcgcgcgcgccgccctcgaggcgctgctgggccggctgcaggccgagcgccgaggcctcgacgcggcccacgaacgcgacgtgagggagctgcgcgcgcgcgccgccagccttaccatgcatttccgcgcccgcgccaccggccccgccgcgccgccgccacgcctgcgggaggtgcacgacagctacgcactgctggtggccgagtcgtggcgggagacggtgcagctgtacgaggacgaggtgcgcgagctggaggaggcgctgcggcgcggccaggagagcagactccaggcggaggaagagacgcggctgtgcgcgcaggaggcagaggcgctgcggcgcgaggcgctcgggttggagcagctgcgcgcgcggctggaggacgcgctgctgcggatgcgcgaggagtacgggatacaggccgaggagcggcagagagtgattgactgcctggaggatgagaaggcaaccctcaccttggccatggctgactggctgcgggactatcaggacctcctgcaggtgaagaccggcctcagtctggaggtggcgacctaccgggccttattggaaggagaaagtaatccagagatagtgatctgggctgagcacgttgaaaacatgccgtcagaattcagaaacaaatcctatcactataccgactcactactacagagggaaaatgaaaggaatctattttcaaggcagaaagcacctttggcaagtttcaatcacagctcggcactgtattctaacctgtcagggcaccgtggatctcagacgggcacatctattggaggtgatgccagaagaggcttcttgggctcgggatattcttcctcggccactacccagcaggaaaactcatacggaaaagccgtcagcagtcaaaccaacgtcagaactttctctccaacctatggccttttaagaaatactgaggctcaagtgaaaacattccctgacagaccaaaagccggagatacaagggaggtccccgtttacataggtgaagattccacaattgcccgcgagtcgtaccgggatcgccgagacaaggtggcagcaggtgcttcggaaagcacacggtcaaatgagaggaccgtcattctgggaaagaaaacagaagtgaaagccacgagggagcaagaaagaaacagaccagaaaccatccgaacaaagccagaagagaaaatgttcgattctaaagagaaggcttccgaggagagaaacctaagatgggaagaattgacaaagttagataaggaagcgagacagagagaaagccagcagatgaaggagaaggctaaggagaaggactcaccgaaggagaagagcgtgcgagagagagaggtgccgattagtctagaagtatcccaggacagaagagcagaggtgtccccgaaaggtttgcagacgcctgtgaaggatgctggtggtgggaccggtagagaggcagaagcaagagagctacggttcaggttgggcaccagtgatgccactggttctctgcaaggcgattccatgacagaaaccgtagcagaaaacatcgttaccagtatcctgaagcagttcactcagtctccagagacagaagcatctgctgattcttttccagacacaaaagtcacttacgtggacaggaaagagcttcctggggaaaggaaaacaaagactgaaatagttgtggagtctaaactgactgaggatgttgatgtttccgatgaagctggcctggactaccttttaagcaaggatattaaggaagtggggctgaaaggcaagtcagccgagcagatgataggagacatcatcaacctcggcctgaaagggagggaggggagagcaaaggtcgtcaacgtggagatcgtggaggagcccgtgagttatgtcagcggggagaagccggaggagttttccgtcccattcaaagtggaggaggtcgaagatgtgtcgccaggcccctgggggttggttaaggaggaggaaggttatggagaaagcgatgtcacattctcagttaatcagcatcgaaggaccaagcagcctcaggagaacacgactcacgtggaagaagtgacagaggcaggtgattcagagggcgagcagagttattttgtgtccactccagatgaacaccccggggggcacgacagagatgacggctcggtgtacgggcagatccacatcgaggaggaatccaccatcaggtactcttggcaggatgaaatcgtgcaggggactcgaaggaggacacagaaggacggtgcagtgggcgagaaggttgtgaagcccttggatgtcccagcgccctctctggagggggacctgggttccactcactggaaagaacaagctagaagcggtgaatttcatgccgaacccacagtcattgaaaaagaaattaaaataccccacgaattccacacctccatgaagggcatctcctccaaggagccccggcagcagctggtggaggtcatcgggcagctggaggaaacccttcccgagcgcatgagggaggagctgtccgccctcaccagagaggggcagggtgggccggggagcgtttccgtggatgtcaagaaggtccagggtgctggtggcagttccgtgaccctggttgctgaagtcaacgtctcacaaactgtggatgccgatcggttagacctggaggagctgagcaaagatgaggccagtgagatggagaaggctgtggagtcggtggttcgggagagcctgagcaggcaacgcagcccagcgcctggcagcccagatgaggaaggtggagcggaggccccggctgctggcattcgctttaggcgttgggccacccgggagctgtacatcccttcaggcgagagcgaggttgctggtggggcctctcacagctcgggacagcgcactccccagggcccagtgtcggccactgtggaggtcagcagccccacaggctttgcccagtcacaggtgctggaggatgtgagccaggctgcaaggcacataaaactcggcccctctgaagtctggaggactgagcgaatgtcatatgaaggacccactgcagaagtggtggaggtaagtgcgggaggtgacctaagtcaggcagcgagcccgaccggagccagccggtctgtgaggcatgtcacgctgggtcccggtcaaagtccactgtccagagaagtcatcttcctaggccctgcccctgcctgtccagaggcatggggctcgccagaacctggcccagcagagtcttctgcagatatggacggatcagggaggcacagcacatttggctgcagacaatttcatgctgaaaaggagattatttttcagggccccatttctgctgcagggaaggttggtgattattttgcaacagaagagtcagtgggtacccagacttctgtcaggcaactccagttaggccctaaagaagggttcagtgggcaaatccagttcacagctccactttcagacaaggtggagttgggtgtcataggagattctgtacacatggaagggttgccagggagcagcacatccatcaggcacatcagcattgggcctcagaggcatcagaccacccagcagatagtttaccatgggctggttccccaactgggggaatctggtgactcagagagcactgtgcacggagagggctcagcagatgtgcaccaggccactcacagtcatacctcgggtagacaaaccgttatgactgaaaagagcaccttccaaagtgtcgtttctgaatctccccaggaggatagtgcagaggacacatcaggggcagaaatgacatcgggtgttagcagatcctttaggcacattcgactaggtcctacagaaacggaaacctctgaacacattgccatccgtggacccgtgtccagaacatttgtgcttgctggttcagcggactcccctgagctaggcaagttagcagacagcagcagaacgctaaggcacattgcaccagggcccaaagaaacttcgtttacctttcagatggatgtgagtaacgtagaggcgatccgcagccggacacaggaagcgggagctctcggtgtgtctgaccgtggttcctggagagacgcggacagtaggaatgaccaggcagttggtgtgagctttaaggcctctgctggggaaggagaccaggcccacagagaacagggcaaggagcaggccatgtttgataagaaggtgcagctccagagaatggtagaccaaaggtcggtgatttcagatgaaaagaaagttgccctcctctatctagacaatgaggaggaggagaatgatgggcattggttttaataagcagaaacattttgttttaatggcagcctgttggcgacgtgccaacatccaaaggccttaacttattttaagaggccgagggagtctatgaaaatctccccttttttacttttttaaagagtactcccggcatggtcaatttcctttatagttaatccgtaaaggtttccagttaattcatgccttaaaaggcactgcaattttatttttgagttgggacttttacaaaacacttttttccctggagtcttctctccacttctggagatgaatttctatgttttgcacctggtcacagacatggcttgcatctgtttgaaactacaattaattatagatgtcaaaacattaaccagattaaagtaatatatttaagagtaaattttgcttgcatgtgctaatatgaaataacagactaacattttaggggaaaaataaatacaatttagactctaaaaagtcttttcaaaaagaaatgggaaataggcagactgtttatgttaaaaaaattcttgctaaatgatttcatctttaggaaaaaattacttgccatatagagctaaattcatcttaagacttgaatgaattgctttctatgtacagaactttaaacaatatagtatttatggcgaggacagctgtagtctgttgtgatatttcacattctatttgcacaggttccctggcactggtagggtagatgattattgggaatcgcttacagtaccatttcattttttggcactaggtcattaagtagcacacagtctgaatgcccttttctggagtggccagttcctatcagactgtgcagacttgcgcttctctgcaccttatcccttagcacccaaacatttaatttcactggtgggaggtagaccttgaagacaatgaagagaatgccgatactcagactgcagctggaccggcaagctggctgtgtacaggaaaattggaagcacacagtggactgtgcctcttaaagatgcctttcccaaccctccattcatgggatgcaggtctttctgagctcaagggtgaaagatgaatacaataacaaccatgaacccacctcacggaagctttttttgcactttgaacagaagtcattgcagttggggtgttttgtccagggaaacagtttattaaatagaaggatgttttggggaaggaactggatatctctcctgcagcccagcaccgagatacccaggacgggcctggggggcgagaaaggcccccatgctcatgggccgcggagtgtggacctgtagataggcaccaccgagtttaagatactgggatgagcatgcttcattggattcattttattttacacgtcagtattgttttaaagtttctgtctgtaaagtgtagcatcatatataaaaagagtttcgctagcagcgcattttttttagttcaggctagcttctttcacataatgctgtctcagctgtatttccagtaacacagcatcatcgcactgactgtggcgcactggggaataacagtctgagctagcaccaccctcagccaggctacaacgacagcactggagggtcttccctctcagattcacctggaggccctcagacccccagggtgcacgtctccccaggtcctgggagtggctaccgcaggtagtttctggagagcacgttttcttcattgataagtggaggagaaatgcagcacagctttcaagatactattttaaaaacaccatgaatcagatagggaaagaaagttgattggaatagcaagtttaaacctttgttgtccatctgccaaatgaactagtgattgtcagactggtatggaggtgactgctttgtaaggttttgtcgtttctaatacagacagagatgtgctgattttgttttagctgtaacaggtaatggtttttggatagatgattgactggtgagaatttggtcaaggtgacagcctcctgtctgatgacaggacagactggtggtgaggagtctaagtgggctcagtttgatgtcagtgtctgggctcatgacttgtaaatggaagctgatgtgaacaggtaattaatattatgacccacttctatttactttgggaaatatcttggatcttaattatcatctgcaagtttcaagaagtattctgccaaaagtatttacaagtatggactcatgagctattgttggttgctaaatgtgaatcacgcgggagtgagtgtgcccttcacactgtgacattgtgacattgtgacaagctccatgtcctttaaaatcagtcactctgcacacaagagaaatcaacttcgtggttggatggggccggaacacaaccagtctttttgtatttattgttactgagacaaaacagtactcactgagtgtttttcagtttcctactggtggttttgatattgtttgtttaagatgtatatttagaatgacatcatctaagaagctgattttgctaaactcctgttccctacaatgggaaatgtcacaagaatgtgcaaaaataaaaatctgaggaaaaaaccca

SEQ ID NO: 6 - RNA, 1501 nt, Homo sapiens
  source 1..1501: mol_type = mRNA
acaccagccctcagtcactgggagaagaacctctcataccctcggtgctccagtccccagctcactcagccacacacaccatgtgtgaagaggagaccaccgcgctcgtgtgtgacaatggctctggcctgtgcaaggcaggcttcgcaggagatgatgccccccgggctgtcttcccctccattgtgggccgccctcgccaccagggtgtgatggtgggaatgggccagaaagacagctatgtgggggatgaggctcagagcaagcgagggatcctaactctcaaataccccattgaacacggcatcatcaccaactgggatgacatggagaagatctggcaccactccttctacaatgagctgcgtgtagcacctgaagagcaccccaccctgctcacagaggctcccctaaatcccaaggccaacagggaaaagatgacccagatcatgtttgaaaccttcaatgtccctgccatgtacgtcgccattcaagctgtgctctccctctatgcctctggccgcacgacaggcatcgtcctggattcaggtgatggcgtcacccacaatgtccccatctatgaaggctatgccctgccccatgccatcatgcgcctggacttggctggccgtgacctcacggactacctcatgaagatcctcacagagagaggctattcctttgtgaccacagctgagagagaaattgtgcgagacatcaaggagaagctgtgctatgtggccctggattttgagaatgagatggccacagcagcttcctcttcctccctggagaagagctatgagctgccagatgggcaggttatcaccattggcaatgagcgcttccgctgccctgagaccctcttccagccttcctttattggcatggagtccgctggaattcatgagacaacctacaattccatcatgaagtgtgacattgacatccgtaaggacttatatgccaacaatgtcctctctgggggcaccaccatgtaccctggcattgctgacaggatgcagaaggagatcacagccctggcccccagcaccatgaagatcaagattattgctcccccagagcggaagtactcagtctggatcgggggctctatcctggcctctctctccaccttccagcagatgtggatcagcaagcctgagtatgatgaggcagggccctccattgtccacaggaagtgcttctaaagtcagaacaggttctccaaggatcccctcgagactactctgttaccagtcatgaaacattaaaacctacaagccttacttctctgtgtggggctcttttttcctgggctatgtctcatacacagtgctaaggacttttcacacattacttttaatccatgcaatagtgctgtaaggtaggtgctatcattatacccatattacagatgaggaaattgaggctcagagaagtcaaggacttgcgaagatcacacagattccagattaaaattcaagtatctgactgcaaa

SEQ ID NO: 7 - RNA, 12883 nt, Homo sapiens
  source 1..12883: mol_type = mRNA
ctcctcccgcgcccgctctgctctaggatgctgcggcaggttctgcacaggggcttgaggacgtgtttctcccggctcggccacttcattgccagtcaccctgtcttcttcgcctcggcgccggtgctcatctccatcctgctcggcgccagcttcagccgctaccaggtcgaggagagcgtggagcacctgctggcgccccagcacagcctggccaagatcgagcgcaacctcgttaacagcctcttcccggtcaaccgctccaagcaccgtctctactcggacctgcagacccccgggcgctacggccgggtcatcgtcacctccttccagaaagccaacatgctggaccagcatcacaccgacctgatcttaaagttgcatgctgctgtcaccaagatccaggttccaaggcctggttttaattacacgtttgcccatatatgtatcctgaataatgataagacttgcatcgtggatgacatagtgcacgtcctggaagagctaaagaatgctcgggccaccaatcggaccaattttgctatcacatacccaatcactcacttaaaggacgggagggctgtgtacaatgggcaccagcttgggggcgtcactgtgcacagcaaagaccgggtgaaatctgcagaggccatccagctcacctactacctgcagtcaatcaacagtctcaatgacatggtggctgagaggtgggagtccagcttctgcgacactgtcagactgtttcagaaatccaacagcaaagtcaaaatgtacccttacacgtcctcctcactgagggaagatttccagaagaccagccgcgtatcagaacgttacctggtcaccagcctgattctggtggttaccatggccatcctgtgttgctctatgcaggactgcgtccgcagcaaaccctggctaggcctgctcggattggtgaccataagcctggccactctcactgcagccgggatcatcaatcttactggtgggaaatataattccaccttcctgggagtccctttcgtcatgctaggtcatggattatatgggacttttgaaatgttatcctcctggaggaaaactagagaagaccaacatgttaaagagagaactgcagcagtctatgcagactccatgctctccttttctctcaccactgccatgtacctggtcacctttggcataggggccagccctttcacgaacattgaggcagccaggattttctgctgcaattcctgtattgcaatcttcttcaactacctctatgtactctcgttttatggttccagcctagtgttcactggctacatagaaaacaattaccagcatagtatcttctgtagaaaagtcccaaagcctgaggcattgcaggagaagccggcatggtacaggtttctcctgacggccagattcagtgaggacacagctgaaggcgaggaagcgaacacttacgagagtcacctattggtatgtttcctcaaacgctattactgtgactggataaccaacacctatgtcaagccttttgtagttctcttttaccttatttatatttcctttgccttaatgggctatctgcaggtcagtgaagggtcagaccttagtaacattgtagcaaccgcgacacaaaccattgagtacactactgcccagcaaaagtacttcagcaactacagtcctgtgattgggttttacatatatgagtctatagaatactggaacactagtgtccaagaagatgttctagaatacaccaaggggtttgtgcggatatcctggtttgagagctatttaaattaccttcggaaactcaatgtatccactggcttgcctaagaaaaatttcacagacatgttgaggaattcctttctgaaagcccctcaattttcacattttcaagaggacatcatcttctctaaaaaatacaatgatgaggtcgatgtagtggcctccagaatgtttttggtggccaagaccatggaaacaaacagagaagaactctatgatctcttggaaaccctgaggagactttctgtcacctccaaggtgaagttcatcgtcttcaatccgtcctttgtatacatggatcgatatgcctcctctctgggagcccccctgcacaactcctgcatcagtgctttgttcctgctcttcttctcggcattcctggtggcagattcactgattaacgtctggatcactctcacagttgtgtccgtggagtttggagtgataggtttcatgacattatggaaagtagaactggactgcatttctgtgctatgcttaatttatggaattaattacacaattgacaattgtgctccaatgttatccacatttgttctgggcaaggatttcacaagaactaaatgggtaaaaaatgccctggaagtgcatggggtagctattttacagagttacctctgctatattgttggtctgattcctcttgcagctgtgccttcaaatctgacctgtacactgttcaggtgcttgtttttaatagcatttgtcaccttctttcactgctttgccattttacctgtgatactgactttcctgccaccctctaagaaaaaaaggaaagagaagaaaaatcctgagaaccgggaggaaattgagtgtgtagaaatggtagatatcgatagtacccgtgtggttgaccaaattacaacagtgtgataatgtctgcttggcatattttcaccttaggtcttatcaagaccaaagagattatgttaatgaaacaattaaattcaaagttcttcccttttttaaagataggaaacaggcattgccaaaaaaaaaaaaaaaaaaaaaaggaaaggacagtggggagaaatgggcctggcatattttcagtctttaaaacaaaggagttgttatgagaattcacacacacatagacacacacacacacacacacacacacacacacacacacacaccctgggagacctatagtctcttaaactaagatcaagtagaagaaagcttattaacaagcaggatcctgccttatccaaactgcagatgttgctggcattgtgacaaaacccactgattgaaaggtcaactgccaaggcagaaacacctttaagcattgttcaaacaataaggcttccagaacttctgtagagcagtagctccagtcatggtctgtggtttgaggttttagctgtctcacctagctccctaacactgaaggagatacttgtgaaagttctgaccagcaaaagcaagccagagccttggaaactgatatgtggtagagtggccatcactcatggactaaaattgattcaccgctaaatttacccaggtgaagcagtttcgttgtctagaatgaaattatcatattccgccattggtatgcctttaacatttgtatagtttggtttgcttaaaacaccttaaaaccaatgacagctccagcactgcagaattggtgtgattctactttggaatagcttgtcacttgtcaccaaatgggtctgctttattagttacagctcttggcaggaggatccagggacccaaaaccacagggccaaacccaaatacctggcatgatggagcaaaagcaggtgtctacttggacccagatatagtgtctccattttaacaacaacaacaaaatagccagctggtacagctgtttgcattggccctacatgcattttttgcatggatatccagaaacatctgcccacacaaaactgcggggaaaaaaaatgaacactgaaatagttatttgctgttgcttccaacttgtagtgccagtctgcctttgctgtgaaacacacctgctcagagacagagaggggaagaagatctttggtaagtctaagtcctgacgctgagaagctttgtaaaagtgcagggagataaagggccaaaagggagatagatggaaaacactggaaaaagtattcactgatacaaatctatcaatgatggcagtccaattctcttgctaaagtggctgcacctcaccttgctggtcccccccacaccttttttgatgtccttctgcgtcatcatagcaaggcccttctgtaaattaacaagcctagatatttatactcttgacttccagtatctacagaagaatggttcatagatctaaacagaaatggtttagatctaaaaaggctgtatacgttgcccaggcccctgcatttctttaaatttataaaaatgaagctaaaacctggttacatttgaagcaaatatctacagtatttttcccttttagagatgtagcttccttagacatctgtagtggtaagcatttcccaaaagcatcttacctttctgaaccttagcagacatactgtgcagcttacctatcttctgcagaggaggaaactgagacctaggagaataaagtgactcactcaggtcacaccactaaagggttttcatcatttcagcatacctaagacagggcagtccaattttcagtattctcataagatggctattactcctctcaaaatgcatttccaaagtaggaacataggacttcgttggccacagggcagacatttttttagtgtctggaattaaaatgtttgaggtttaggtttgccattgtctttccaaaaggccaaataattcagatgtaaccacaccaagtgcaaacctgtgctttctatttcacgtactgttgtccatacagttctaaatacatgtgcaggggattgtagctaatgcattacacagtcgttcagtcttctctgcagacacactaagtgatcataccaacgtgttatacactcaactagaagataataagctttaatctgagggcaagtacagtcctgacaaaagggcaagtttgcataatagatcttcgatcaattctctctccaaggggcccgcaactaggctattattcataaaacacaactgaagaggggattggttttactgttaaatcatgtgttgctaaatcattttctgaacagtgtgttctaaatcagtcattgatttagtgtcagccacgtggagcacctcggcttaaagcagctccacaaaacctgacacaacacacacaccaattaaatggattttgttgagaatttaatcattcaatttggtcaaccagaatgacttcctgtggaactctgttttatgacagataatagttttccaacttgattgagtctctgtataccctgggatattgtattttttaatgaagggcattttcaaacttgtcaacttctcttttcagcacttgaaatgaaggcttatggaattctgactgtgaaatgaatttttctattgggagattatgcatgccaagatttattatttattgttagataattattatttatttgttaatactgattattgattattgctctgctgcattggtttagccccgctatggagaagacactttagaagtaactcagaatcacatccccataaaatctaagtctttacttcatcaagttttactttttgaattgctataaagacggaaaaattgatccctgcaaacacttgaagaagctgtgttttttttctttcaattaattccaaccaagacattaacgtccactttaccaaagaaacttacttggttggtttttagttggtgtttgttgtttgtttaccaaagaaaatattcgattcatcaaaaatattgctcctggtcaactaaaaaactgtgatactgggacttttttggccattcataaggaaaatttttaaaagtcaaggtaagggtgatattctctcatttagtggaagaagaagatgtcaattcacagggaatgtggtgttcgcaagaaagaaaatgatacttgaaatagggcattattgtttagcctacagcaacatttcaacaagcagcatcagggctcctcaggttaaaagaagtacagtttgtttcagagaaaaaggaagacaaaccctcgtgaaatgtttctccattgttccagctcataagttttactttgttttgggttttggagtttttagtttctttgatgtttgttttgctttaatttggtttgtggtttgtgtttgcttgtgtttgcttctgcctttcctaccttctgccttttactccctcagttttcagtcagaagtgtgataatcagatgccatcctccatggccacgcttatgtatgcaatataccgctccaaatgaggaccttggtaacccttgaccctttaattctaactaaccatcacccaatcgtaagtggcattatgggaccatgataccacttttctccagtgtcaatgacagagctcagctgtgtccatcacaagaaaaggtggaatgggcagctgtcttgggggtgtggcaagaggcagaacctcttggacacaaatgttatcttcctcataatggctttattcttttggatcctattaaagtacccctgtagcttatagtagtgtttgacctctgtgactctgttttctcatctgtaaaatggggataatatcagtaaatgtctttaaattcagcaaatacttatcgagtgccaaatatcgcccagatactgttcgagaggctggggacacaacagtcaacaaatcagattttttaaaatctgctcttgtagagtctacctttgagtgacattgcaggtatattgtggggattgaatgagatgagagatgacatttggaaagcactcttggaaaggcctggcaaagaaaagagactcaagacattatttgtaattcagcaatctcgcacagtagcattagggctcgggatgtaaagctactgagaagtagatttgagcctgagaattagggctacaaatacaatgagttgccacagaaggtagttaattaccagtcattttaggacatcaaaatgaagctgatcaccacatagtggggccactgtaaaggggctgcaagtcctggatgttggcatcatactatgatctttgaaaaaaacagatacaggcacttgcttttggggatggggaagggacaccactgattactgaataactgtggctggcttgtctgagggaatgtaaacattcccttgaggtaatttgcttttaattttgtgtaaaaagcaccaggtatttagagacataaagttcccgttttttaaaagaatagtaaatctgcaatacaaagaaaaatattaagttagtggattcgctggcaaagaactaagaatggctgcagccaacacactgcagagttcctccctgtggtggttacaactgttatttctgtttcatgccagtccaggagaaagcaaagaggaaagtggatgagctataatccgttcacctgaataggcagtgccaggatgtcccccccagcttgcctctcacccgccccgctgctgcccagctgatttgtttgaagtcctctttgatatctatgagagcaccgtggaaggaagaagaagggaggcgaccggagagctatggcctctgtgcagatttttgagttagattaaaattagtaccacctgattaggagcctacctggtgaggaaaaaagccttcttttcaaagtacaaaaaaaagcgatgtgtaccaaggagaaaaccagcagagaaagcttggtggaagaagtgatgttcttgtggaatgtgccagcagcttctccttccagaatgctgacaccagatgaatctttggttagaattaagcctacccctttgtttttcacatgagaaaactgaaccctcgagtaatgaaattatattcacagagctaattagaaacaggagactataattgaaatctagtttttagcctcaattctttctccattttgccactttactgccaaattctattcatctaaattattggggtcttaacctgggggccaaatgagttcatgggaggggtctctgagtttcctacaattaagttacatgcaaaaatgtgtgtatatgttcaacatgtgcattttcctaaactgagggctcagattccaaaagaggtctatgaccgaaaaagggtgaagaaccactgtcctaaattaatacagacctcattgggagtgtgatcctggtgtcctcattttggctaatgagcaatcaagaacttttgaactatcttttctctaaggatccaaaaatgcttcaaaatattggtttcttcatcccaagccaagtgcctacttctattcatttattcttcattcattctttcattcattcatttctttattctgcaaatgtattttcagtgccaattcatgttctagcagcagctaaatatgccctccacagcaggaccaggaaaggagccctctgtactgtgctcttgttggcaagaggaacaccaggttgctaccacattctcactgttgcaacaaattatatatagcctcaaattttcagtaaccatcccacacacacatacacacataaaggcagcagccaacaaagccaacatatagaagtgtgccctgtcaaagaaccaggaagagcagcctatttccaggttatatacagtgatatgctgtttacaactgcataccacatccttagaaggcctgctcccaaatgagccctactctgagatgtctacaccaggcatgctttcacacacgtgcagtaccctactctcaaaacaagtatggagagaataagtctcattcatctcgttaatatttttagtgggcaaagaagcaaccgtggccatggacagatgggtgcatttaaggacaggtgtggccgggcacagtggctcaagcctgtaatcccagcactttgggaggcggaggcgggcagatcacgaggttaagagattgagaccatcctggccagcatggtgaaaccccgcctctactaaaaaatacaaaaaaattagctgggcgtggtggcacgtgcctgtagtcccagctactcaggaggcaggagaatcccttgaacccgggaggtagaagttgcagtgagccgagatttcaccactgccctccagactggcaacagagtgagacttcgtctcaaaaaaataaaggacaagtgtgttttatacacaaatatgcagaagcccagttctcttgactccaagtcagaagctagataaaatagaggttgctgggggaagttggaaaataaatgactatactgtacttgttggctctgctgctgctgatataacttcaggcacaacggaagccgcctcggttggcctatgggaagggctgggtgaatcactgcttggccttgcatgaagcacaaaggacacaccaatggctgatcagtggcccttccatcatcttctgcccagccatgataaggaaagccttctattgagatggaggaatattagctcaactttgtagcatctgatgtaaagtttgaggggtttgtcttttttgtttgtttgtttgtttttttttgagatggagtctcactctgtcacccaggctggagtgcagtggcgccatctcagctcactgcaagctccacctcccaggttcacgacattctcctgcctcagcctcctgagtagctgggactacaggtgcccgccaccgcgcccggctaattgtgtgtgtgtgtgtgtgtgtgtgtgtgtgtgtgtttagtagagatggggtttcaccgtgttacccatgatagtctcgatctcctaacctcgtgatccacccgcctcggcctcccaaagtgctgggattacaggcgtgagccaccgtgcccggcaagggctttgttcattaggatcaacaaagtgctttgtctaattcctgcaaaatggcaaagacccagcccatttccattactcattccaggctcatgctcaggaaaactaataacgttctctttgacaaaacaatttccttaattttctaggatgaatcttgaacatgtttagctcagcctttcagatatttattctttaaattaccatcctgtcaaaattgcctttacgcactgatccagaatcaccaaggcagttgccacgatgcctcccaggactgtgggtgactgggcaaactggtaatgacccgttggctctgcttcacacacacacatacacattgacacacataaatgtacacatgcatatatgtgtgtacaacacaactataaaacatagaaacatatacctgtacatatgcacatgcttacatacacacatatcacagatgtgcatgcacacatacacatgcacaccaccttttacaatatgcctgacacatttgaggcacattaaaatgccttggcaggcccagccctatagttctgtaaggtttggcaggccaaaggcttcggatgtctgcaggataccattgaaaaaatgttatcttccccttctatatgtttcttatgcacgagcacagctaagagcagccaaatagtaagctttaaagaaaagaaacctggaaaagtgaatgtgccttgcaatttaaaaattgctaacagtttcacagtgggaaaattgcatttgttggaattttccaagtcataagcaagaagaatagcatagacccaaaacgacagagatctcttccaaggtatggaattgtggaaatttatttagaatatttgcttggtgatccagagaagggggaaagaagtggtgaggaagaatatatggggtgatccctccaaattgccaactcctcgtcttaggaagaagtgggcagtttccattgatccctagcatcagtttgacgggaaaaccggtgcatttcatcaacctcaaggaaaggaagtgccatgcatggaggcctggtgataggcaacatccatttagaagaacagtcacacaagcaacagaagaactatccaagactagaagcttagaagcttataccaaactctctgtctctctctctctctctcacacacacacacacagagtggatgggaggggacattaagaggaaccctagtgcagttcccccaaaaaaccttggcatagagtataacagggaaaaagtaattactgggaagctgaaaacaatcaaatatgtgaggaatgactgaatatgagctgaggataatgtaaattgttctggattgtctataagataaagatacagagcctgaatctatgtttttctgaataaagagaccccatattctcttttgaattattgacctataattcctcttcagcagctttgaatacactcaagttctcttcctattgtttatgatcccataatacaaccacccactatttgttgtggtttacaatccagcttagaacccttgagcaaaattattgaattattgaatgctaggcccaaacaaaagaaatttcagcttggttttagtaatttcttgatcaaacttctctcattcctctaaatgtacaaaggtttcaaagttgtaaaaaatatgtctacatagccaatgctcttagtatttttaacagcaaagataatctctgccaataattattaatgacaaaatagtgataactgttcaatgttgctttaacagtccaattgtagtaggtgagaaaacaaaaaagaagagaagctatgttgaatatttagtaatgttggaaaagatcctcaccctagacataaaatagtttaaacatttaaacatggcccctctcttattgtcattgctagtgaaagaagttcctgaaattgcatattacattgtaaagttttgggctaaatcacaatacatttttaagttgcttccatggcaatagatcgtaagaccacagcttgtcaaagtaaccactaattcagtattcagaaaccttatcatctgttcctccaaaaagaccccatagttaatgttgtgtttcccagtattttagttgggtttcttcacacttaggcaagtgggtgattctggtcataataaactattttcaaactaggaaaaagtatccaaatgctagagcacataatgagttcagcttggtcagttttgagacagataagcataaaaccctactagaaaaaaataatagtcaaacctaaagctttaaaaaatgtgagtcacatcacttttctccaggaaaggcagaacgtgctcagggtggaatttaatcaaaaatgtacccagaacaatttcccacaaagagctgtaatactttgcagcaaggggcattaataaactctaatttttaccgaaagtcaagagacacacagatcttttttggtaccctctacatcatcatagcaaggcccttctgaacattaacaagcctagatgtttctactgcttatttgcagtatctacaggggaatggttcgtggatataaacagaaatgttttatctgaagaggctgtgtatgccaccccagacccctgcatttcttaatatctataaaaatatgactaaacttgttacatttgaggcaaatatgtacagtatttttcccttttaaagatagtttaaaaaatcaaggtaataaaaaacggccaactctttcaggaaaaaaaaaatccggtattttgtactacttgagtttctctaatgcctaaaatatgcatttaaatcatcccacacctacacagaaacaaaatcagcagggaaaaccatcccactgatgattggcaattccaccgttcctctccatctgaccagctttcaccagagggcgatctttcatgcttgcacatcgagtttatacaatgtagaagcccccaagtcacctgggaaatggctcatgccaaatacatggagtccttagttgactatcttttcatattaaaatcccatcttccaatgaagcatcctgttttcaatactgatatcaaatttcgaatgtaaaggagatttcaaatgtattgctttcaccttttcttttttattcatttatttttaattgacataaaaattgtatatatttatgggatacaatgtgatgttttgatatatgtatgcattgtggaatgattaaatcaagctaattaacata

SEQ ID NO: 8 - RNA, 2144 nt, Homo sapiens
  source 1..2144: mol_type = mRNA
acgctcgcccagaggcctgcgcccacaccctctcctgtccagccctcgcccgcctgggcagggcccggcgccgtccgtggatgagccacagaacctcttccaccttccgagcggagagaagtttccattcctcttcctcttcctcctcctcttccacctcctcctcggcctcccgtgctctcccggcccaggacccgcccatggagaaggccctgagcatgttttccgatgactttggcagcttcatgcggccccactcggagcccctggccttcccagcccgccccggtggggcaggcaacatcaagaccctaggagacgcctatgagtttgcggtggacgtgagagacttctcacctgaagacatcattgtcaccacctccaacaaccacatcgaggtgcgggctgagaagctggcggctgacggcactgtcatgaacaccttcgctcacaagtgccagctgccggaggacgtggacccgacgtcggtgacctcggctctgcgggaggacggcagcctcactatccgggcacggcgtcacccgcatacagaacacgtccagcagaccttccggacggagatcaaaatctgagtgcctctcccttccctttccctgtccccccgccccacgcctgccagcaaagcctcgctaaccccattacaacagctccaggacatctcagcccaggttctagcccccacgcaccccagaccccaggtggaccatcctcccaaactagggccctccactctatccagggcaggccagggactccctggcctgacacatgatgcccagatttcagatttggcctccgtcacttaatccagagtacaggggctggggtcagggaaggaagatctaaagaacccactgtgggtcaggggaatgggaccagcaggacatatgggcaagctctgcaggacagacagacagacaaaccctctgatctatgaagtctctgcagggcaaggggaccagggacctggaaccctcttggccaaggggagtgggagggacagagggaaggtcacaggcaagggtgcctatctaagtggaactaattgcccgagggctcagcaaggccaagaggagacagccgtgacggtaaacttcccctctaccagcctccaagccccacgccagcgagcaggctgcctgcccaccccgtgcccccagccagctggctgtgccagggcagagccatgccacatctgtatatagatggggtttttccaatacagctggttcgtgataaactgcatgaaactcctgccgtcctgcgcctgctggggcctccaggcaaggccaagtggggttgggggtggggctggtccttctccctcccacaggcctgtgttcttggggctgctcccatgcagacaggatcacctaacagagatggaagccagggcatggatggggctttgggtcctcgaggttggaccccagcttcttgccaccttcccctccgggcagtcagctctccatccatccccctctttaatctatgaatctataggctcggtgtgtgtaacacacacacccctatcgttgtccttcaaatactcagcattaccattggttgaggccaaattcagagctttctcaaatcagatttacaatctccattttcattaacggggaaacatccccgagccactgagtgctgtgctttgtcactgaaggttagatctgaacccagggtgtcaactgctgctctcaactccccacctctgggcactgaggagtatttcccctcattctacctctctaaggctatgcaaccctccccacgtcttccagctgggggatgggggggagtcataggaaaagcccccatctcccatctgggatagggaccttccatcagccttaaccctgggaaatgcctgctgcccccaatgactcttggtttcgtctcccacatacagaagcagggtggaggggaagggtgggtctcagttagcaggggtccccagggcaagtcagcctcctccctccatgcctctctggtcagtgtgccttagggtggcctctcactcccaccactctgggccccttgggggaggactggggagggggccgtgggagagccctgacgctggaacctgtatacacaataaaggacagtctcacaga

SEQ ID NO: 9 - RNA, 9159 nt, Homo sapiens
  source 1..9159: mol_type = mRNA
gcccttcccgagcaccgctccggccctggagggagagagagccagagagcggccgagcgcctaggaggcccgccgagcctcgccgagccccgccagccccggcgcgagagaagttggagaggagagcagcgcagcgcagcgagtcccgtggtcgcgccccaacagcgcccgacagcccccgatagcccaaaccgcggccctagccccggccgcacccccagcccgcgccagcatgatgaacaacagcggctactcagacgccggcctcggcctgggcgatgagacagacgagatgccgtccacggagaaggacctggcggaggacgcgccgtggaagaagatccagcagaacacattcacgcgctggtgcaatgagcacctcaagtgcgtgggcaagcgcctgaccgacctgcagcgcgacctcagcgacgggctccggctcatcgcgctgctcgaggtgctcagccagaagcgcatgtaccgcaagttccatccgcgccccaacttccgccaaatgaagctggagaacgtgtccgtggccctcgagttcctcgagcgcgagcacatcaagctcgtgtccatagacagcaaggccatcgtggatgggaacctgaagctgatcctgggcctgatctggacgctgatcctgcactactccatctccatgcccatgtgggaggatgaagatgatgaggatgcccgcaaacagacgcccaagcagcggctgcttggctggatccagaacaaggtgccccagctgcccatcaccaacttcaaccgtgactggcaggacggcaaagctctgggcgccctggtggacaactgcgcccccggtctctgccccgactgggaggcctgggaccccaaccagcccgtggagaacgcccgggaggccatgcagcaggccgacgactggcttggggtgccccaggtcattgcccctgaggagattgtggaccccaacgtggatgagcattctgttatgacctacctgtcccagttccccaaggccaagctcaaacctggtgcccctgttcgatccaagcagctgaaccccaagaaagccatcgcctatgggcctggcatcgagccacagggcaacaccgtgctgcagcctgcccacttcaccgtgcagacggtggacgcgggcgtgggcgaggtgctggtctacatcgaggaccctgaaggccacaccgaggaggctaaggtggttcccaacaatgacaaggatcgcacctatgctgtctcctatgtgcccaaggtcgctgggttacacaaggtgaccgtgctctttgctggccagaacattgaacgcagtccctttgaggtgaacgtgggcatggccctgggagatgccaacaaggtgtcagcccgtggccctggcctggaacctgtgggcaatgtggccaacaaacccacctactttgacatctacactgcgggggccggcactggcgatgttgctgtggtgatcgtggacccacagggccggcgggacacagtggaggtggccctggaggacaagggtgacagcacgttccgctgcacatacagacctgccatggaggggccacataccgtgcatgtggcctttgcgggtgcccccatcacccgcagtcccttccctgtccatgtgtcggaagcctgtaaccccaacgcctgccgcgcctctgggcgaggcctgcagcccaagggtgttcgcgtgaaagaggtggctgacttcaaggtgtttaccaagggtgccggcagcggggagctcaaggtcacggtcaaggggccaaagggcacagaggagccagtgaaggtgcgggaggctggggatggtgtgttcgagtgcgagtactacccggtggtgcctgggaagtatgtggtgaccatcacgtggggcggctacgccatccctcgcagcccctttgaggtacaggtgagcccagaggcaggagtgcaaaaggtccgggcctggggtcctggtttggagactggccaggtgggcaagtcagccgattttgtggtggaagccattggcaccgaggtggggacactgggcttctccatcgaggggccctcacaagccaagatcgaatgtgacgacaagggggatggctcctgcgatgtgcggtactggcccacggagcctggggagtacgctgtgcacgtcatctgtgacgatgaggacatccgagactcacccttcattgcccacatcctgcccgccccacctgactgcttcccagataaggtgaaggcctttgggcctggcctggagcctaccggctgcatcgtggacaagcccgctgagttcaccattgatgctcgtgcagctggcaagggagacctgaagctctatgcccaggacgccgacggctgtcccatcgacatcaaggtgatccccaacggcgacggcaccttccgctgctcctacgtgcccaccaagcccattaagcacaccatcatcatctcctggggaggcgtaaacgtgcccaagagccccttccgggtgaacgtgggcgagggcagccaccccgagcgggtaaaggtgtacggccccggagtggagaagacaggcctcaaggccaatgagcccacctacttcacggtggactgcagcgaggcggggcaaggcgacgtgagcatcggcatcaagtgcgccccaggcgtggtgggccctgcagaggctgacattgacttcgacatcatcaagaatgacaacgacaccttcaccgtcaagtacacgccaccaggggcgggccgctacaccatcatggtgctgtttgccaaccaggagatccccgccagccccttccacatcaaggtggacccatcccacgatgccagcaaagtcaaggccgagggccctgggctgaatcgcacaggtgtggaagtcgggaagcccacccacttcacggtgctgaccaagggagccggcaaggccaagctggatgtgcagtttgcagggacagccaagggcgaggttgtgcgggactttgagatcatagacaaccatgactactcctacactgtcaagtacaccgctgtccagcagggcaacatggcagtgacagtgacttatggcggggaccctgtccccaagagcccctttgtggtgaatgtggcacccccgctggacctcagcaaaatcaaagttcagggccttaatagcaaggtggctgtgggacaggaacaagcattctctgtgaacacacgaggggctggcggtcagggccaactggatgtgcggatgacttcgccctctcgccggcccatcccctgcaagctggagccaggcggtggagcggaagcccaggctgtgcgctacatgcccccggaggaggggccctacaaggtggatatcacctacgatggtcacccggtgcctggcagcccgtttgctgtggagggtgtcctgccccctgatccctccaaggtctgtgcttatggcccgggtctcaagggtggactggtaggcacccccgcgccattctccatcgacaccaagggggctggcacaggtggcctggggctgaccgtagagggcccctgcgaggccaagatcgagtgccaggacaatggtgatggctcatgtgctgtcagctacctgcccacggagcctggcgagtacaccatcaacatcctgtttgctgaggcccacatccctggctcgcccttcaaagccaccattcggcctgtgtttgacccgagcaaggtgcgggccagtggaccgggcctggagcgcggcaaggtcggtgaggcagccaccttcactgtggactgctcagaggcaggcgaggcggagctgaccattgagatcctgtcggatgccggggtcaaggccgaggtgctgatccacaacaacgcggatggcacctaccacatcacctacagccctgccttccctggcacctacaccattaccatcaagtatggcgggcatcccgtgcccaaattccccacccgtgtccatgtgcagcctgcggtcgataccagtggcgtcaaggtctcagggcctggtgttgagccacacggtgtcctgcgggaggtgaccactgagttcactgtggatgcaagatccctaacagccacaggcggcaaccacgtgacggctcgtgtgctcaacccctcgggggccaagacagacacctatgtgacagacaatggggacggcacctaccgagtgcagtacaccgcctacgaggagggcgtgcatctggtggaggtcctgtatgatgaggtcgctgtgcccaagagccccttccgagtgggcgtgaccgagggctgtgatcccacccgcgtccgagccttcgggccaggcctggagggtggcttggtcaacaaggccaaccgattcactgtggagaccaggggagcgggcaccgggggccttggcctagccatcgagggtccctcggaagccaagatgtcctgcaaggacaacaaggatggtagctgcaccgtggagtacatccccttcactcctggagactatgacgtcaacatcaccttcggggggcggcccatcccagggagcccgttccgcgtgccagtgaaggatgtggtggaccctgggaaggtgaagtgctcagggccagggctgggggctggtgtcagggcccgggttcctcagaccttcacagtggattgcagtcaagctggccgggcgcccctgcaggtggctgtgctgggccccacaggtgtggccgagcctgtggaggtgcgggacaatggagatggcacccacactgtccactacaccccagccactgacgggccctacacggtagccgtcaagtatgctgaccaggaggtgccacgcagccccttcaagatcaaggtcctcccagctcatgatgccagcaaggtgcgggccagcggcccaggcctcaacgcctctggcatccctgccagcctgcctgtggagttcaccatcgacgcacgggacgcgggcgaggggttgctcactgtccagatcttggaccccgagggtaagcccaagaaggccaacatccgggacaatggggatggcacgtacactgtgtcctacctgccggacatgagtggccggtacaccatcaccatcaagtatggcggtgatgagatcccctactcgcccttccgcatccatgctctgcccactggggatgccagcaagtgcctcgtcacagtgtccattggaggccatggcctgggtgcctgcctgggccctcgaatccagattgggcaggagacggtgatcacggtggatgccaaggcagccggtgaggggaaggtgacatgcacggtgtccacgccggatggggcagagctcgatgtggatgtggttgagaaccatgacggtacctttgacatctactacacagcgcccgagccgggcaagtacgtcatcaccatccgcttcgggggtgagcacatccccaacagccccttccacgtgctggcgtgtgaccccctgccgcacgaggaggagccctctgaagtgccacagctgcgccagccctacgctcctccccggcccggcgcccgccccacacactgggccacagaggagccagtggtgcctgtggagccaatggagtccatgctgaggcccttcaacctggtcatccccttcgcggtgcagaaaggggagctcacaggagaggtgcggatgccctcggggaagacggcacggcccaacatcaccgacaacaaggacggcaccatcacggtgaggtatgcacccactgagaaaggcctgcaccagatggggatcaagtatgacggcaaccacatccctgggagccccttacagttctatgtggatgccatcaacagccgccatgtcagtgcctatgggccaggcctgagccatggcatggtcaacaagccagccaccttcactattgtcaccaaagatgctggagaagggggtctgtcactggccgtggagggcccatccaaggcagagatcacctgtaaggacaacaaggatggcacctgcaccgtgtcctatctgccgactgcgcctggagactacagcatcatcgtgcgcttcgatgacaagcacatcccggggagccccttcacagccaagatcacaggtgatgactccatgaggacctcacagctgaatgtgggcacctccacggacgtgtcactgaagatcaccgagagtgatctgagccagctgaccgccagcatccgtgccccctcgggcaacgaggagccctgcctgctgaagcgcctgcccaaccggcacattgggatctccttcacccccaaggaggtcggggagcacgtggtgagcgtgcgcaagagtggcaagcatgtcaccaacagccccttcaagatcctggtggggccatctgagatcggggacgccagcaaggtgcgggtctggggcaaggggctttccgagggacacacattccaggtggcagagttcatcgtggacactcgcaatgcaggttatgggggcttggggctgagtattgaaggcccaagcaaggtggacatcaactgtgaggacatggaggacgggacatgcaaagtcacctactgccccaccgagcccggcacctacatcatcaacatcaagtttgctgacaagcacgtgcctggaagccccttcactgtgaaggtgaccggcgagggccgcatgaaggagagcatcacccggcggagacaggcaccttccatcgccaccatcggcagcacctgtgacctcaacctcaagatcccaggaaactggttccagatggtgtctgcccaggagcgcctgacacgcaccttcacacgcagcagccacacctacacccgcacggagcgcacggagatcagcaagacgcggggcggggagacaaagcgcgaggtgcgggtggaggagtccacccaggtcggcggggaccccttccctgctgtgtttggggacttcctgggccgggagcgcctgggatccttcggcagcatcacccggcagcaggagggtgaggccagctctcaggacatgactgcacaggtgaccagcccatcgggcaaggtggaagccgcagagatcgtcgagggcgaggacagcgcctacagcgtgcgctttgtgccccaggaaatggggccccatacggtcgctgtcaagtaccgtggccagcacgtgcccggcagcccctttcagttcactgtggggccgctgggtgaaggtggtgcccacaaggtgcgggccggaggcacagggctggagcgaggtgtggccggcgtgccagccgagttcagcatctggacccgggaggctggcgctgggggcctgtccattgctgtggagggtcctagcaaagcggagattgcatttgaggatcgcaaagatggctcctgcggcgtctcctatgtcgtccaggaaccaggtgactatgaggtctccatcaagttcaatgatgagcacatcccagacagcccctttgtggtgcctgtggcctccctctcggatgacgctcgccgtctcactgtcaccagcctccaggagacggggctcaaggtgaaccagccagcgtcctttgccgtgcagctgaacggtgcccggggcgtgattgatgcccgggtgcacacaccctcgggggctgtggaggagtgctacgtctctgagctggacagtgacaagcacaccatccgcttcatcccccacgagaatggcgtccactccatcgatgtcaagttcaacggtgcccacatccctggaagtcccttcaagatccgcgttggggagcagagccaggctggggacccaggcttggtgtcagcctacggtcctgggctcgagggaggcactaccggtgtgtcatcagagttcatcgtgaacaccctgaatgccggctcgggggccttgtctgtcaccattgatggcccctccaaggtgcagctggactgtcgggagtgtcctgagggccatgtggtcacttatactcccatggcccctggcaactacctcattgccatcaagtacggtggcccccagcacatcgtgggcagccccttcaaggccaaggtcactggtccgaggctgtccggaggccacagccttcacgaaacatccacggttctggtggagactgtgaccaagtcctcctcaagccggggctccagctacagctccatccccaagttctcctcagatgccagcaaggtggtgactcggggccctgggctgtcccaggccttcgtgggccagaagaactccttcaccgtggactgcagcaaagcaggcaccaacatgatgatggtgggcgtgcacggccccaagaccccctgtgaggaggtgtacgtgaagcacatggggaaccgggtgtacaatgtcacctacactgtcaaggagaaaggggactacatcctcattgtcaagtggggtgacgaaagtgtccctggaagccccttcaaagtcaaggtcccttgaatcccaaaagtgcctccccagcctcagcccccacctccagccacacacacattacacacacacacacacacacacaaatgtgccacacccagacacgcacagaatcagacactacaaacacctgccttgggggtgaagtgaaggcccagcctccccaccccaccgcgccccaggggttggaggaccttgtctgtgtcaggacagtgtccctccctgggaatgtgacatgagggccgactggggccaggctcaggggcagaggctgggacacaaggggctggcgagggctgcgaggccagggaagccctgagtttctggcggggctgagcagtgggggagcattgtgttgtgggtgtctgtgtgtgaggtcaccctcaaactgcaccgccggccagataccctcctgaccccgaggacttggtctggtctctctggtggctacaaccccagagttttaaggacttggaaaggaaagcacaatcagagaagaaaacagcccccgaaccagcaggagtggcctggcacatggaccggcctgagcgatgtgcactccacccaagccaggctcccagggggcctgatttctctctcactgtctctttttttaaaatggttgcacggctctgccccatggggggccttttttacacactgcgaggcccagctttctaggggacttttgcacatgtcatgcagctcagctgggagctgcttaggtggaaaactccaaataaagtgcggctgtcgca

SEQ ID NO: 10 - RNA, 3544 nt, Homo sapiens
  source 1..3544: mol_type = mRNA
acacgcgcagccagccggccgcctcccgcgcccaagcgcgccgctctgctgtgccctgcgcccttgccccgcgccagcttctgcgcccgcagcccgcccggcgcccccggtgaccgtgaccctgccctgggcgcggggcggagcaggcatgtcccgcccggggaccgctaccccagcgctggccctggtgctcctggcagtgaccctggccggggtcggagcccagggcgcagccctcgaggaccctgattattacgggcaggagatctggagccgggagccctactacgcgcgcccggagcccgagctcgagaccttctctccgccgctgcctgcggggcccggggaggagtgggagcggcgcccgcaggagcccaggccgcccaagagggccaccaagcccaagaaagctcccaagagggagaagtcggctccggagccgcctccaccaggtaaacacagcaacaaaaaagttatgagaaccaagagctctgagaaggctgccaacgatgatcacagtgtccgtgtggcccgtgaagatgtcagagagagttgcccacctcttggtctggaaaccttaaaaatcacagacttccagctccatgcctccacggtgaagcgctatggcctgggggcacatcgagggagactcaacatccaggcgggcattaatgaaaatgatttttatgacggagcgtggtgcgcgggaagaaatgacctccagcagtggattgaagtggatgctcggcgcctgaccagattcactggtgtcatcactcaagggaggaactccctctggctgagtgactgggtgacatcctataaggtcatggtgagcaatgacagccacacgtgggtcactgttaagaatggatctggagacatgatatttgagggaaacagtgagaaggagatccctgttctcaatgagctacccgtccccatggtggcccgctacatccgcataaaccctcagtcctggtttgataatgggagcatctgcatgagaatggagatcctgggctgcccactgccagatcctaataattattatcaccgccggaacgagatgaccaccactgatgacctggattttaagcaccacaattataaggaaatgcgccagttgatgaaagttgtgaatgaaatgtgtcccaatatcaccagaatttacaacattggaaaaagccaccagggcctgaagctgtatgctgtggagatctcagatcaccctggggagcatgaagtcggtgagcccgagttccactacatcgcgggggcccacggcaatgaggtgctgggccgggagctgctgctgctgctggtgcagttcgtgtgtcaggagtacttggcccggaatgcgcgcatcgtccacctggtggaggagacgcggattcacgtcctcccctccctcaaccccgatggctacgagaaggcctacgaagggggctcggagctgggaggctggtccctgggacgctggacccacgatggaattgacatcaacaacaactttcctgatttaaacacgctgctctgggaggcagaggatcgacagaatgtccccaggaaagttcccaatcactatattgcaatccctgagtggtttctgtcggaaaatgccacggtggctgccgagaccagagcagtcatagcctggatggaaaaaatcccttttgtgctgggcggcaacctgcagggcggcgagctggtggtggcgtacccctacgacctggtgcggtccccctggaagacgcaggaacacacccccacccccgacgaccacgtgttccgctggctggcctactcctatgcctccacacaccgcctcatgacagacgcccggaggagggtgtgccacacggaggacttccagaaggaggagggcactgtcaatggggcctcctggcacaccgtcgctggaagtctgaacgatttcagctaccttcatacaaactgcttcgaactgtccatctacgtgggctgtgataaatacccacatgagagccagctgcccgaggagtgggagaataaccgggaatctctgatcgtgttcatggagcaggttcatcgtggcattaaaggcttggtgagagattcacatggaaaaggaatcccaaacgccattatctccgtagaaggcattaaccatgacatccgaacagccaacgatggggattactggcgcctcctgaaccctggagagtatgtggtcacagcaaaggccgaaggtttcactgcatccaccaagaactgtatggttggctatgacatgggggccacaaggtgtgacttcacacttagcaaaaccaacatggccaggatccgagagatcatggagaagtttgggaagcagcccgtcagcctgccagccaggcggctgaagctgcgggggcagaagagacgacagcgtgggtgaccctcctgggcccttgagactcgtctgggacccatgcaaattaaaccaacctggtagtagctccatagtggactcactcactgttgtttcctctgtaattcaagaagtgcctggaagagagggtgcattgtgaggcaggtcccaaaagggaaggctggaggctgaggctgttttcttttctttgttcccatttatccaaataacttggacagagcagcagagaaaagctgatgggagtgagagaactcagcaagccaacctgggaatcagagagagaaggagaaggaggggagcctgtccgttcagagcctctggctgcatagaaaaggattctggtgcttcccctgtttgcgtggcagcaagggttccacgtgcatttgcaatttgcacagctaaaattgcagcatttccccagctgggctgtcccaaatgttaccatttgagatgctcccaggcgtcctaagagaatccaccctctctggccctgggacattgcaagctgctacaaataaattctgtgttcttttgacaatagcgtcattgccaagtgcacatcagtgagcctcttgaatctgtttagtctcctttttcaacaaaggagtgtgttcagaaaaggagagagaggctgagatcattcaggagtttgttgggcagcaagcatggagcttcttgcacaaattctgggtccataaacaacccccaaagtccctgctgatccagtagccctggaggttccccaggtagggagagccagaggtgccagccttcctgaagggccagaaaatttagcctggatctcctcttttacctgctaggactggaaagagccagaagtggggtggcctgaagccctctctctgcttgaggtattgcccctgtgtggaattgagtgctcatgggttggcctcatatcagcctgggagttatttttgatatgtagaatgccagatcttccagattaggctaaatgtaatgaaaacctcttaggattatctgtggagcatcagtttgggaagaattattgaattatcttgcaagaaaaaagtatgtctcactttttgttaatgttgctgcctcattgacctgggaaaaatgaaaaaaaaaaataaagcaaatggtaagacc

SEQ ID NO: 11 - RNA, 4377 nt, Homo sapiens
  source 1..4377: mol_type = mRNA
atgcctcccgccgccccgtccgtcgcccggagccggggagggagggagcgaggttcggacaccggcggcggctgcctggcctttccatgagcccgcggcggaccctcccgcgccccctctcgctctgcctctccctctgcctctgcctctgcctggccgcggctctgggaagtgcgcagtccgctcttgcccctgttctttgcttctcgttttgttggtgaagatatcacagtgatgtctgcattcaacctgctgcatttggtgacaaagagccagccagtagcccttcgagcctgtgggcttccctcagggtcgtgtagggataaaaagaactgtaaggtggtcttttcccagcaggaactgaggaagcggctaacacccctgcagtaccatgtcactcaggagaaagggaccgaaagtgcctttgaaggagaatacacacatcacaaagatcctggaatatataaatgtgttgtttgtggaactccattgtttaagtcagaaaccaaatttgactccggttcaggttggccttcattccacgatgtgatcaattctgaggcaatcacattcacagatgacttttcctatgggatgcacagggtggaaacaagctgctctcagtgtggtgctcaccttgggcacatttttgatgatgggcctcgtccaactgggaaaagatactgcataaattcggctgccttgtcttttacacctgcggatagcagtggcaccgccgagggaggcagtggggtcgccagcccggcccaggcagacaaagcggagctctagagtaatggagagtgatggaaacaaagtgtacttaatgcacagcttattaaaaaaatcaaaattgttatcttaatagatatattttttcaaaaactataagggcagttttgtgctattgatattttttcttcttttgcttaaacagaagccctggccatccatgtattttgcaattgactagatcaagaactgtttatagctttagcaaatggagacagctttgtgaaacttcttcacaagccacttataccctttggcattcttttctttgagcacatggcttcttttgcagtttttccccctttgattcagaagcagagggttcatggtcttcaaacatgaaaatagagatctcctctgcagtgtagagaccagagctgggcagtgcagggcatggagacctgcaagacacatggccttgaggcctttgcacagacccacctaagataaggttggagtgatgttttaatgagactgttcagctttgtggaaagtttgagctaaggtcatttttttttttctcactgaaagggtgtgaaggtctaaagtctttccttatgttaaattgttgccagatccaaaggggcatactgagtgttgtggcagagaagtaaacattaccacactgttaggcctttattttattttattttccatcgaaagcattggaggcccagtgcaatggctcacgcctgtgatcccagcactttgggaggccaaggcgggtggatcacgaggtcaggagatggagaccatcctggctaacatggtgaaaccccgtctctactaaaaatacgaaaaattagccaggcgtggtggtgggcacctgtagtcccagctactcaggaggctgaggcaggagaatggcgtgaacccggaaggcggagcttgcagttagccgagatcatgccactgcactccagcctacatgacaatgtgacactccatctcaaaaaataataataataacaatataagaactagctgggcatggtggcgcatgcatgtagtcccagctactcctgaggctcagtcaggagaatcgcttgaacttgggaggcggaggttgcagtgagctgagctcataccactgcactccagcctgaacagagtgagatcctgtcaaaaaagaaaagaaaaagaaagcagcattcaaatgtaagacaactgtaaaatattgagccccacttggtctaaaattcaaaaagaagaacgcctgtccatcgcctttttataagtccttctctccacacctaaaagcagctgcagctggaagggcacaaattccactgtgtaaaataaaatattaggggcaacacacttcatcaaggcagcaggaatgagagagagcagagaagatcaaggatgaagtcttgggtactgaaaaattcagtgctgggcagaaaaactgacagggcagtacaagtaacaaacagaatccaagtggggtggcccttgtgcacagagctccaggtgacctctggagagacatgggcattcacatggaaagctaaaacggaagctcaagtttcatactcaacataatcttctgtgtgacaaaggacaagccatgtagcctctctgtgcctatttcttcatgcataaactgggactcataatatttgtaaaatgtattgatactctcagggcaaattcactatattgctatacagttgagatcagtgttgtaaaattaaactgatctggttctaattgcctcaaaggccaaagcccaggcatttgaaatggaaagaagcagagaggaggctgacttagctgattggtatggaaacagttgggccaagagccagaatttccctttgtagcaacacggctagttttactttgagaagctctgctcagctgctttataacattaagtctggcggaatggatgtcactgtgcacaataaagttttcacaagtataaacaatggtgatgtaagtcaacattgctgtagccaggtgtgaaggttgtatggtgtgtgacgaatgtacatcatgtttgtaggtttggatgctaatcttgaattgtagtttaaaaaatacgtatttttgtaactctttgaaagtttatgaagactgacagctttccttgtaagcactaagagaaaaaaaagaaagagggacatttgacaattttaaagaaacaacaagaaattagaatgaaaatctgtgacaaacagcgtcagtgtggccatgtccacattcctacatgtctctctctacaagcacctctctaagaagcctgacatcccggtggactctttatagtcatgtacacttgattccagatgagctctggtcttatctggatgctcagataagaggtttctatctgagcatccagatgttccctcaggttccaagacatttcaccccaggccctgggttcactctggaattcgtaggcttcacgtctctctagaaatgacgtgtaaaatttaagaccagacctcagccatcagcgtccagaccatcctagaagtctttcccaatctcacagagaaagccctagtatttcccagtgaccccaggattccacgttggggtggccaaagaaataggtctctcagggctttgccacagcctccagcccatccttcagaggcacacacagcacctctcggctgctccagctctgtaggatagcctcccctggggtccgtgggacgcgggccacagtgttgaggtagacaaggaggatcagtgagaggcctcttccctctccacagagactggattgtcattgttccttcatttatatcgtagggcttaacatttcactcaaaaaaaagcccctctttttctaatccttagtctttgtttcaaggaaagccagtttttcttctaccacattttccaggatcgactttaagaaaaatgcaacatctattgaaaaaaagtggggtgtatgcatgtggtttaattccagattgcttttgggtttaagtggtatcaaatttcagtatatttctgtcttatgtgaaagaaatatattactaaaacgtcagtgagcaataatgtcagctgtcaagcactagatttatttttgcaggatatggagtgcaatgaactgagtcaatatggcaaggtgtatgtgatctgtgggagttatgccatttaacataggaagtgcatgggactttccctctctgcactccagctcttactgtaccattagaagatgcagaattctgttggtgtgcaaaaagtatagccttacattcaagcagaatggatctgaagaaagcagcaatatctgttactagagaacattcccatgtgtttaaactcttcacttcttagatgcatttaaattcttaatgcaaatgacgtagcaatttgaaaacttctccgtattacttgtgtttaaaatgtcttgctttaaatacaaaacaaatggtaaaggggattatcttttgtttagatggttaaatattatttttgccttagatagctttgtaataatttttctccagacagttcaacacttttgaaaaatgacatgaattttcattaaaaacccttttcctatgtttattgtatacaagaattatgcaataaaatttctttataaaaata

SEQ ID NO: 12 - RNA, 1705 nt, Homo sapiens
  source 1..1705: mol_type = mRNA
cctttggcttggcttgtcagggcttgtccaggagttccgctcctctctccaaccggggtccccctccagcgaccctaaagcttcccagacttccgcttcaattcctgtccgcaccccacgcccacctcaacgtggagcgcagtggtctccgaggagcgccggagctgccccgcctgcccagcggggtcagcacttcgcatcaaggcccaagaaaagcaagtcctccagcgttctgagcacccgggcctgagggaaggtcctaacagcccccgggagccagtctccaacgcctcccgcagcagcccgccgctcccaggtgcccgcgtgcgccgctgccgccgcaatcccgcacgcgtcccgcgcccgccccactttgcctatccccgggactaagacgggaatcctgtgaagcagctccagctatgtgtgaagaagaggacagcactgccttggtgtgtgacaatggctctgggctctgtaaggccggctttgctggggacgatgctcccagggctgttttcccatccattgtgggacgtcccagacatcagggggtgatggtgggaatgggacaaaaagacagctacgtgggtgacgaagcacagagcaaaagaggaatcctgaccctgaagtacccgatagaacatggcatcatcaccaactgggacgacatggaaaagatctggcaccactctttctacaatgagcttcgtgttgcccctgaagagcatcccaccctgctcacggaggcacccctgaaccccaaggccaaccgggagaaaatgactcaaattatgtttgagactttcaatgtcccagccatgtatgtggctatccaggcggtgctgtctctctatgcctctggacgcacaactggcatcgtgctggactctggagatggtgtcacccacaatgtccccatctatgagggctatgccttgccccatgccatcatgcgtctggatctggctggccgagatctcactgactacctcatgaagatcctgactgagcgtggctattccttcgttactactgctgagcgtgagattgtccgggacatcaaggagaaactgtgttatgtagctctggactttgaaaatgagatggccactgccgcatcctcatcctcccttgagaagagttacgagttgcctgatgggcaagtgatcaccatcggaaatgaacgtttccgctgcccagagaccctgttccagccatccttcatcgggatggagtctgctggcatccatgaaaccacctacaacagcatcatgaagtgtgatattgacatcaggaaggacctctatgctaacaatgtcctatcagggggcaccactatgtaccctggcattgccgaccgaatgcagaaggagatcacggccctagcacccagcaccatgaagatcaagatcattgcccctccggagcgcaaatactctgtctggatcggtggctccatcctggcctctctgtccaccttccagcagatgtggatcagcaaacaggaatacgatgaagccgggccttccattgtccaccgcaaatgcttctaaaacactttcctgctcctctctgtctctagcacacaactgtgaatgtcctgtggaattatgccttcagttcttttccaaatcattcctagccaaagctctgactcgttacctatgtgttttttaataaatctgaaataggctactggtaa

SEQ ID NO: 13 - RNA, 2570 nt, Homo sapiens
  source 1..2570: mol_type = mRNA
aatatagcggctcgccgaggcgctggtgcacgggggcagcgcgcagcaggccggcgggcaggcgggcgggctggctggcaggcaggactgggatcgaggcccagaaaacggagcagcgggcaccagggaggcctggaacggggcgagcgccatgagcaacaaatgcgacgtggtcgtggtggggggcggcatctcaggtatggcagcagccaaacttctgcatgactctggactgaatgtggttgttctggaagcccgggaccgtgtgggaggcaggacttacactcttaggaaccaaaaggttaaatatgtggaccttggaggatcctatgttggaccaacccagaatcgtatcttgagattagccaaggagctaggattggagacctacaaagtgaatgaggttgagcgtctgatccaccatgtaaagggcaaatcataccccttcagggggccattcccacctgtatggaatccaattacctacttagatcataacaacttttggaggacaatggatgacatggggcgagagattccgagtgatgccccatggaaggctccccttgcagaagagtgggacaacatgacaatgaaggagctactggacaagctctgctggactgaatctgcaaagcagcttgccactctctttgtgaacctgtgtgtcactgcagagacccatgaggtctctgctctctggttcctgtggtatgtgaagcagtgtggaggcacaacaagaatcatctcgacaacaaatggaggacaggagaggaaatttgtgggcggatctggtcaagtgagtgagcggataatggacctccttggagaccgagtgaagctggagaggcctgtgatctacattgaccagacaagagaaaatgtccttgtggagaccctaaaccatgagatgtatgaggctaaatatgtgattagtgctattcctcctactctgggcatgaagattcacttcaatccccctctgccaatgatgagaaaccagatgatcactcgtgtgcctttgggttcagtcatcaagtgtatagtttattataaagagcctttctggaggaaaaaggattactgtggaaccatgattattgatggagaagaagctccagttgcctacacgttggatgataccaaacctgaaggcaactatgctgccataatgggatttatcctggcccacaaagccagaaaactggcacgtcttaccaaagaggaaaggttgaagaaactttgtgaactctatgccaaggttctgggttccctagaagctctggagccagtgcattatgaagaaaagaactggtgtgaggagcagtactctgggggctgctacacaacttatttcccccctgggatcctgactcaatatggaagggttctacgccagccagtggacaggatttactttgcaggcaccgagactgccacacactggagcggctacatggagggggctgtagaggccggggagagagcagcccgagagatcctgcatgccatggggaagattccagaggatgaaatctggcagtcagaaccagagtctgtggatgtccctgcacagcccatcaccaccacctttttggagagacatttgccctccgtgccaggcctgctcaggctgattggattgaccaccatcttttcagcaacggctcttggcttcctggcccacaaaagggggctacttgtgagagtctaaagagagagggtgtctgtaatcacactctcttcttactgtatttgggatatgagtttggggaaagagttgcagtaaagttccatgaagacaaatagtgtggagtgaggcggggagcatgaagataaatccaactctgactgtaaaatacatggtatctctttctccgttgtggcccctgcttagtgtcccttacctggcttagcgttctgtttcaccagtttccaagtttattgccctcaaaatctttagaatagttaaattggcttgtttaaggttcttgctgccccacaacacaccttgcccatgcacaaggaatgaattttttcctaccattatggctttgtgcttgttcttcctcttacctgtaatagcctcaccttccctagttctttgcattcgtccttagaatactgtattgttacagctgaaagacagtaaagaccatttagtcctcaccttctgttttagagttgagcaaactgaagcccacagaggtggaacttaattacctaagagccacaataagccactggtatctgggggactagaacacaaatccaacgcttttcccacctctttggatgttttccccaattatcctccttcactccctgtcatagttaccgatggtgtcccgttgtgtgggtttactctgtgctaagttgtcttacacttctcaaatgctactcagtatatagccttaagtcttactgttttgtgcggtgtgtctccagctgattttaacttttttgatggtagaaattttatctcttcttccttttgtatcctccattgtatcttcatacaaaggacagtacacacttgggtaattaaaaataaaagttgattgaccata

SEQ ID NO: 14 - RNA, 3282 nt, Homo sapiens
  source 1..3282: mol_type = mRNA
agccagaggactcccagcggctggagcagaagtgttagcggccagagctcccagacccctacccacagccaggcgggacgcgcacagtccctccacgcggaaagaagtaccttcgccggtcaccggctcctgcagggtgcaaatatatacagagcttcataatcagcccaagaccacatagagcaaacatgaatgatatttcccaaaaggctgagattctgctttcttcatctaaacctgtcccaaaaacctatgtaccaaaacttggcaagggtgatgtaaaggataagtttgaagccatgcagagagccagggaagaaagaaatcaaaggagatctagagacgaaaaacaaagaagaaaagaacaatatattagagagagagaatggaacaggagaaagcaggagattaaagaaatgcttgcttctgatgatgaggaagatgtatcttctaaagtagaaaaggcttatgttccaaaattaacaggaactgtgaagggtagatttgctgaaatggagaaacaaagacaagaggaacaaaggaagagaacggaggaggaacgaaaacgcagaattgagcaggatatgttagaaaagaggaaaatacagcgtgaattagcaaaaagggctgaacagattgaggacataaacaatacgggaactgaatcagcatcagaggaaggagatgattcactacttataactgtggtacctgtcaaatcatataaaacatctggaaaaatgaaaaagaattttgaggatctagaaaaagaacgtgaagagaaagaaaggatcaagtacgaggaagataaaagaataagatatgaagaacaacgaccatctctcaaggaagcaaagtgtctttcattagttatggatgatgaaatagaaagtgaagcaaaaaaagaatcactttctcccggaaaattgaaactaacttttgaagaactggagcgacaaagacaagaaaaccgaaagaagcaagctgaagaggaagcaagaaaacgtttagaagaagagaagcgtgcttttgaagaagcaaggcggcaaatggtaaatgaagatgaggaaaaccaagacacagcaaaaatttttaaagggtaccgccctggtaaactcaaactcagttttgaagaaatggaaaggcaaagaagagaagatgaaaaaaggaaagcagaagaagaagccagaaggagaatagaggaagaaaagaaggcgtttgctgaagcaaggagaaatatggtagtagatgatgactccccagagatgtataagacaatctctcaagaatttcttacaccgggaaaactggaaattaattttgaagaattattaaaacaaaaaatggaagaagaaaaacgacgaacagaggaggaacggaagcataagctagaaatggagaaacaagaatttgaacaactgagacaggaaatgggagaggaagaggaagaaaatgaaacctttggattgagcagagaatatgaagaactgatcaaattaaaaaggagtggctctattcaagctaaaaacctaaaaagcaagtttgaaaaaattggacagttgtctgaaaaagaaatacagaaaaaaatagaagaagagcgagcaagaaggagagcaattgaccttgaaattaaagagcgagaagctgaaaattttcatgaggaagatgatgttgatgttaggcctgcaagaaaaagcgaggctccatttactcacaaagtgaatatgaaagctagatttgaacaaatggctaaggcaagagaagaagaagaacaaagaagaattgaagaacaaaagttactacgcatgcagtttgaacaaagggaaattgatgcagcactacaaaagaaaagagaagaggaggaggaggaagaaggtagcatcatgaatggctccactgctgaagatgaagagcaaaccagatcaggagctccatggttcaagaagcctcttaaaaacacatcagttgtagacagtgagccagtcagatttacggttaaagtaacaggagaacccaaaccagaaattacatggtggtttgaaggagaaatactgcaggatggagaagactatcaatatattgaaaggggagaaacttactgcctttacttaccagaaactttcccagaagatggaggagagtatatgtgtaaagcagtcaacaataaaggatctgcagctagtacctgtattcttaccattgaaagtaagaattaatcactctttttatcttttattctattaatttttttttccttaaaatcacttttcttcttctcttttttagctgatgactactagctcccctcccctctccctggaactttctctttcactccaactttcttactacatccatcttttctgtggcggggccaaaaaaggaaaccaggagtgccactatgctgacttcttattccttttcataacagtcttcaaagcacagctcatctaaagaatgcctacttcttttccaaataagcatcagatttatcgcctattatgcagtaacagtcaataaaatgtacttatgggggggaattactcaattattctatcagaacctattataaagactgtatttcccatagacgtttacagcaactatgtttaaaaaacaaaaacaaaaaaaaaacacacaaacctaagtagaatacattattttgcatgaaggaatgtcatttctgagctttttacacctaaaattaggctgaaatagctgagataattaatttggaacctatcaatttgagtggactttttctttagtagtacaccattttggttgttgtagtttcaaagtctttctgaagcagatatattgggattggagcggggtggggaaaactgtcactcctttcagaggaaaaggggaggagcatggagaaaaacaaaaattaaaggacttaaagaatggctatacagtgttgagtgttgaggatattaaacatgttatttttcaaacgtatgtaatatatattaaatttataaagcaaatttatgttgtgatcttgcctgaacaaattatattttaatgaaaaaactttctattaatagttcacgcaagagaaaacactttcaacatagtcgaaggcttcaagatctaagtgtatcagacttagggaaaaagtggcacaaccttcgatttaaaattctagtctttaaaatgagtttgtaaataattagctattacgttctattaagttgttttatattttaattttctggaagacaattttattttacaacgtgaacccaaataaagtaacttctgtatttaaaa

SEQ ID NO: 15 - RNA, 3537 nt, Homo sapiens
  source 1..3537: mol_type = mRNA
gccccggggtaagctcgcgccgccgcgtcagctcagcgctgggtctctcggtcccgcagccgtgaggaggacggtctgcatactcgctgcccgccggctccctcccccgcgtccctgcgaccgccgcggcgaagatgattttcagttcacccactagaggcaaagacgtaagagagctaccagcgtattgagaggagatacacaggcactacgagaatggagtttagaagaaggtcagagccctgggcagtgttgggccaggctttagggcctcaggagtgcaagtagctgatgaagtatgtcgcattttttatgacatgaaagttcgtaaatgctccacaccagaagaaatcaagaaaagaaagaaggctgtcattttttgtctcagtgcagacaaaaagtgcatcattgtagaagaaggcaaagagatcttggttggagatgttggtgtaaccataactgatcctttcaagcattttgtgggaatgcttcctgaaaaagattgtcgctatgctttgtatgatgcaagctttgaaacaaaagaatccagaaaagaagagttgatgttttttttgtgggcaccagaactagcacctctgaaaagtaaaatgatctatgcaagctccaaggatgcaattaaaaagaaatttcaaggcataaaacatgaatgtcaagcaaatggaccagaagatctcaatcgggcttgtattgctgaaaagttaggtggatccttaattgtagcctttgaaggatgccctgtgtagattattcagtgccacaaattgaaagcttccatgtttaatgttatcctcttgctatataaataaagcaaatatatttaggccagggtctcactgagggggagctgtcttgtcatcttttagagtaaactattctataaacatatgcaaacagccctaaataaatctaaagtctaaagttttattgatgtgaaattaaattcttattggccaaatgcctgttttgatgagttgatttataaagatttttgttaagctcaggattttaaattacacagttcacaaacagtaaaggccatgtgaagagaattattacatctttattaacctcagcatttactttgtttcttttgcttaggaaattgctcataatctggttataattttggtccaaattctttattcttccttgagctaagcagaataatggaatataatatgtcttcataatataacaacactaatacactaatagtaagattaagttaggcagtcttctaccaaatgtgtaatggagattgcctcaaaattgtgtccacataatccacgctcatcttgcaaagcgctatttcaggcacatcattggaatacaggaagtagccctgcacctgccagtgagctcgccattcactgattggaagagtgacctggcatcttggaaatcattgtgtgtcttcaggagaatgtgcagtgtcttgtaacaactaattataatgcaaattagggctacattgtaatctgctttgttaatgaaaatgataaaacagaatattgacaagctaggacacctgtggtatctttaattgtatctccttcagaagtttgcttcttatggtataataaagtatggaagaatattgagtatatgtttactctgggcctgggagaacttaactttctagagcagtttgttgacttgtgtgcaatggggagaggtaccatgatgacactcacagggagccactgttcactgacacttggaagcggtcattgttaatatcacgggcgtaacactttgaacgatatagagatgcacaaacagttgaacttagaagtagcagtattggctttatgtaataaaggaagcatttttgacttacctctcgtgtaattttcatgtgtgaattgggaatacaggattttgccttccatatggggtaaggcattgaggtttgggtatttccaataattaagagttaaggttggctgagtgtggtggctcactcctgtaatcccagcattttgggaggccgaggcaagaggatagtttgaggccaggagtttgacaatcagcgtgggcaacatagtgggatctcatctactaaaaataaacaaaattagccgggtgtggtggtgcacgtcagtagtcccagctactttggatgctgaggtgggaggatcacttgagcccaggaggtgagctgagatcgtgccactgtactccagcctggatgacagagcaagaccttgtctcaaaaaaaaaaaaaaaagtcacaactccctctggtgaataagaaagttggtgtaaaagttgggaacgttttcaatgtttattacactataagtgtaataaatattatacaaaattataaattcacatttaaaatttagaaaatagagaaaagggaaattatacattgtcctaccacatgccatcacatggttagcattttgatacacagctgtgcattattacatgtcaaagactgcatatactatggtggtcccatacaattataatgtattttctactgtaattagatacacaaataccattgtgttacagttgccgacagtattcagtatagtaacgtgctgtccaggtttgtggtctaggagtaataggctctaccatacagcctaggtgtgtagtaggctatgccactaggtttaagtgcagtctagggtggggaacattttaatgttgatccacatgccaggtgtttgtgagacaagattatgctttaatcaaaatattttggaattgtctagaaaatagtgctggctgcttgtcattcatcctgaattgcttgtttctttactttgtagcaatgcttttagtgtgggttttgttttttgagacagggtctcactctttcccccaggctagagtgcagtggtgcaatcataactcactgcatccttgaactcttgggctccagcaagcctcctgccttggcctcctaaagtgctgtgattacaggtgtgagccactgtgtcctgctagtgattgtgattaacaggcctccagggaagtgccataagcccaagactgccgtactcaaaagtcagccatgtaggtaaagcaagatatttggtcaaggagttttagaaggagatttttcctgtggtgttggcttaagtgtggcactgttgtgcgtgtgtgaggtgtcttctgtgggaaggatttcaaacagtacaaagggatgtgatgtaagcatccagaactcactccagaaattgaataaaatgctagtagttagtctctaggggaacttttgagaaagtctcagtggattcctgaggcccaagaattgtgctaacaagcactcaaggcgattctggtacataattagggttcagacctcagctgattggtctactgttggtcaggaacaaaactgcaagtatactctgtttccagaaaatacgtttacctcttcacaaatgctaacacactgcaaaaatatgtttgtggaaagctgacttagtctcatctagcggttactctcttgccctgacaaagcagcaaataaagccattgctaacaattcaa

SEQ ID NO: 16 - RNA, 5020 nt, Homo sapiens
  source 1..5020: mol_type = mRNA
agtgtgcgaggcgcacgcacaggagcctgcactctgcgtcccgcaccccagcagccgcgccatgagccggagtctcttgctctggttcttgctgttcctgctcctgctcccgccgctccccgtcctgctcgcggacccaggggcgcccacgccagtgaatccctgttgttactatccatgccagcaccagggcatctgtgtccgcttcggccttgaccgctaccagtgtgactgcacccgcacgggctattccggccccaactgcaccatccctggcctgtggacctggctccggaattcactgcggcccagcccctctttcacccacttcctgctcactcacgggcgctggttctgggagtttgtcaatgccaccttcatccgagagatgctcatgcgcctggtactcacagtgcgctccaaccttatccccagtccccccacctacaactcagcacatgactacatcagctgggagtctttctccaacgtgagctattacactcgtattctgccctctgtgcctaaagattgccccacacccatgggaaccaaagggaagaagcagttgccagatgcccagctcctggcccgccgcttcctgctcaggaggaagttcatacctgacccccaaggcaccaacctcatgtttgccttctttgcacaacacttcacccaccagttcttcaaaacttctggcaagatgggtcctggcttcaccaaggccttgggccatggggtagacctcggccacatttatggagacaatctggagcgtcagtatcaactgcggctctttaaggatgggaaactcaagtaccaggtgctggatggagaaatgtacccgccctcggtagaagaggcgcctgtgttgatgcactacccccgaggcatcccgccccagagccagatggctgtgggccaggaggtgtttgggctgcttcctgggctcatgctgtatgccacgctctggctacgtgagcacaaccgtgtgtgtgacctgctgaaggctgagcaccccacctggggcgatgagcagcttttccagacgacccgcctcatcctcataggggagaccatcaagattgtcatcgaggagtacgtgcagcagctgagtggctatttcctgcagctgaaatttgacccagagctgctgttcggtgtccagttccaataccgcaaccgcattgccatggagttcaaccatctctaccactggcaccccctcatgcctgactccttcaaggtgggctcccaggagtacagctacgagcagttcttgttcaacacctccatgttggtggactatggggttgaggccctggtggatgccttctctcgccagattgctggccggatcggtgggggcaggaacatggaccaccacatcctgcatgtggctgtggatgtcatcagggagtctcgggagatgcggctgcagcccttcaatgagtaccgcaagaggtttggcatgaaaccctacacctccttccaggagctcgtaggagagaaggagatggcagcagagttggaggaattgtatggagacattgatgcgttggagttctaccctggactgcttcttgaaaagtgccatccaaactctatctttggggagagtatgatagagattggggctcccttttccctcaagggtctcctagggaatcccatctgttctccggagtactggaagccgagcacatttggcggcgaggtgggctttaacattgtcaagacggccacactgaagaagctggtctgcctcaacaccaagacctgtccctacgtttccttccgtgtgccggatgccagtcaggatgatgggcctgctgtggagcgaccatccacagagctctgaggggcaggaaagcagcattctggaggggagagctttgtgcttgtcattccagagtgctgaggccagggctgatggtcttaaatgctcattttctggtttggcatggtgagtgttggggttgacatttagaactttaagtctcacccattatctggaatattgtgattctgtttattcttccagaatgctgaactccttgttagcccttcagattgttaggagtggttctcatttggtctgccagaatactgggttcttagttgacaacctagaatgtcagatttctggttgatttgtaacacagtcattctaggatgtggagctactgatgaaatctgctagaaagttagggggttcttattttgcattccagaatcttgactttctgattggtgattcaaagtgttgtgttcctggctgatgatccagaacagtggctcgtatcccaaatctgtcagcatctggctgtctagaatgtggatttgattcattttcctgttcagtgagatatcatagagacggagatcctaaggtccaacaagaatgcattccctgaatctgtgcctgcactgagagggcaaggaagtggggtgttcttcttgggacccccactaagaccctggtctgaggatgtagagagaacaggtgggctgtattcacgccattggttggaagctaccagagctctatccccatccaggtcttgactcatggcagctgtttctcatgaagctaataaaattcgctttctaaagttacctgttatatatctcttttggtcccatcctctaaagcagaggcaacactggaacatggctagcctttcttgtagccatggctgggcgtgctagaggttgcagcatgagactttctgctgggatccttgggcccatcactgtatagacatgctaccactggtacttcctttctccctgcgggccaggcactgcccttttcaggaagctctcttaaaatacccattgccccagacctggaagatataacattcagttcccaccatctgattaaaacaacttcctcccttacagagcatacaacagagggggcacccggggaggagagcacatactgtgttccaatttcacgcttttaattctcatttgttctcacaccaacagtgtgaagtgcgtggtataatctccatttcaaaaccaaggaagcagcctcagagtggtcgagtgacacacctcacgcaggctgagtccagagcttgtgctcctcttgattcctggtttgactcagttccaggcctgatcttgcctgtctggctcagggtcaaagacagaatggtggagtgtagcctccacctgatattcaggctactcattcagtcccaaatatgtattttcctaagtgtttactatgtgccagttcctgtaacaggtgtggggacacagcagtgagtaatcaatacagacaaggttctgcccttatggagctcacactccagtggcagacaaacagaccataaataaggaaacgatgaaataagatatatacaaggtgagtgtgacttcccttctaaccccctctgctctgtcctcccctattgcgctctcaagaccagagacccaacagcagtgatctcagggcagacagccctccactccagctctgagacccttttctcaggacctctgtaggcagcagagagagaggacagaggggtaagatgaggggttgagggaaggttcttcatgatccacactttgggcttagtatttctcaggaagagctatggcccagaaacaacaggggaaactagagttcggtctgacagtccttggggttaagtctcctgtcttatggtccagaaactcctgtttctccttagttggctggaaactgctcccatcattccttctggcctctgctgaatgcagggaatgcaatccttccctgctcttgcagttgctctgacgtagaaagatccttcgggtgctggaagtctccatgaagagcttgtgtcctgtcctttcttgcagattctatttcccctcttctgctaatacctcttactttgcttgagaatcctctcctttcttattaatttcagtcttggtggttctatcaggggtgcattctggccaaggggtgggcctgtgaatcaatcctgggcaatcagacaccctctccttaaaaactggcccgtggagactgagatcactgactctgactcatccccacagctggctctgacaagatggtccatttgttcctgcttccgagatccccagggcagcctggatccctgcccttctcaagactttagcttttccttccatccggtggcctattccaggaattcctcttttgcttaaatcagttggagtttgtgtctgttgcttgtaatcaagcctttatggctgctgggctgagtgacacaagcactttaatggcctggagggacttttaatcagtgaagatgcaatcagacaagtgttttggaaagagcaccctcgagaagggtggatgacagggcagagcaggaaggacaggaagctggcagaacggaggaggctgcagccgtggtccaaccaggagctgatggcagctggggctaggggaagggctttgagggtggaaggatgggatgggttccagaggtattcctctcttaaatgcaagtgcctagattaggtagactttgcttagtattgacaactgcacatgaaagttttgcaaagggaaacaggctaaatgcaccaagaaagcttcttcagagtgaagaatcttaatgcttgtaatttaaacatttgttcctggagttttgatttggtggatgtgatggttggttttatttgtcagtttggttgggctatagcacacagttatttaatcaaacagtaatctaggtgtggctgtgaaggtattttgtagatgtgattaacatctacaatcagttgactttaagtgaaagagattacttaaataatttgggtgagctgcacctgattagttgaaaggcctcaagaacaaacactgcagtttcctggaaaagaagaaactttgcctcaagactatagccatcgactcctgcctgagtttccagcctgctagtctgccctatggatttgaagtttgccaaccccaacaattgtgtgaattaatttctaaaaataaagctatatacagcca

SEQ ID NO: 17 - RNA, 4081 nt, Homo sapiens
  source 1..4081: mol_type = mRNA
gccccgctcgccgcacggcccggcgacgggggagttcccgcgagtggcctcgcgcccagaccgtgcggggggctgttcgggtggaggcgggggagccgccgggacaccaaaataggagctgcttgtggggtggagcggcactagctggcggcttccgagcgcctcttccaaagatggtcagaggggccggaggcgtccccgctcccgctcgctactagcccgcgggccagcgccgcgtcccgagccccggcgggagccatggctctaaaaggacaagaagattatatttatcttttcaaggattcaacacatccagtggattttctggatgcattcagaacattttacttggatggattatttactgatattactcttcagtgtccttcaggcataattttccattgtcaccgagccgttttagctgcttgcagcaattattttaaggcaatgttcacagctgacatgaaagaaaaatttaaaaataaaataaaactctctggcatccaccatgatattctggaaggccttgtaaattatgcatacacttcccaaattgaaataactaaaagaaatgttcaaagcctgcttgaggcagcggatctgctacagttcctttcagtaaagaaggcttgtgagcggtttttggtaaggcacttggatattgataattgtattggaatgcactcctttgcagaatttcatgtgtgtccagaactagagaaggaatctcgaagaattctatgttcaaagtttaaggaagtgtggcaacaagaagaatttctggaaatcagccttgaaaagtttctctttatcttgtccagaaagaatctcagtgtttggaaagaagaagctatcatagagccagttattaagtggactgctcatgatgtagaaaatcgaattgaatgcctctataatctactgagctatatcaacattgatatagatccagtgtacttaaaaacagccttaggccttcaaagaagctgcctgctcaccgaaaataagatccgctccctaatatacaatgccttgaatcccatgcataaagagatttcccagaggtccacagccacaatgtatataattggaggctattactggcatcctttatcagaggttcacatatgggatcctttgacaaatgtttggattcagggagcagaaataccagattataccagggagagctatggtgttacatgtttaggacccaacatttatgtaactgggggctacaggacggataacatagaagctcttgacacagtgtggatctataacagtgaaagtgatgaatggacagaaggtttgccaatgctcaatgccaggtattaccactgtgcagtcaccttgggtggctgtgtctatgctttaggtggttacagaaaaggggctccagcagaagaggctgagttctatgatcctttaaaagagaaatggattcctattgcaaacatgattaaaggtgtgggaaatgctactgcctgtgtcttacatgatgttatctacgtcattggtggccactgtggctacagaggaagctgcacctatgacaaagttcagagctacaattccgatatcaacgaatggagcctcatcacctccagtccacatccagaatatggattgtgctcagttccgtttgaaaataagctctatctagtcggcggacaaactacaatcacagaatgctatgaccctgaacaaaatgaatggagagagatagctcccatgatggaaaggaggatggagtgcggtgccgtcatcatgaatggatgtatttatgtcactggaggatactcctactcaaagggaacgtatcttcagagcattgagaaatatgatccagatcttaataagtgggaaatagtgggtaatcttcccagtgccatgcggtctcatgggtgtgtttgtgtgtataatgtctaattgaatctgcagaaatgaccaagcaatcacttttttggagtatagttttataaaaaaagaatgcagggtttgaagttccttacctgataattgtgtctggcacatgataggggatcagtaaattgtaattcctaaccctactgtactcccaaacatggtgattcatggtcaagaaaaatcttatatatatatatatatacacacacacatatatgtgttcatatatatgtatacatatatatgtgtatatatacgtatgtatacatatatgtgtatatatacgtatgtatgtatacatatgtgtatatatagtatgtatgtatacatgtatgtgtatatatacgtatgtatgtatacatatatgtgtatacatatatatgtgtgtatatatatacacatatatacgtatatatgtgtatatatatacacagttgaatcagtgggattaatacctataatctctggttttcaaaggtaatatagaatatttgacacttggtaaaaggtgaactacctttgtagtgaatcttttcctcttggtagcatcaacactggggataaatcagaaccattctgtggaatgaaatgtttctcaagagcctataatatagtagatagtgcatattaagatgtctggctgggcatggtggctcatgcctgtaatcccagcactttgggaggctgaggcgggaggatcacttgagcctagaagttggagactaacctggcgagaccctgtctcaaaaaaaaaaaaaaatcaatttagctagcaggaatttgacatttaaagagggaatcttctctacctctacaaaatcaacccttaacacttttttcaccttcagaattatttagaatgtggatttactttgtctagttttttcctttatagtgtaatttattgttactctctatttactgactaccagagatatacaaaatactgtgcaaaagattgttactgttcaaagagcttacaaactaaatttaaaagaatagcaagtctgaaaaatagaagatagtcaaatatttgtttatgctaagaactgtttttaattttcagctttgatgtaaattgctagcttagttgtctttagttcaagcatgttaggaaatcctctttattcttaaatatagatacatgtctgcatatatgattgaattttagagccagaaagcatgtagagcagttgtgattagtagaaaatacactgacaagaagatatttgcatttatttcccaaagctgccagtaactagattttgtgacttaagtcatttaacctctccttgattagagcttcctgagccatgcacactggcactgcaaatcacagacaggcctagatacagatcccctcaccccttgctacatccaaaggtggcctgggtggctggagcctctgggccagaaccacctttgtccattttcctcagtgtgcctacagcatcgctttccatgtgtgccataacttgggaatagttgggatgtgttgcttaactcctttacaccattagttatctgtgagaccatctattccacactcttcattttttaaaaagagacaataattatttttaactcactgaagtttaaaactacctagcatttctgattaaaaaaaatttagaaggaaaattttaatgcatttatttcagatggcgttttaaatagatacaaccctttggaaacacaatatggtactacatagcaagggctgtaaaaatgaccatatcctttgccccataaattctacttctatacttttaaccttaaaaataattcagaaaaaagataaatgcatgaagacatttatgtctgcattctttataataacaaaaattggggaaaaaaactccatgtcaagaaagtgggataagaaaaatagtgaagtattatactgccattaaaataattatttggaagactgtagaaacgtggacatgtttgatatggtaagtaaaatgagcacaatacaaaatagtatgcatactatgattgtgactttgtaaaatctttatgcatgtggaaggtaatctgcaaaacaaattcattgtgttagtgtagcgggatatggaatgactttatttatttaaatcttttctttaatattactttgtattttcaataaaaataaatcactgta

SEQ ID NO: 18 - RNA, 3270 nt, Homo sapiens
  source 1..3270: mol_type = mRNA
ggggcgccgcagctagcgctggtctcggtggcagctcctccgcgccgcaggactcggctctacgggacatgtccgtgccgcgctcgccgcgcgcccgggcctgctagctcctctgtgctccctgaacgcgcggcgccgcacctggcagcggcctcggagctcggctcgggcaggagcgcgcggccgtgcgcaccgcgcagcgaccgctgccgtcatggggctgcagcccctggagttcagcgactgctacctcgacagcccgtggttccgggagaggatccgcgctcacgaagcggaactcgagaggaccaacaagttcatcaaagagctcattaaggacgggaagaacctcatcgctgcgacgaaaagtctgtcagtggcccagcggaagtttgctcattcactcagagactttaagtttgagtttatcggtgatgctgtgacagatgatgaacgatgcatagatgcttccttacgtgaattttcaaattttttgaagaatctggaggaacagagagaaattatggcattaagtgtaactgaaaccctgattaaacccttggaaaaattcagaaaagagcaacttggagctgtaaaggaagaaaaaaagaagtttgacaaagagacagaaaagaattatagtctaattgataaacatttgaatttatcagcaaaaaagaaagactcacatttacaagaggcagatatccaagtagagcagaaccggcaacacttctatgaactgtctctcgagtatgtgtgtaagctgcaggaaatccaagaaagaaagaagtttgagtttgtggaacctatgctgtcattttttcaggggatgtttaccttctatcatcagggccatgaacttgccaaagacttcaatcactacaaaatggaactacagatcaacattcagaatacacggaatcgatttgaaggaacaaggtcagaagtggaagagctcatgaacaaaatcagacagaatcccaaggaccacaaacgagcaagtcagtttacagccgaaggctacctgtatgtccaggaaaaaaggcctgctccgtttggttccagttgggtcaaacactattgcatgtatcgaaaagcagcaaagaagttcaacatgatcccatttgagcacagatctggagggaaacttggggacggagaggtgttctttttgaaagaatgtaccaagaggcatactgactccattgacagaaggttttgttttgacatagaagctgctgatcggcctggcgtttccttgaccatgcaggcattttccgaagaggaaaggaagcagtggttggaagctctgggtggaaaggaagctctgtcccatagttttaatacagccatcatcccaagaccagaaggaaatgcacagttggataagatggggttcacaattatcagaaaatgcatcagtgccgttgaaacacgaggtataaatgaccaaggattgtacagagttgtgggggtgagttcaaaggtccagagacttctgagtatgttgatggatgtaaaaacatgcaatgaggtggacctggagaattctgcagattgggaagtgaagacaataacaagtgccttgaaacagtatttgaggagtcttccagagcctctcatgacctatgagttacatggagatttcattgttccagccaaaagcggcagcccagaatctcgtgttaatgcgatccatttcttggtacacaaactgccagagaagaataaagagatgttggatattttggtgaaacacttaacaaatgtttcaaatcactccaagcagaacctgatgactgtggcaaacttaggagtggtgtttggaccaactctgatgaggccacaggaagaaactgtcgctgccctcatggacttgaagtttcagaatattgttgtggaaatcttaattgaaaaccatgaaaagatttttcggacgccgcccgatactacattccctgagcccacctgcctgtcagcatcacccccaaatgcgccaccaaggcagtcgaagagacaaggccagagaaccaagaggcccgtggccgtctacaatctttgtctggagctggaagatggtgacaatccttacccttccaaggaggacacccctaccagcagtctggactcactttcctccccgtctcccgtgactacagctgtccctgggcctcctggaccagacaaaaaccaccttctggcagatggagggagctttggagactgggcatccactatcccaggccagacccgatcgtctatggtccagtggcttaacccacagtctccaaccacaacaagctccaactcagctgtgacacctctttcacccgggtcgtcccctttccccttttctcctcctgctactgtagcggacaagccacctgaaagcatccgcagtcggaaggctcgagccgtgtatccgtgtgaagcagaacacagctcggaattatcttttgaaataggagcaatttttgaggatgtacaaacctccagggaacctggctggctagaagggactctgaacggcaagagggggctgattccacagaactacgtcaagctgctgtagctcctggcctcagagcccctgctgaccctggcacccagggacctgcctgggggcagagagctgtcttcctcctccgaggctctgggctgcacccacaggtacctccacacttgggagttaccatcatcacagtcagccctgggggtggggggtggtgggcagggatgggacgcaccacacagaactgtgattgtggatcaggaggggaatgtcaggattcgcaaaatggacttttcatttgtcaagtattgggacttgtgatttttaattatccagcatatagaatgagagggagggcagccttctgccacctgtgtcgcctccactggcagtcacgccaccagagccaccctggctccctctcctccctgagcacctgctgctgcgattttaaagggaactgtactactcgcagtgataggtttgcagagtgtgtgcttggctgtggcagcctagcttggagaagctgctgttggtgcaagggagatggtctcaagtcagagggaagcagagacgcgcgtctcaagcctgcccttcctagacggccacctgcaggaccccacactcactgcactggcagcgtgcactggcgtatttgtaacaggcttctcggtgctcctcacccgtgtgctgttttccaaacaccacctttttgcctcaaggtctctgtaaatgaaataaactgtaatttacta

SEQ ID NO: 19 - RNA, 3859 nt, Homo sapiens
  source 1..3859: mol_type = mRNA
ctcattggcgccgtgcagagaggcggaatgttcaactcctaactgcagcggaaacgtgggagccgcgcgggccgctgtcgtcccaacccccgccgccctcgtcgcgcgcggggcctccgcgcccccggctgctgctcacgccccgcccgggagccagattttgtggaagtataatactttgtcattatgagatgtcgtctctcggtgcctcctttgtgcaaattaaatttgatgacttgcagttttttgaaaactgcggtggaggaagttttgggagtgtttatcgagccaaatggatatcacaggacaaggaggtggctgtaaagaagctcctcaaaatagagaaagaggcagaaatactcagtgtcctcagtcacagaaacatcatccagttttatggagtaattcttgaacctcccaactatggcattgtcacagaatatgcttctctgggatcactctatgattacattaacagtaacagaagtgaggagatggatatggatcacattatgacctgggccactgatgtagccaaaggaatgcattatttacatatggaggctcctgtcaaggtgattcacagagacctcaagtcaagaaacgttgttatagctgctgatggagtattgaagatctgtgactttggtgcctctcggttccataaccatacaacacacatgtccttggttggaactttcccatggatggctccagaagttatccagagtctccctgtgtcagaaacttgtgacacatattcctatggtgtggttctctgggagatgctaacaagggaggtcccctttaaaggtttggaaggattacaagtagcttggcttgtagtggaaaaaaacgagagattaaccattccaagcagttgccccagaagttttgctgaactgttacatcagtgttgggaagctgatgccaagaaacggccatcattcaagcaaatcatttcaatcctggagtccatgtcaaatgacacgagccttcctgacaagtgtaactcattcctacacaacaaggcggagtggaggtgcgaaattgaggcaactcttgagaggctaaagaaactagagcgtgatctcagctttaaggagcaggagcttaaagaacgagaaagacgtttaaagatgtgggagcaaaagctgacagagcagtccaacaccccgctgctgccttcctttgagattggtgcatggacggaagacgatgtgtattgttgggttcagcagctcgtcagaaaaggtgactcttcagcagagatgagtgtatatgcaagcttgtttaaagaaaacaacattacagggaagcggctgctgctgctggaggaagaagacctgaaagacatgggcattgtctccaaggggcatatcattcacttcaagtcagccattgagaaattaacccatgattacataaatttgtttcacttcccaccactaattaaggactcaggaggtgaacctgaagaaaatgaggaaaaaatagtgaacctggaactggtttttggttttcacttgaaaccaggaactggcccacaggattgtaagtggaaaatgtatatggagatggatggggatgaaattgcaataacctacataaaagatgtgacattcaacactaacctacctgatgcggagattttaaagatgacaaagccaccatttgtaatggagaagtggattgtaggaatagcaaaaagtcagactgtggagtgcactgtcacatatgagagtgatgttagaactccaaaaagcactaaacatgtccattcgattcagtggagtagaacaaaacctcaggatgaagtgaaagcagtccaacttgccattcagacattattcaccaattcagatggcaaccctggaagcaggtccgactcaagtgctgattgccagtggttagatactctgaggatgcggcagattgcatccaacacttctttacagcgttcccagagcaatcctattctggggtcaccgttcttctcacactttgatggccaggattcctacgctgctgctgtgagacggccccaggtgcccattaagtatcaacagattacacctgtgaaccagtccagaagctcgtctcctactcagtatggactgaccaaaaacttctcttccctacatctcaactctagggacagtggcttttccagtggcaatactgacacctcttcagagaggggtcgatactcagacagaagcaggaacaaatatggacgtggtagtatatcactcaattcttctcctagaggaagatacagtggaaagagtcagcattccactccttcaagaggaagataccctggaaagttctacagggtttctcagtcagcactcaatcctcaccagtcgcctgacttcaagagaagccccagggacctccaccaacccaacaccataccagggatgcctttgcaccctgagactgactcaagagccagtgaagaggacagcaaagtcagcgaagggggctggacaaaagtggaataccggaaaaagccccacaggccatctcccgccaaaaccaataaagagagagccagaggggaccaccgtggatggagaaacttttgatgaattgaactacatagcttttctaagcaggttaaaaaaaaaaaaaaaaagaaatgtaatggtttttgataatatgatcccttcagattgaattaacgaaaagacaacacttccagtttttggattgggaaataccttctaattgagactatagccaaaccagggccaaaattatggatattggtcacccagtgatcataactaggcttgaaaatcactacacatattttctgccttgagtgaacatttttagaggaaaggttatgccatctttttaccctaaccactgatattctggttagcagggccaggacaaggggaaggaaaatgaggtcaacaaaaaaatcaaatttttaggaaaagataagatgaatgttactgatttttccttttggctgaggctgcaatatggcctggcaaggcactgttactgatcttgtctttaacattttgatattttgttcatcataatttttgcatttatttttttaaatattgcattaaaatatcatttagcttgattatcgagttttttggtttgaggttttttgttgcttcttttttcttttctttctttccccctcttttttttggatgtccccttaaattttgtgcccaaggcaggtacctcactcatctcatccttggctcagccctgctggttagtatttagtatttattttagtaagatatttgtgtctgtatgatggtcagagttgaactgatctggcttgtcatttttcagtaataaaaaaagttactgaatttaatgttgaatatgatgcatatctcattcattacgatttatcagaaaccaaagatttaaattgcctagatttgtggttctttctcttcctaagttcccagcgactgctttcaaatactattttctaaatttcaccaaaggagcaaagaggataaaacaacactccataaaggcctcttgggatgtcagaaatctaaaatctaaaagaaaacagacacagagcaagacaataacatcacaagctaaaagccagagaaatttaaaattaccaacatccttgttggagtaagacagtaaatatcagccttgcagcaagacagctctgagcagctgtgggcaaagaggtaaaccagtgggggtgcaaggagactgtctgcagcttagggcagaaatggtgggatccaacttgtgaaatgcttcatgttttacaaaccaaaaagtcaggtagcaacaaacttattgtatgtcaaatcaataaatgttactttcaatattctga

SEQ ID NO: 20 - RNA, 3731 nt, Homo sapiens
  source 1..3731: mol_type = mRNA
cttccctctagaatcctccaacatggagcctcttgcagcttacccgctaaaatgttccgggcccagagcaaaggtatttgcagttttgctgtctatagttctatgcacagtaacgctatttcttctacaactaaaattcctcaaacctaaaatcaacagcttttatgcctttgaagtgaaggatgcaaaaggaagaactgtttctctggaaaagtataaaggcaaagtttcactagttgtaaacgtggccagtgactgccaactcacagacagaaattacttagggctgaaggaactgcacaaagagtttggaccatcccacttcagcgtgttggcttttccctgcaatcagtttggagaatcggagccccgcccaagcaaggaagtagaatcttttgcaagaaaaaactacggagtaactttccccatcttccacaagattaagattctaggatctgaaggagaacctgcatttagatttcttgttgattcttcaaagaaggaaccaaggtggaatttttggaagtatcttgtcaaccctgagggtcaagttgtgaagttctggaagccagaggagcccattgaagtcatcaggcctgacatagcagctctggttagacaagtgatcataaaaaagaaagaggatctatgagaatgccattgcgtttctaatagaacagagaaatgtctccatgagggtttggtctcattttaaacattttttttttggagacagtgtctcactctgtcacccaggctggagtgcagtagtgcgttctcagctcattgcaacctctgcctttttaaacatgctattaaatgtggcaatgaaggatttttttttaatgttatcttgctattaagtggtaatgaatgttcccaggatgaggatgttacccaaagcaaaaatcaagagtagccaaagaatcaacatgaaatatattaactacttcctctgaccatactaaagaattcagaatacacagtgaccaatgtgcctcaatatcttattgttcaacttgacattttctaggactgtacttgatgaaaatgccaacacactagaccactctttggattcaagagcactgtgtatgactgaaatttctggaataactgtaaatggttatgttaatggaataaaacacaaatgttgaaaaatgtaaaatatatatacatagattcaaatccttatatatgtatgcttgttttgtgtacaggattttgttttttctttttaagtacaggttcctagtgttttactataactgtcactatgtatgtaactgacatatataaatagtcatttataaatgaccgtattataacatttgaaaaagtcttcatcattttcagtatttctctctgcattattttttagaagcaactcaaattctgtaatcataatattaccaagtaagtcagtctttatttttgcgtgaaaatcccaagtgtagaaaaaaggacatgagtataagatcatttaacttgattccttataggctgatttgggttgctaatgtattcgtactagattagccacttgggaggaattcaatgctgcatcattctgatagctgaaatagtaaaagtcaactccaaacagcctaaattctagtataaaaagggggtgatcatacaagtcctaaagtgtagatcagcagtcactgaacctcttagagtcacaaggcatttcttctcccaaagtcatgacctttatattttgttagccttataattgactaacaaagcaacctgccaagttggtgaaggttaattattgcctcatgaaatatacattcatcgcataaaagaattaaataggaagatggccaaaaatgtaaaaaagtcgtataaatttgtctaagaagaaaaagacccaatttaagtagtctgtgacttgactcccaaattctgacctgatggatgaaagtgaagatgtttcgtatggcaaattcagtaatgctacctcagtatatagttctgtatacgtatttggaccaaagttattagataaaccaaaaatatttcatgaagcatcttctgcttcagagtccatatccagccacccagctatgaatgtatttagaaagatatttggtggaggtggaatttctaccagaggtcaagaggatttgtagggatagcctcaagaatgccagatgagtgtgtcagaaagcctgctcctacctctcgccagctgcgtgactttaggcaagtcacttaagtaccttatttcagtttcctcacctgtaaattgaacaggggttgaatggaataaaaagccctttgcaactctaaaagtcaattaacacacttactaaggtgttttaagtgaccaggaaggaaatcagaactaacctggattgttagcgaagaaaacagaagccaccaacaagcctatctgtcctttgcaattttgctccaagagcctattagcaatttgaattctgagcctctaagaaaacttatgctcaggtggcccctccaagtgttggtgccagagcactcttgccttgtatcctcacctacgccttccatgaactcatagcagtgctgtggcactgcaggggtgttttatgcattcacgttaggagcatgagcagaactgcatatgccagcaccacatgggcagcagagactccccactgccagatggatgataatggagctgcactgggaacaaccaggactgtcccagtcaacatgatacagatgaacatcctgccttaagtcactagctctctccaaagccagataaagtgggtttcttcacttacatctctctaatcttggctgccttattcaacctacagactctatgtcagtgctggattttctccccttgccctttaggtaagcagagtaggcaggaggagatttgaaagcgtgtcatacatattgccttgaaagaaaggacattcaggtgtcccttcggggttctgtaacaattaggctatgtgtgctgagagagggagcggagtcatttgctgatgtgctgctacctgtaactcaaatgcctcataggaataccagcggacaaacacatagaggaaaagttgaatctttcctatattggacaatcttccttcagtcttgtttctgcatcaaaaagtctgggacacagagtgctacaggatgcctgggctaaggactgtaacagaaaaatatcaacatcagagcctggcacagtggctcacaccggtaatcccagcactttgggaggccgaggcgggtggatcacttcaggtcaggagttcgagaccatcctggccaacatggtgaaacccccatctctactaaaaatacaaaaattagccgggcacggtggcacatgcctgtaatcccagctacctgggaggctgagtcagaagaatcacttgaaaacaggaggctgaggttgcaatgagccaagattgcaccactgcactccaacctgggcaacagagcgagaccccatcttaaagaccctgtctcaaaaaagagagaaaaagaaaaagaaaaatatcaggcatcacatgaaagagtattcagctgtcgttcttgtgaaaaaggaaaaggacaaaatcaaatgcattttaactgtggtaactaattcactgacttgaagtttgctttgtttgttttctttggtgcgtagagaagaatacttcatactaactcctgatcatcttacagcagacataacaacagagtgttagagactggaataaatatgaatttggctgaaa

SEQ ID NO: 21 - RNA, 10311 nt, Homo sapiens
  source 1..10311: mol_type = mRNA
agatgctggcggagccggagcagccgcggactcagagagcccttctgccagcgccgcggggactctagcttcaggggctcttcacaggccctgggcgtgcctcagtgacgggacccagcaaagatgacgtggatctgtctgtcctgcatgctctggccagaggatctggaggcccccaagacacaccgcttcaaggtgaagaccttcaagaaggtgaagccctgtgggatctgccgccaggtcatcacccaggaaggctgcacctgcaaagtctgcagcttctcctgtcatcggaaatgccaggccaaggtggctgccccctgcgttcctccatccaaccatgagctggtgcccatcaccactgagaatgcaccaaagaatgtagtggacaagggagaaggagcctcccggggtggaaacacacggaaaagcctcgaggacaacggctccaccagggtcaccccgagtgtccagccccacctccagcccatcagaaacatgagtgtgagccggaccatggaggacagctgtgagctggacctggtgtacgtcacagagaggatcatcgctgtctccttccccagcacagccaatgaggagaacttccggagcaacctccgtgaggtggcgcagatgctcaagtccaaacatggaggcaactacctgctgttcaacctctctgagcggagacctgacatcacgaagctccatgccaaggtactggaatttggctggcccgacctccacaccccagccctggagaagatctgcagcatctgtaaggccatggacacatggctcaatgcagaccctcacaatgtcgttgttctacacaacaagggaaaccgaggcaggataggagttgtcatcgcggcttacatgcactacagcaacatttctgccagtgcggaccaggctctggaccggtttgcaatgaagcggttctatgaggataagattgtgcccattggccagccatcccaaagaaggtacgtgcattacttcagtggcctgctctccggctccatcaaaatgaacaacaagcccttgtttctgcaccacgtgatcatgcacggcatccccaactttgagtctaaaggaggatgtcggccatttctccgcatctaccaggccatgcaacctgtgtacacatctggcatctacaacatcccaggagacagccagactagcgtctgcatcaccatcgagccaggactgctcttgaagggagacatcttgctgaagtgctaccacaagaagttccgaagcccagcccgagacgtcatcttccgtgtgcagttccacacctgtgccatccatgacctgggggttgtctttgggaaggaggaccttgatgatgctttcaaagatgatcgatttccagagtatggcaaagtggagtttgtattttcttatgggccagagaaaattcaaggcatggagcacctggagaacgggccgagcgtgtctgtggactataacacctccgaccccctcatccgctgggactcctacgacaacttcagtgggcatcgagatgacggcatggaggaggtggtgggacacacgcaggggccactagatgggagcctgtatgctaaggtgaagaagaaagactccctgcacggcagcaccggggctgttaatgccacacgtcctacactgtcggccacccccaaccacgtggaacacacgctttctgtgagcagcgactcgggcaactccacagcctccaccaagaccgacaagaccgacgagcctgtccccggggcctccagtgccactgctgccttgagtccccaggagaagcgggagctggaccgcctgctgagtggctttggcttagagcgagagaagcaaggcgccatgtaccacacccagcacctcaggtcccgcccagcagggggctcggctgtgccctcctctggacgccacgttgtcccagcccaggttcatgtcaatggtggggcgttagcatctgagcgggagacagacatcctggacgatgaattgccaaaccaggatggtcacagtgcgggcagcatgggcacactctcttctctggacggggtcaccaacaccagtgaggggggctacccagaggccctgtccccactgaccaacggtctggacaagtcctaccccatggagcctatggtcaatggaggaggctacccctacgagtctgccagccgggcggggcctgcccatgctggccacacggcccccatgcggccctcctactctgcacaggagggtttagctggctaccagagggaggggccccacccagcctggccacagccagtgaccacctcccactatgcccatgaccccagcggtatgttccgctctcaatccttttcggaagctgaaccccagctgcccccagctccggtccgagggggaagcagccgggaggctgtgcaaaggggactgaattcgtggcagcagcagcagcagcagcagcagcagcctcgcccacctccacgccagcaggaaagagcccacttggagagtcttgtagccagcaggcccagccctcagccattggcagagacccccatccccagtctccctgagttcccgcgagcagcctcccagcaggagattgaacagtccatcgaaacactcaatatgctgatgctggacctggagccagcctccgctgctgccccactacacaagtcccagagtgtccccggggcctggccaggggcttctccactctcctcccagcccctctctggatcctcccgtcagtcccatccactgacccagtccagatctggctatatccccagtgggcattcgttgggaacccctgagccagccccacgggcctctctggagtctgtccctcctggcaggtcttactcaccttatgactatcagccatgtttggctgggcctaaccaggatttccattcaaagagcccagcctcttcctccttgcctgccttccttccgaccacccacagccctccagggcctcagcaacccccagcctctctccctggcctcactgctcagcctctgctctcaccaaaggaagcgacttcagacccctcccggactccagaggaggagccattgaatttagaagggctggtggcccacagggtagcaggggtacaggctcgggagaagcagcctgcagagcccccagcccctctgcggaggcgggcggccagtgatggacagtatgagaaccagtctccagaagccacatcccctcgtagccctggggttcgctcccctgtccagtgtgtctccccggagctggctcttaccatcgctctcaatcctggagggcggcccaaagagccccatttgcacagctacaaggaggccttcgaggagatggagggaacctccccgagcagcccaccacccagtggggtgcggtcccccccgggtctggccaagacacccctgtctgctctgggcctgaaacctcacaacccagcggacatcctgttgcaccccacaggagagccccggagctatgtggagtctgtggcacggacagcggtggctggaccccgagctcaggactctgagcccaagagctttagtgctccagccacccaggcctatggccatgagatacccctgaggaacgggaccctgggtggctcctttgtctcccccagccccctctccaccagcagccccatcctcagtgctgacagcacttcagtggggagtttcccgtcgggagagagcagtgaccagggtccccggacgcccacccagcctctgttggagtctggcttccgctcaggcagcctgggacagcccagcccgtctgcccagagaaactaccagagctcttctcctctcccgactgtgggcagtagctacagcagccccgactactcacttcagcatttcagctcctctccggaaagccaggctcgagctcagttcagtgtggctggcgtccacacggtgcctgggagccctcaggcgcgccacagaacagtgggcaccaacactccccctagtcctggcttcggctggcgggccatcaatcccagcatggctgcccccagcagtcccagtttgagccatcaccagatgatgggtccaccaggcactggcttccatggtagcactgtctccagcccccagagcagtgcagcgaccaccccggggagccccagcctgtgtcggcacccagcaggggtctaccaggtttctggcctccacaacaaagtggccaccaccccggggagtcccagcctgggccggcaccctggggctcaccaaggcaacctggcctccggtcttcatagcaatgcaatagccagccctggaagccccagcctgggccgtcacctcggagggtctggatctgtggttcccggcagcccctgcttggaccggcatgtggcctatggtggctattctaccccggaggatcggagacccacactgtcccggcagagcagtgcctctggctaccaggctccttccacgccctccttccctgtctcccctgcctactaccctggcctgagcagccctgccacctccccgtcaccagactccgcagccttccggcaagggagcccaacaccagccttgccagagaagcgaaggatgtcagtgggagaccgggcaggcagcctccccaactatgccaccatcaatgggaaggtgtcttcgcctgtcgccagcggcatgtccagtcccagtgggggcagcaccgtctccttctcccacactctgcccgacttctccaagtactccatgccagacaacagcccggagacgcgggctaaagtgaagtttgtccaggacacttctaagtattggtacaagcctgagatctccagggagcaggccatcgcgctcctcaaggaccaggagccgggggccttcatcatccgcgacagtcactccttccgaggcgcgtacgggctggccatgaaggtgtcttcgccacctccaaccatcatgcagcagaataaaaaaggagacatgacccatgagctggtcaggcattttctgatagagactggccccagaggagtcaagctcaagggctgccccaatgagccaaacttcggatcgctgtctgccctggtctaccagcactccatcatcccattggccctgccttgcaagctggtcattccaaaccgagaccccacagatgaatcgaaagatagctccggccctgccaactcaactgcagacctgctgaaacaaggggcagcctgcaatgtgctcttcgtcaactctgtggacatggagtcactcactgggccacaggccatctctaaagccacatctgagacgttggctgcagaccccacgccagctgccaccatcgttcacttcaaagtctctgcccagggaatcactctgactgacaaccagagaaagctctttttcagacgccactaccctctcaacactgtcaccttctgtgacctggatccacaggaaagaaagtggatgaaaacagagggtggtgcccctgctaagctcttcggcttcgtggcccggaagcagggcagcaccacggacaacgcctgccacctctttgctgagcttgaccccaaccagccggcctctgccatcgtcaacttcgtctccaaggtcatgctgaatgccggccaaaagagatgaaccctgccccttgcccagggccagtgccatggggaaggggcttgtggggaggggacccatgaatcctgaccactcttgaacccagaaggaggactttgggccaatttcggaggagagaagaaagtgcaacgtggggagagggaagtgaattgcagaggggagggggaaaagagagagagagagagagagagagagagagagaaagatggaggagaagaacttggattcccctgggtagatggaaactgcaaaaacccaaagcctccaaaactaaccaggtccacctaacaccccctccctcccctaagaagatggatgtcctcaaaagagaaggaacaaacctccttgggaatccacattttttgggggaatggaaaagctctgtctccctaactcaactgctttgcaaggggaaatcaagctgggagaatctttttctggccacctgtggggtaggttgtcaaaccaaacagagccaccgtgggacatcaagtggaagaacttgtttgcttgaaagtatctcagacccaaggcacctcaggtctctttgctgtgcctccactatattgtcgtgtgggtgtgtgtctgcacccacatcctcacacattgatctagatctgcctttatccactcgaattataaacagctcggcttgtccttgtcccatgtgtttgtagacacacatgcatactgtccaaagattagggttggtggtggcagtgcagcaggggagggacaaacaaccaagctatgggtgacagaggctctctcctggtgcctgcacctgcactctagtgaccctgggtgccgccagacccttctcttctacaaagaccccagcaggagtgggagggtctgcaatggcatcgccctgtcctgccttggccagaagcctggagctttggtttgaggaggtagagatatgtgtatccataggaagagatctgtcagaacaggcagctgttgagctcggggtgtcttccccaaggcatgtggctcagcagcaagaaaggcaagttgctcctgctggggccctggactctgccttagctcccacctctcagccttgttattgggtttcatgcccctggaccagccttatctcagacctgcttacctgcatgatgcctttttgggggctggggattgagtcttgctgctctgcccagccctgttctattctgcagggtccctgtgttggaattctccctggggaacctactttctgctcagtgaggctccggccagaaacctggagtccttatcctcccctctgtaagtgttttagggtctggcttttgcaggcaccctctgacctcagcagagctcctgggcctgctgcctgcacaccacatcgcctacctacaatgccaaagcctcactgtcaccctttctgccttggtttccctagctgagccacgctgcccatgcagcagagggcagaaggcttgcacttgggccaaagggcctaaggtccactggacagttgggaaaacacctgaccaccatttaaggactctaagccagaatggaaaattcaccaggactccattcttaagcctatgcgagtcccctagagagaggcattgtactgatatataaatattatataatatatacatgagacatactgacagaatctgtaagctaataaaatgtaagaaaaggttaaaaaaagaataggtaaattgacaagaagtatttattgtttttccatattgctttattgccttccttggggataaaccaattcctatccttttttatatgtgtaagtaaagcctgaagtgtagggggcctttgttcttgaagcagccagggtctccttgccctggccttggccttccctagactgtgtggggctcagcattgggaggggttgcacatgtcccagcctttggcccccttacttttcagcaagccaggggcccagcagtcagctcccaggatgtgtggggagctgtccctgactctgcaggcctgagcgagtgtgtgagcatgcggggacatgggtgtgtatggcacacataggtgcgtgtgtgtcttttgtattttttctcctccaaggagctgtgtcagtgtggacgttctgtttcagggagttggaaaggagggtgtctgcagaaggtggagagcaggggcagaggccccactggccaccccctgcttcccagagtgaaaccttgtgcctggtgaccaaagtccctccaaagtgctcttccttctgggttattcaagccaaatatctgggtttccccctctcctcattccctagcaaaccccaattatcttccaagataggagatatttcccatccccttcctttgtaaatatctcatctcccactggagagcccaggagcctattcctggcatggatgttctgtccacacttgaggctgggcggtgtatcagacccttcaagcagcctggctggggcccaggactgagtctggggtcagctttcacggtcgcttttcccttcctcaccacccaccacagcccaccttgcatgcatggccagcccctccactccagcctgagccatgtgtgcccctgcgggaggacccattcatgccagaaagctggtaactccctcccagcatccctgcggaaggagtcagtttctgagagtgtgacttttcaaggcgaatgatggggaagggttccccagtccccacagtggccccacctctgggccctgcaccagagcccttctgtgtcacggcgggctgtgcacccatgcacacacctacgcacacacaacactccgcactgcagtatattcttgccaaagatttcctttaaaagcaagcacttttactaattattattttgtaaatgtttatcttcttctgtcttctccctccctgaatctattttactgttgtttattgttgaatctgtgtgtcagccaggagagcgctgtctggccttgaacatgggctgggatgggaaagggtctgggagaagatgggcaacaaagagccagggagtcatggacatcgcagcgacgcagaccccagcaggttcagtcccgtgctgccaccagctgtccagctgggtgtctggagggaagagggcagaggagggtcatgtcccttcagctgggggaggggcccagtgagctccacgtggctttttcccaaagggagcaagagggaaggattgggcgagaaaacaatggagaggggacctgcgaaggaaaacagggaggaagtgagcggtttgatcagcctgctatcacggtgttctggctctcttatttagccaggcgcttaagggacagatacatcacatcctaagtttgggaaaggcctttgacccatgtcatctgagcgtctcctccagtagctctgaaagctgtggacaccaatggccaggattccttctcccctggtttttgaggatccctgggtcttctgagactggccaggagagggatggtggggccagtggttgtgtgaaagcaggaggggcagccctcctggacaagtgtgatccccctataaacggctctcaggaggttagtgagtaggagattctgccttgttctgatgagcctgtgcaggggctccaggggagcatgctgtccagggggcacagaagggtggtgagtgtgatcaaatctagtctcactcccactttttagtctcactcctacttttgtccaccacccctgcctcctggatcttctcccactttttttttcagctttaggacctggggagatcctgtgagtcaaggcagacacccaatcctgcccccacactcggggtcctccaagaggttggggggcagagtcccagagcagccctttaccccaggtccaggccctggaatcctgagactcgcgtttccttggccagtggtaacacaggacgtgtgtgcgcatgtgcaagtgtggatgtatgtgtgtgcgtgtgttttgctcatttctttagggaacttgggagtcggggttggaggtgctgggcaatggaacttcaaattcaatgtcgcccagcagtgaggggagtcgggaggtgaggcctgtaggccaaccaattggtggagtctcagcgatagcccaggtgagaagtggttcacccagaggggcagggtgggggcctcgggcagatctgtccctcttggcacctctgtcctcaaatgtccaaaatgttggaggacctctgttcatatcccacgcctgggctcttgccagcagtggagttactgtagagggatgtcccaagcttgttttccaatcagtgttaagctgtttgaaactctcctgtgtctgtgttttgtttgtgcgtgtgtgtgagagcacatcagtgtgtgcaggctgtgtttccccatttctctcctcccttcagacccatcattgagaacaaatgtaagaaatcccttcccaccaccctccctgcctcccaggccctctgcgggggaaacaagatcacccagcatccttccccaccccagctgtgtatttatatagatggaaatatactttatattttgtatcatcgtgcctatagccgctgccaccgtgtataaatcctggtgtatgctccttatcctggacatgaatgtattgtacactgacgcgtccccactcctgtacagctgctttgtttctttgcaatgcattgtatggctttataaatgataaagttaaagaaaactc

SEQ ID NO: 22 - RNA, 8053 nt, Homo sapiens
  source 1..8053: mol_type = mRNA
acttggtgttatttatttgggaagcgcccggacggcggagcttggcggcggcggtggtggtggctgccgcagactgtggttaaaaaaaagaaggcggcggcggcggcggcggcggaggcggaggcagctgcgaggcatgggagcgccgaagcgcccaggcgcaggccgaagctgccgcgctttctgggcacggcgggagtgctgagcagaaaggggagcgccgggggcccgcagccggctccggaggcgcgggccgggtttttgtttggctacgctgagcgccagtcagccccagcgaacaactccagttacgacaacaacccaccttccttccagacaagcgagacttgggctgctgcgtccgtcctattgtttagacacttgccaggggctccggagtcggcagagccaccgagtccccgctctgagtcgtcgccctccctctccccgacctcgctccctggagcgggaggccaggaaagcagcgggagaggggaaggggctagaaggagaaggactacccgggactgcggccgccgcgtcaggtgcagcgccaggagccgggcggcgtcgccacgccggcaggggtaccgccactgtggccttgggggacggaattcaaagcctgggaaaagttgctgcactttgagaaggacgaaccactagtgggagaccgccgggggccggccgtggctctgcgccctccggaacccggctcttgtttcttctacctttgccatcaggtgtctgccgcggagctgcggcttatctgggagacgagcggggttgacacgcgcgcacacactactgccattcagctgccgcctggctctgcctggagtagtggatcccacccgcccacctgccaccgagccattctccagtacgccccagcaggacgctgacacctccaaccttggcctttgcctttccactccttccggtctgcctggtttttaagtccgcccccagtcagtccccactcagtcttcgcagcagctctcatcctccacttggcctcttggagttcctcgccggagtgctgactagtggatatttctgcccggctgcggcggcccgactgcccttttgtcttttctgcgtgacctcggggcaggtcctggtgcagagcgtcgccaaggacgccgagcgggaggcgggattgcccagacatccttcagcgaagtgcatgtgtgtttgtaaaccatcgttggctgtcgggagaccgcgaggaccggtccaggctgcggcggagtcgagggcgagggagaggccgcgtgagtgagcagagtccagagccgtgcgcccccagaactgcgcgtccgccccgtgcacccccgcgcgccatgcccagttgccccgcgcgctctgctacgggcccgctgggcttccgcgccttctagcttccggagcccactttgatcggggccataatacctattgagatcccctcttctgtcttgtaccttcgccactggcatcggatttgcagaagcgtgcgtgggatcagaggaccgccctccccacaacaaccggcccctgcatcttagcagccgttggaagccccagctcttttaccgccaagttcatccttgggagacagaagacgcgtgatctcctctccgctgctcttggggtctccttgcagccctggccaggcggattcatcctcaggacctaaagttgcccaaggagctcctgctctgccagaggagggtggagagggcggtgggaggcgtgtgcctgagtgggctctactgccttgttccatattatttggtgcacattttccctggcactctgggttgctagccccgccgggcactgggcctcagacactgcgcggttccctcggagcagcaagctaaagaaagcccccagtgccggcgaggaaggaggcggcggggaaagatgcgcggcgttggctggcagatgctgtccctgtcgctggggttagtgctggcgatcctgaacaaggtggcaccgcaggcgtgcccggcgcagtgctcttgctcgggcagcacagtggactgtcacgggctggcgctgcgcagcgtgcccaggaatatcccccgcaacaccgagagactggatttaaatggaaataacatcacaagaattacgaagacagattttgctggtcttagacatctaagagttcttcagcttatggagaataagattagcaccattgaaagaggagcattccaggatcttaaagaactagagagactgcgtttaaacagaaatcaccttcagctgtttcctgagttgctgtttcttgggactgcgaagctatacaggcttgatctcagtgaaaaccaaattcaggcaatcccaaggaaagctttccgtggggcagttgacataaaaaatttgcaactggattacaaccagatcagctgtattgaagatggggcattcagggctctccgggacctggaagtgctcactctcaacaataacaacattactagactttctgtggcaagtttcaaccatatgcctaaacttaggacttttcgactgcattcaaacaacctgtattgtgactgccacctggcctggctctccgactggcttcgccaaaggcctcgggttggtctgtacactcagtgtatgggcccctcccacctgagaggccataatgtagccgaggttcaaaaacgagaatttgtctgcagtggtcaccagtcatttatggctccttcttgtagtgttttgcactgccctgccgcctgtacctgtagcaacaatatcgtagactgtcgtgggaaaggtctcactgagatccccacaaatcttccagagaccatcacagaaatacgtttggaacagaacacaatcaaagtcatccctcctggagctttctcaccatataaaaagcttagacgaattgacctgagcaataatcagatctctgaacttgcaccagatgctttccaaggactacgctctctgaattcacttgtcctctatggaaataaaatcacagaactccccaaaagtttatttgaaggactgttttccttacagctcctattattgaatgccaacaagataaactgccttcgggtagatgcttttcaggatctccacaacttgaaccttctctccctatatgacaacaagcttcagaccatcgccaaggggaccttttcacctcttcgggccattcaaactatgcatttggcccagaacccctttatttgtgactgccatctcaagtggctagcggattatctccataccaacccgattgagaccagtggtgcccgttgcaccagcccccgccgcctggcaaacaaaagaattggacagatcaaaagcaagaaattccgttgttcagctaaagaacagtatttcattccaggtacagaagattatcgatcaaaattaagtggagactgctttgcggatctggcttgccctgaaaagtgtcgctgtgaaggaaccacagtagattgctctaatcaaaagctcaacaaaatcccggagcacattccccagtacactgcagagttgcgtctcaataataatgaatttaccgtgttggaagccacaggaatctttaagaaacttcctcaattacgtaaaataaactttagcaacaataagatcacagatattgaggagggagcatttgaaggagcatctggtgtaaatgaaatacttcttacgagtaatcgtttggaaaatgtgcagcataagatgttcaagggattggaaagcctcaaaactttgatgttgagaagcaatcgaataacctgtgtggggaatgacagtttcataggactcagttctgtgcgtttgctttctttgtatgataatcaaattactacagttgcaccaggggcatttgatactctccattctttatctactctaaacctcttggccaatccttttaactgtaactgctacctggcttggttgggagagtggctgagaaagaagagaattgtcacgggaaatcctagatgtcaaaaaccatacttcctgaaagaaatacccatccaggatgtggccattcaggacttcacttgtgatgacggaaatgatgacaatagttgctccccactttctcgctgtcctactgaatgtacttgcttggatacagtcgtccgatgtagcaacaagggtttgaaggtcttgccgaaaggtattccaagagatgtcacagagttgtatctggatggaaaccaatttacactggttcccaaggaactctccaactacaaacatttaacacttatagacttaagtaacaacagaataagcacgctttctaatcagagcttcagcaacatgacccagctcctcaccttaattcttagttacaaccgtctgagatgtattcctcctcgcacctttgatggattaaagtctcttcgattactttctctacatggaaatgacatttctgttgtgcctgaaggtgctttcaatgatctttctgcattatcacatctagcaattggagccaaccctctttactgtgattgtaacatgcagtggttatccgactgggtgaagtcggaatataaggagcctggaattgctcgttgtgctggtcctggagaaatggcagataaacttttactcacaactccctccaaaaaatttacctgtcaaggtcctgtggatgtcaatattctagctaagtgtaacccctgcctatcaaatccgtgtaaaaatgatggcacatgtaatagtgatccagttgacttttaccgatgcacctgtccatatggtttcaaggggcaggactgtgatgtcccaattcatgcctgcatcagtaacccatgtaaacatggaggaacttgccacttaaaggaaggagaagaagatggattctggtgtatttgtgctgatggatttgaaggagaaaattgtgaagtcaacgttgatgattgtgaagataatgactgtgaaaataattctacatgtgtcgatggcattaataactacacatgcctttgcccacctgagtatacaggtgagttgtgtgaggagaagctggacttctgtgcccaggacctgaacccctgccagcacgattcaaagtgcatcctaactccaaagggattcaaatgtgactgcacaccagggtacgtaggtgaacactgcgacatcgattttgacgactgccaagacaacaagtgtaaaaacggagcccactgcacagatgcagtgaacggctatacgtgcatatgccccgaaggttacagtggcttgttctgtgagttttctccacccatggtcctccctcgtaccagcccctgtgataattttgattgtcagaatggagctcagtgtatcgtcagaataaatgagccaatatgtcagtgtttgcctggctatcagggagaaaagtgtgaaaaattggttagtgtgaattttataaacaaagagtcttatcttcagattccttcagccaaggttcggcctcagacgaacataacacttcagattgccacagatgaagacagcggaatcctcctgtataagggtgacaaagaccatatcgcggtagaactctatcgggggcgtgttcgtgccagctatgacaccggctctcatccagcttctgccatttacagtgtggagacaatcaatgatggaaacttccacattgtggaactacttgccttggatcagagtctctctttgtccgtggatggtgggaaccccaaaatcatcactaacttgtcaaagcagtccactctgaattttgactctccactctatgtaggaggcatgccagggaagagtaacgtggcatctctgcgccaggcccctgggcagaacggaaccagcttccacggctgcatccggaacctttacatcaacagtgagctgcaggacttccagaaggtgccgatgcaaacaggcattttgcctggctgtgagccatgccacaagaaggtgtgtgcccatggcacatgccagcccagcagccaggcaggcttcacctgcgagtgccaggaaggatggatggggcccctctgtgaccaacggaccaatgacccttgccttggaaataaatgcgtacatggcacctgcttgcccatcaatgcgttctcctacagctgtaagtgcttggagggccatggaggtgtcctctgtgatgaagaggaggatctgtttaacccatgccaggcgatcaagtgcaagcatgggaagtgcaggctttcaggtctggggcagccctactgtgaatgcagcagtggatacacgggggacagctgtgatcgagaaatctcttgtcgaggggaaaggataagagattattaccaaaagcagcagggctatgctgcttgccaaacaaccaagaaggtgtcccgattagagtgcagaggtgggtgtgcaggagggcagtgctgtggaccgctgaggagcaagcggcggaaatactctttcgaatgcactgacggctcctcctttgtggacgaggttgagaaagtggtgaagtgcggctgtacgaggtgtgtgtcctaaacacactcccggcagctctgtctttggaaaaggttgtatacttcttgaccgtgtgggactaatgaatgcttcatagtggaaatatttgaaatatattgtaaaatacagaacagacttatttttattatgagaataaagactttttttctgcatttggaaaaaaaaaaaaagaaatgcttgaactaaagcttcccctatgctggagaagtatgaagaaagatatacctggagacattagaacagcgatgggaaccattgcaactcgggtccatctttgtaacatgctgaagacaagcagaagcacatgcacgagggacagaggagctactgtgcactgctgtgaaattgcccagagcataaaacctgtgtaccctccttcacatcaaccaagttcactaggacataccaagcacatgcgtgtgaatgaggatgcaaggcaagagaatggaactccagaattcacagatagaacaaatggatgagaaatatttcatgcaaaatataaagtgtcctgaggatctgggttccatttacgagaggaaatgaaagtgctaaaataaattttatcttccttttaaatgtcagcatgtcagcagaagcagcacacaaaagtctttaccattttccagtattaatttttttgtaatataaatgataaaggagatgataaagaaccaatagattattgataaataaattagtaataatatgattttttgtttctatgagttctaaacagccctatacagtattcagtttccatgagaaatatttattgtatcaaagtacattgtacttaacattttaggccatccttttactgttccttgatgctttaatatatattaatttataattatcctgatatttttgtacatttttcaaacttaaaaatcaggatttttttttttttttttttggcaatagtactaacatagggttttatcttgggatacatatgtattggtctgtttgttgaccttgacatctgatcactgatgtcaatgacctactggcctcattcaggacacctgcagagagtatgcaaagtccgagagaggaaaacagaaatctgtatgtgagatggtcattgtacagaaagaagtggcccctctgcaacatgtcctcacagaaacgaaatggtgtgtagcaatcaacactagaaagtagaccttttgcaaattaatatgtccttgaccttttttgcccttttgtgggggtgaggtggggataaaaagactgtcatatcaagaactgtgacttttctttccctcaaacaataaaactcctttattatcttaatgctcccatgttaacatgtttgctgctaaattacaatgtagaattgataatggtttatagtgaactgtgctcttccctcattaaaatcccagggtgccctgtaaagatgcagatgtttcttcctgaaaacttctttttttacaaagaaaattagatgtacatgtataattcagtgtgctttgtctttctccagattaatatcggttacactgctgatgtttgtaaattaaacagatatttacttcattaa

SEQ ID NO: 23 - RNA, 1182 nt, Homo sapiens
  source 1..1182: mol_type = mRNA
gcggccgcaccccccggccgggccgtgcttctgcccctacaaggtttgggccgaggtgggggagggtcctggttgccggccccgcccggtccctccccgccttttaggcgcccgcgtggccgggacgtcccagtcccgctccgtcctcctcgcctgccaccggtgcacccagtccgctcacccagcccagtccgtccggtcctcaccgcctgccggccggcccaccccccaccgcagccatggacgccatcaagaagaagatgcagatgctgaagctggacaaggagaacgccatcgaccgcgccgagcaggccgaagccgacaagaagcaagctgaggaccgctgcaagcagctggaggaggagcagcaggccctccagaagaagctgaaggggacagaggatgaggtggaaaagtattctgaatccgtgaaggaggcccaggagaaactggagcaggccgagaagaaggccactgatgctgaggcagatgtggcctccctgaaccgccgcattcagctggttgaggaggagctggaccgggcccaggagcgcctggctacagccctgcagaagctggaggaggccgagaaggcggctgatgagagcgagagaggaatgaaggtcatcgaaaaccgggccatgaaggatgaggagaagatggaactgcaggagatgcagctgaaggaggccaagcacatcgctgaggattcagaccgcaaatatgaagaggtggccaggaagctggtgatcctggaaggagagctggagcgctcggaggagagggctgaggtggccgagagccgagccagacagctggaggaggaacttcgaaccatggaccaggccctcaagtccctgatggcctcagaggaggagtattccaccaaagaagataaatatgaagaggagatcaaactgttggaggagaagctgaaggaggctgagacccgagcagagtttgccgagaggtctgtggcaaagttggagaaaaccatcgatgacctagaagagaccttggccagtgccaaggaggagaacgtcgagattcaccagaccttggaccagaccctgctggaactcaacaacctgtgagggccagccccacccccagccaggctatggttgccaccccaacccaataaaactgatgttactagcctctcaaggccctttaatcctt

SEQ ID NO: 24 - RNA, 5011 nt, Homo sapiens
  source 1..5011: mol_type = mRNA
agtgtgtattcggctgcctgcctgcccgcctgcttgctctctggctgtgctcctgcttaaagaaatcagtccttcctttccgacttagtcctcgggaagaagtttcagactacaaggtatcattggaacatttcaagatcatcaaatcaaattccacagggattggtgaccaaccagaaggctcagacatctgattgctgacctgtccagacatcatctggtctccctgaacctgaaatcacaccatggatgattttgagcgtcgcagagaacttagaaggcaaaagagggaggagatgcgactcgaagcagaaagaatcgcctaccagaggaatgacgatgatgaagaggaggcagcccgggaacggcgccgccgagcccgacaggaacggctgcggcagaagcaggaggaagaatccttgggacaggtgaccgaccaggtggaggtgaatgcccagaacagtgtgcctgacgaggaggccaagacaaccaccacaaacactcaagtggaaggggatgatgaggccgcattcctggagcgcctggctcggcgtgaggaaagacgccaaaaacgccttcaggaggctctggagcggcagaaggagttcgacccaacaataacagatgcaagtctgtcgctcccaagcagaagaatgcaaaatgacacagcagaaaatgaaactaccgagaaggaagaaaaaagtgaaagtcgccaagaaagatacgagatagaggaaacagaaacagtcaccaagtcctaccagaagaatgattggagggatgctgaagaaaacaagaaagaagacaaggaaaaggaggaggaggaagaggagaagccaaagcgagggagcattggagaaaatcaggtagaggtgatggtggaagagaaaacaactgaaagccaggaggaaacagtggtaatgtcattaaaaaatgggcagatcagttcagaagagcctaaacaagaggaggagagggaacaaggttcagatgagatttcccatcatgaaaagatggaagaggaagacaaggaaagagctgaggcagagagggcaaggttggaagcagaagaaagagaaagaattaaagccgagcaagacaaaaagatagcagatgaacgagcaagaattgaagcagaagaaaaagcagctgcccaagaaagagaaaggagagaggcagaagagagggaaaggatgagggaggaagagaaaagggcagcagaggagaggcagaggataaaggaggaagagaaaagggcagcagaggagaggcagaggataaaggaggaagagaaaagggcagcagaggagaggcagaggataaaagaggaagagaaaagggcagcagaggagaggcaaagggccagggcagaggaggaagagaaggctaaggtagaagagcagaaacgtaacaagcagctagaagagaaaaaacatgccatgcaagagacaaagataaaaggggaaaaggtagaacagaaaatagaagggaaatgggtaaatgaaaagaaagcacaagaagataaacttcagacagctgtcctaaagaaacagggagaagagaagggaactaaagtgcaagctaaaagagaaaagctccaagaagacaagcctaccttcaaaaaagaagagatcaaagatgaaaagattaaaaaggacaaagaacccaaagaagaagttaagagcttcatggatcgaaagaagggatttacagaagttaagtcgcagaatggagaattcatgacccacaaacttaaacatactgagaatactttcagccgccctggagggagggccagcgtggacaccaaggaggctgagggcgccccccaggtggaagccggcaaaaggctggaggagcttcgtcgtcgtcgcggggagaccgagagcgaagagttcgagaagctcaaacagaagcagcaggaggcggctttggagctggaggaactcaagaaaaagagggaggagagaaggaaggtcctggaggaggaagagcagaggaggaagcaggaggaagccgatcgaaaactcagagaggaggaagagaagaggaggctaaaggaagagattgaaaggcgaagagcagaagctgctgagaaacgccagaagatgccagaagatggcttgtcagatgacaagaaaccattcaagtgtttcactcctaaaggttcatctctcaagatagaagagcgagcagaatttttgaataagtctgtgcagaaaagcagtggtgtcaaatcgacccatcaagcagcaatagtctccaagattgacagcagactggagcagtataccagtgcaattgagggaacaaaaagcgcaaaacctacaaagccggcagcctcggatcttcctgttcctgctgaaggtgtacgcaacatcaagagtatgtgggagaaagggaatgtgttttcatcccccactgcagcaggcacaccaaataaggaaactgctggcttgaaggtaggggtttctagccgcatcaatgaatggctaactaaaaccccagatggaaacaagtcacctgctcccaaaccttctgacttgagaccaggagacgtatccagcaagcggaacctctgggaaaagcaatctgtggataaggtcacttcccccactaaggtttgagacagttccagaaagaacccaagctcaagacgcaggacgagctcagttgtagagggctaattcgctctgttttgtatttatgttgatttactaaattgggttcattatcttttatttttcaatatcccagtaaacccatgtatattatcactatatttaataatcacagtctagagatgttcatggtaaaagtactgcctttgcacaggagcctgtttctaaagaaacccatgctgtgaaatagagacttttctactgatcatcataactctgtatctgagcagtgataccaaccacatctgaagtcaacagaagatccaagtttaaaattgcctgcggaatgtgtgcagtatctagaaaaatgaaccgtagtttttgtttttttaaatacagaagtcatgttgtttctgcactttataataaagcatggaagaaattatcttagtaggcaattgtaacactttttgaaagtaacccatttcagatttgaaatactgcaataatggttgtctttaaaaaaaaaaaagaaatgtactgttaaggtattactttttttcatgctgatgattcatatctaaattacattattatgttagctgacagtggtactgattttttaggttggttgttttgtggatttctttagtagtgatagtagcctgaaccacattttagataactcaattatgtatgtatgtgcatacacatatacaaacacactaatggtagaatgcttttttatgtgctagactattatatttagtagtatgtcattgtaactagccaatatcacagcttttgaaaaattaaaaaatcacactatattaatattttatatttgccaacagaaacatggcagataggtatcaatatgttttcaatgcctgatgacctataagaagaaagtattgaaaagaagagagattagaactgttagaaggagttgaaattttctaaaagacatagtatttagtttataattaaatgcattcttgaagtccagtgtgaattttattaatgctatcatctcgaccaagctcaaagcctacttattagaaacaatgaagttcacaataggtcataaggtctcttccttttctaaaattgaaagacaagaaatttagtgccaatattgtacagacagaaattccatgtatgagtctcaacaaagactacctttggctaaatgtctagaagcagagaagtaaagtgagcaaaatccagtgttgaggagtcatgacagtactttgatctttatatactctgaagcatttcttcaaacttttctacttttatttgtcattgatacctgtagtaagttgacaatgtggtgaaatttcaaaattatatgtaacttctactagttttactttctcccccaagtcttttttaactcatgatttttacacacacaatccagaacttattatatagcctctaagtctttattcttcacagtagataatgaaagagtcctccagtgtcttggcaaaatgttctagtatagctggatacatacagtggagttctataaactcatacctcagtggacttaaccaaaattgtgttagtctcaattcctaccacactgagggagcctcccaaataactattttcttatctgcagtattcctccagaagagctaaccagggcagggctggcatgagaagtgacatctgcgttacaaagtctatcttcctcataagtctgtaaagagcaattgaatcttctagctttagcaaacctaagccaaaggaaggaaagccatgaagaatgcagaagtcaaaccctcatgacaaagtaggcacaagtctacaataagctaaatcagaatttacaaatacaagtgtcccaggtagcattgactcccgtcattggagtgaaatggatcaaagtttgaattaaggcctatggtaaggtaacattgctttgttgtacttttgaacaagagctcctcctgatcactattacatatttttctagaaaatctaaagttcagaagagaatgtatcactgctgacttttattccaatatttggatggagtaagttttagggtagaattttgttcagtttggatttaatcttttgaaaagtaaattccttgtttactggtttgactataattctctgttatctttacgaggtaaaactgcaagctgactagcatgttctgtgaatctgccattcctaaaaattttataaacacttgatacttttcactgataatggatcgctccaataaacatatattgtgaaaatgcatccacaataaatggaattccttcctgcaaaatgtctttttctcacttatttttatgtacaatattgatagtgagaggtatgtctattataataaagattatggcacagtaaaacctgta

SEQ ID NO: 25 - RNA, 884 nt, Homo sapiens
  source 1..884: mol_type = mRNA
agtcctcagcggggcgcgtggcgagcggactcgactcggcaccgctgtgcaccatggcccgggccctgtgccgcctcccgcggcgcggcctctggctgctcctgggcaggatagcctgaggcacgcttgcttcactcccaggcagaatggccactgagaaatccggcccatcacctcttcatgaccactgcctgccaggaggctaactacggtgccctcctccgggagctctgcctcacccagttccaggtagacatggaggccgtcggggagacgctgtggtgtgactggggcaggaccatcaggagctacagggagctggccgactgcacctggcacatggcggagaagctgggctgcttctggcccaatgcagaggtggacaggttcttcctggcagtgcatggccgctacttcaggagctgccccatctcaggcagggccgtgcgggacccgcccggcagcatcctctaccccttcatcgtggtccccatcacggtgaccctgctggtgacggcactggtggtctggcagagcaagcgcactgagggcattgtgtaggcggggcccaggctgcccgcgggtgcacccaggctgcagggtgaggccaggcaggcctgggtaggggcagcttctggagccttgggacagagcaggcccacaatgccccccttcttccagccaagaagagctcacaggagtccagagtagccgaggctctggtattaacctggaagcccccctggctggaggccaccgccaccctaggaagggggcagggacgtgaccttgacttacctctggaaagggtcccagcctagactgcttaccccatagccacatttgtggatgagtggtttgtgattaaaagggatgttcttgaa

SEQ ID NO: 26 - RNA, 4260 nt, Homo sapiens
  source 1..4260: mol_type = mRNA
cgaggagcgagccagtgggggaggctgacatcaccacggcggcagccctttaaacccctcacccagccagcgccccatcctgtctgtccgaacccagacacaagtcttcactccttcctgcgagccctgaggaagccttgtgagtgcattggctggggcttggagggaagttgggctggagctggacaggagcagtgggtgcatttcaggcaggctctcctgaggtcccaggcgccagctccagctccctggctagggaaacccaccctctcagtcagcatgggggcccaagctccaggcagggtgggctggatcactagcgtcctggatctctctcagactgggcagccccgggctcattgaaatgccccggatgacttggctagtgcagaggaattgatggaaaccaccggggtgagagggaggctccccatctcagccagccacatccacaaggtgtgtgtaagggtgcaggcgccggccggttaggccaaggctctactgtctgttgcccctccaggagaacttccaaggagctttccccagacatggccaacaagggtccttcctatggcatgagccgcgaagtgcagtccaaaatcgagaagaagtatgacgaggagctggaggagcggctggtggagtggatcatagtgcagtgtggccctgatgtgggccgcccagaccgtgggcgcttgggcttccaggtctggctgaagaatggcgtgattctgagcaagctggtgaacagcctgtaccctgatggctccaagccggtgaaggtgcccgagaacccaccctccatggtcttcaagcagatggagcaggtggctcagttcctgaaggcggctgaggactatggggtcatcaagactgacatgttccagactgttgacctctttgaaggcaaagacatggcagcagtgcagaggaccctgatggctttgggcagcttggcagtgaccaagaatgatgggcactaccgtggagatcccaactggtttatgaagaaagcgcaggagcataagagggaattcacagagagccagctgcaggagggaaagcatgtcattggccttcagatgggcagcaacagaggggcctcccaggccggcatgacaggctacggacgacctcggcagatcatcagttagagcggagagggctagccctgagcccggccctcccccagctccttggctgcagccatcccgcttagcctgcctcacccacacccgtgtggtaccttcagccctggccaagctttgaggctctgtcactgagcaatggtaactgcacctgggcagctcctccctgtgcccccagcctcagcccaacttcttacccgaaagcatcactgccttggcccctccctcccggctgcccccatcacctctactgtctcctccctgggctaagcaggggagaagcgggctgggggtagcctggatgtgggccaagtccactgtcctccttggcggcaaaagcccattgaagaagaaccagcccagcctgccccctatcttgtcctggaatatttttggggttggaactcaaaaaaaaaaaaaaaaaatcaatcttttctcaggcctggctggcagagtttgatttgccctggtcacttttgttatggtttcagatctgcgcaggggacaggcaggcatctcgggcttgtatgtgttcctggctgccgtcctctgaaggacccttcatgtgccaagattccaggacagtcagattctttcagaggaaacaggccatagaacaggagagtgaatcttggggaccgaagggaaaaaggagccactcagcagcatgcagtggctttggggagacagaggaaaggagagattgcgagtggcagaattgtttggaaggtttttattttggaaaagctgtgcagaaaaaaattcaagaaaatgttgctgtgaaaagagaaaaacaaatcttaagcattaaaaaaaattcaaccaactagctcagaagaggggagaaggccaaggttgagagaagagtcacagcctgtcaggcagatagctggcctccggcgggaaggccatttccctgagcacttgcagaggaagacagggtggtggcaggactggagtggcagtggctcccaaggctctctcctccaacatgtgcatctgccatctgctctgcagtcctgccgcaggattccctagtgaagcagctcaggcctgggggagccgtgtgtatcccagctgtgccggcagcatcataccaatcgtgggggtggtgaaggagccaggggttcattcatggttggtttctgatcaggcatcttgggaatggataatggaggcagccgctttcaggacaggcatgtccaggggctcctcccagcctctaccccgaagtcctcttcccaagtgaccccagtgatgtttccattgagatgcgctcctggctatggcaggcaccttctcaacttatatgtgggaaggggtcccccatgcttgggggacctaggcagctggcttggcccaagagagatgaggatggaggccaaaccaaaggggggcgccaatcccctgtccaacaccttctcaccaaaagctcccgtttggctggaggcagaccctgtggctctgaccagacttctctggcagcaatcctccaccatttgtatcttaagaaggccctcaccctctttgagtggagtcagaggatgcctcagattccagatgtaagcatcagaactgctttctgtcaagagctccctaattttgggaaagaagagcctgtcccacactgtcaggccctgaggtcagcagatctgctcctccttcccgtgcggtacgtctaggtgctgatgagggcagtccagggcgctcttgttctgggacaggctccagtccccttgctccagcaggtctggggcaaggaggtcagaggtggtgggagggcccctgctctctgtttccacttcgtctggatccttgctgctgcaaagtggcactgattctagctctgtcccttcctccttggctttccggctccgatggggccagtggcagggtccactcctacaaacttgattggaagccacattcctctggctcaaatatacttccagcatgtagtaaacagtccagaagacggtgaaacagcctaccagcaccagggtctggggccgaggcaagcacctacgtgaggcactgtttcccgaagcctacagcctttctcagcccaggacaatgagctcagaaagtctttttccttctagggactgcctttttcacccaaactgttccctctgccccctcccccgacaaggcctgtcctgtaagagttaggctagcagggtaggagcaatgctatgaaaccactgctgggacccaggtcttcccagtccttcaccccgcaggtcaccctgagaaacacactaagaactccatcccccagacaggacagtcccatctacccgcagcttgagtcttggccctagtaccttgagggtgttgggggtgatggtgtaaccatcttcctcaggaattttcagccccggtgggcagggcagggcgaagtcatcgtgcaggtattttccactcatggcactctctaacagcctgtggagaagaaaagaggtgaggatgccccactgactatggttcctataccatctgccctcacccattttcctgccttacaggtgaagacagggaagccccacagcaaaaaggagaggcccagactgtgagttcccagcccggggctccatctaccggcttgacgctggaactgggaagcacagctggggttcagagggcgatgggctccctaggcggcccttcccctgtgactggccttccctctgacacatgcggctttacccacctttgtctgtccctgatgtctactgcactccacacagagccatatagggtcagctgccattgccggaggatgccgacctggaatgactcatcccctagggcagcaaggggcagctcgtgagccacgcccctctgtcagccatgccagacagcagaggccctgcccgccctgccacccaaaggggctcaggccacatggtctgctccaggagctgcctcactgtgtcccactgaccccaggttctgcagaagggcctcactgggtgcccttagggatggaaagggttgaaaggctgtactccaaagcagagtcttgcttttctctcccgtattttgggggttcagctgggattagaaaaaaatgtctttccaccaaattaaagaaagctttgaaaaccac

SEQ ID NO: 27 - RNA, 2786 nt, Homo sapiens
  source 1..2786: mol_type = mRNA
agttccacgcacccagcgagcccaagcgccttctccgcaccagggaagccccacccaccagaagccaagatgtccagcaagcgggccaaagccaagaccaccaagaagcggccacagcgggccacatccaatgtcttcgcaatgtttgaccagtcccagatccaggagtttaaggaggctttcaacatgattgaccagaaccgtgatggcttcattgacaaggaggacctgcacgacatgctggcctcgctggggaagaaccccacagacgaatacctggagggcatgatgagcgaggccccggggcccatcaacttcaccatgttcctcaccatgtttggggagaagctgaacggcacggaccccgaggatgtgattcgcaacgcctttgcctgcttcgacgaggaagcctcaggtttcatccatgaggaccacctccgggagctgctcaccaccatgggtgaccgcttcacagatgaggaagtggacgagatgtaccgggaggcacccattgataagaaaggcaacttcaactacgtggagttcacccgcatcctcaaacatggcgccaaggataaagacgactaggccaccccagccccctgacaccccagcccccgccagtcacccctccccgcacacacccgtccataccagctccctgcccatgaccctcgctcagggatccccctttgaggggttagggtcccagttcccagtggaagaaacaggccaggagaagtgcgtgccgagctgaggcagatgttcccacagtgaccccagagccctgggctatagtctctgacccctccaaggaaagaccaccttctggggacatgggctggagggcaggacctagaggcaccaagggaaggccccattccggggctgttccccgaggaggaagggaaggggctctgtgtgccccccaggaggaagaggccctgagtcctgggatcagacaccccttcacgtgtatccccacacaaatgcaagctcaccaaggtcccctctcagtccccttccctacaccctgaccggccactgccgcacacccacccagagcacgccacccgccatgggagtgtgctcaggagtcgcgggcagcgtggacatctgtcccagagggggcagaatctccaatagaggactgagcactgcttctggtctgtgtgtctgtggctggggtgaagtaaggggaccccgggcctgaaaccctctcccaccttctcctgccatctccagttactgccctgctcctcccaccctggcccagggaaggactgggtgtcctccggccatatggtccctgaagcctctagggaccagagtccctagtaagtgggctctgtgctcagctgagaccagcaggggacaggggacggagggaatgggcctcatggccttctcagggcttgtgggaaagggaggaccatgggaatcaccacagccaatcccgtggagggttccaggcctcttggggggcagaggtcaggccacacagccctcaggactaaagctccgggttccagaagaacagggaggctccaacagtgatgaggcaggcgtcccagcagctcagggttggaggtgggaatgaggggtttcccagccccaggcaggtggagggcgagttcagccccaggaccaacagcatgggggccacagctttccatgtccctgtgtacgcagggcaggcagggccgggacccctgctactggtggatgatggggacactgatggcagtgcctggggcctaagaggggcagaaagagcgctgaatgactgagcagagagtccagaggggcatggactgcctgggtcacccaataggcctagggaagagtgagggccggacccaccccacctgaccccagcgagtggacccagcttggtcctgaggccttctccagaggtcacccagcgcaggcagccgcagcactcagcaaaggtcccagatcagggccaagggggagctgagcaccaggggaccctgtgcctgaccaggaggccctaacctcctgcaggcctcaacgccaggccctgctcagagctcggctgaaactcctcatcctggctccaaacagaggcccaaaagtccctggtatcaactccagaaggggcgagacccgaacaagttccaaaccaggcccaaatagtatcccaaactcagtcccaaacacattctcacccccggcagcaggctgcaggcctccagctacacacacggccctgggcaactctcagtctggccacccattcgatgctgccagccccaagggtgtgggaggggggtctcagagtgtcccagggtactggccacacatgcccgacaccagggtcataaggtcctctcagcagagccactgcagcaccaaaggcatttctggaaggaggcaaggacgcgtcatctagatgtcaagccccagcgtgcgattctgtcacagttcaccccaccttcaccccgagacggaagacggaagagcttcgcacacaggcgggaagaggtcaggaccagtccagcctcactggcttcagaactggcctgggggctaccttgacccacaggaagggaagaggaacgtgctctgggcagggcaaggcaggacctgcagcacccacagaccagcagtaaaggacccccggaactttccaagtctagcacaaaacccagaagccacaaaggaaaatactggcagatttaaatgcatgaagtcaacattctttttgtagagctaaagaaaccataagcaaaattaaaagccaaatgcattctgggaggaaa

SEQ ID NO: 28 - RNA, 10548 nt, Homo sapiens
  source 1..10548: mol_type = mRNA
ggaagctgccggactaacactccgcgggtgtttccatggagaccgaggccgagcctgcgcggcctcacggcgttgccatggagacaactccggggctggggctccgaagtcccggcgcaccgctggctcagaaccccgcggagctgctgtgcgaggccggagccgcggtggcggctgcacgctgggacctgcagaagcactctttgctaattgtgatcggcgatatcggtacagagagtcagctgagggccgtgcgggcccaccttgaacaagggattctctcctggaacattgacctgtcatcctttgacttgaaccaacagttgagactcttcattacccggcacctagctcacttctcctcagaggtcaaaggccagaggaccctttgccaccagagtgagatcctagagaccatcatcctggtaaatcccagtgcagacagcatcagctctgaggttcatcatcttcttagcagctcatcagcttataaactactaatcttgagtgggcaaagtttagagcctgggggagacctcatcctacagagtggcacctactcatatgaaaactttgcccaggtccttcacaaccccgagatttcccaattgctcagcaatagagaccctgggatacaggccttccttaccgtgtcctgcttaggggaaggtgattggagccacctgggattatccagttcccaagagaccctgcacctccggctaaaccctgagcccactctgcccaccatggacggcgtggctgagttctccgagtatgtctctgagactgtggacgtgccatccccatttgacctactagagccccccacctcagggggcttcctcaagctctccaagccttgttgctacatcttcccaggtggtcgtggggactctgccctctttgctgtcaatggtttcaacatcctggtggatggtggctctgatcgcaagtcctgtttttggaagctggtacggcacttggaccgcattgactcggtgctactcacacacattggggcagacaacctgccaggcatcaatggactactgcagcgcaaagtggcagagctagaggaggagcagtcccagggctctagcagttacagcgactgggtgaagaaccttatctctcctgagcttggagttgtctttttcaacgtgcctgagaagctgcggcttcctgatgcctcccggaaagccaagcgtagcattgaggaggcctgcctcactctgcagcacttaaaccgcctgggcatccaggctgagcctctatatcgtgtggtcagcaataccattgagccactgaccctcttccacaaaatgggtgtgggccggctggacatgtatgtcctcaaccctgtcaaggacagcaaggagatgcagttcctcatgcaaaagtgggcaggcaatagtaaagccaagacaggcatcgtgctgcccaatgggaaggaggctgagatctccgtgccctaccttacctctatcactgctctggtggtctggctaccagccaatcccactgagaagattgtgcgtgtgctttttccaggaaatgctccccaaaacaagatcttggagggcctagaaaagcttcggcatctggacttcctgcgttaccctgtggccacgcagaaggacctggcttctggggctgtgcctaccaacctcaagcccagcaaaatcaaacagcgggctgatagcaaggagagcctcaaagccactaccaagacggccgtgagcaagttggccaaacgggaggaggtggtagaagagggagccaaggaggcacgttcagagctggccaaggagttagccaagacagagaagaaggcaaaagagtcatctgagaagcccccagagaagcctgccaagcctgagagggtgaagacagagtcaagtgaggcactgaaggcagagaagcgaaagctgatcaaagacaaggtagggaaaaagcaccttaaagaaaagatatcaaagctggaagaaaaaaaagacaaggagaaaaaagagatcaaaaaggagaggaaagagctcaagaaggatgaaggaaggaaggaggagaagaaggatgccaagaaggaggagaagaggaaagataccaaacctgagctcaagaagatttccaagccagacctaaagccctttactcctgaggtacgtaagaccctctataaagccaaggtccctggaagagtcaaaatagacaggagccgtgctatccgtggggagaaggagctgtcttctgagccccagacacccccagcccagaagggaactgtaccactcccaaccatcagtgggcacagggagctggtcctatcctcaccagaggacctcacacaggactttgaggagatgaagcgtgaggagagggctttgctggctgaacaaagggacacaggactaggagataagccattccctctagacactgcagaggagggacccccaagtacagctatccagggaacaccaccctctgttccagggctgggacaagaagaacatgtgatgaaggagaaagagcttgtcccagaggtccctgaggaacaaggcagcaaggacagaggcctagactctggggctgaaacagaggaagagaaagatacctgggaggaaaagaagcagagggaagcagagaggctcccagacagaacagaagccagagaggaaagtgaacctgaagtaaaggaggatgtgatagaaaaggctgagttagaagaaatggaggaggtacacccttcagatgaggaggaagaggacgcgacaaaagctgagggtttttaccaaaaacatatgcaggaacccttgaaggtaactccaaggagccgggaggcttttgggggtcgggaattgggactccagggcaaggcccctgagaaggagacctcgttattcctaagcagcctgaccacacctgcaggagccactgagcatgtctcttacatccaggatgagacaatccctggctactcagagactgagcagaccatctcagatgaggagatccatgatgagccggaggagcgcccagctccacccagatttcatacaagtacatatgacctgcccgggcctgaaggtgctggcccattcgaagccagccaacctgccgatagtgctgttcctgctacctctggcaaagtctatggaacgccagagactgaactcacctaccccactaacatagtggctgcccctttggctgaagaggaacatgtgtcctcggccacttcaatcactgagtgtgacaaactttcttcctttgccacatcagtggctgaggaccaatctgtggcctcacttacagctccccagacagaggagacaggcaagagctccctgctgcttgacacagtcacaagcatcccttcctcccgtactgaagctacgcagggcttggactatgtgccatcagctggtaccatctcacccacctcctcactggaagaagacaagggcttcaaatcaccaccctgtgaggacttctctgtgactggggagtcagagaagagaggagagatcatagggaaaggcttgtctggagagagagctgtggaagaggaagaggaggagacagcaaacgtagagatgtctgagaaactttgcagtcaatatggaactccagtgtttagtgcccctgggcatgccctacatccaggagaaccagcccttggagaagcagaggagcggtgccttagcccagatgacagcacagtgaagatggcttctcctccaccatctggcccacccagtgccacccacacaccctttcatcagtccccagtggaagaaaagtctgagccccaagactttcaggaggcagactcctggggagacactaagcgcacaccaggtgtgggcaaagaagatgctgctgaggagacagtcaagccagggcctgaagagggcacactagagaaggaagagaaagttcctcctcccaggagcccccaggcccaggaagcacctgtcaacattgatgaggggcttacaggctgtaccattcaactgttgccagcacaggataaagcaatagtctttgagattatggaggcaggagagcccacaggcccaattctgggagcagaagcccttcccggaggtttgaggactttaccccaagaacctggcaaacctcagaaagatgaggtgctcagatatcctgaccgaagcctctctcctgaagatgcagaatccctctctgtcctcagcgtgccctccccagacactgccaaccaagagcctacccccaagtctccctgtggcctgacagaacagtacctacacaaagaccgttggccagaggtatctccagaagacacccagtcactttctctgtcagaagagagtcccagcaaggagacctccctggatgtctcttctaagcagctctctccagaaagccttggcaccctccagtttggggaactaaaccttgggaaggaagaaatggggcatctgatgcaggccgaggatacctctcaccacacagctcccatgtctgttccagagccccatgcagccacagcgtcacctcccacagatgggacaactcgatactctgcacagacagacatcacagatgacagccttgacaggaagtcacctgccagctcattctctcactctacaccttcaggaaatgggaagtacttacctggggcgatcacaagccctgatgaacacattctgacacctgatagctccttctccaagagtcctgagtctttgccaggccctgccttggaggacattgccataaagtgggaagataaagttccagggttgaaagacagaacctcagaacagaagaaggaacctgagccaaaggatgaagttttacagcagaaagacaaaactctggagcacaaggaggtggtagagccgaaggatacagccatctatcagaaagatgaggctctgcatgtaaagaatgaggctgtgaaacagcaggataaggctttagaacaaaagggcagagacttagagcaaaaagacacagccctagaacagaaggacaaggccctggaaccaaaagacaaagacttagaagaaaaagacaaggccctggaacagaaggataagattccagaagagaaagacaaagccttagaacaaaaggatacagccctggaacagaaggacaaggccctggaaccaaaagataaagacttggaacaaaaggacagggtcctagaacagaaggagaagatcccagaagagaaagacaaagccttagatcaaaaagtcagaagtgttgaacataaggctccggaggacacggtcgctgaaatgaaggacagagacctagaacagacagacaaagcccctgaacagaaacaccaggcccaggaacaaaaggataaagtctcagaaaagaaggatcaggccttagaacaaaaatactgggctttgggacagaaggatgaagccctggaacaaaacattcaggctctggaagagaaccaccaaactcaggagcaggagagcctagtgcaggaggataaaaccaggaaaccaaagatgctagaggaaaaatccccagaaaaggtcaaggccatggaagagaagttagaagctcttctggagaagaccaaagctctgggcctggaagagagcctagtgcaggagggcagggccagagagcaggaagaaaagtactggagggggcaggatgtggtccaggagtggcaagaaacatctcctaccagagaggagccggctggagaacagaaagagcttgccccggcatgggaggacacatctcctgagcaggacaataggtattggaggggcagagaggatgtggccttggaacaggacacatactggagggagctaagctgtgagcggaaggtctggttccctcacgagctggatggccagggggcccgcccacactacactgaggaacgggaaagcactttcctagatgagggcccagatgatgagcaagaagtacccctgcgggaacacgcaacccggagcccctgggcctcagacttcaaggatttccaggaatcctcaccacagaaggggctagaggtggagcgctggcttgctgaatcaccagttgggttgccaccagaggaagaggacaaactgacccgctctccctttgagatcatctcccctccagcttccccacctgagatggttggacaaagggttccttcagccccaggacaagagagtcctatcccagaccctaagctcatgccacacatgaagaatgaacccactactccctcatggctggctgacatcccaccctgggtgcccaaggacagacccctcccccctgcacccctctccccagctcctggtccccccacacctgccccggaatcccatactcctgcacccttctcttggggcacagccgagtatgacagtgtggtggctgcagtgcaggagggggcagctgagttggaaggtgggccatactcccccctggggaaggactaccgcaaggctgaaggggaaagggaagaagaaggtagggctgaggctcctgacaaaagctcacacagctcaaaggtaccagaggccagcaaaagccatgccaccacggagcctgagcagactgagccggagcagagagagcccacaccctatcctgatgagagaagctttcagtatgcagacatctatgagcagatgatgcttactgggcttggccctgcatgccccactagagagcctccacttggagcagctggggattggcccccatgcctctcaaccaaggaggcagctgccggccgaaacacatctgcagagaaggagctttcatctcctatctcacccaagagcctccagtctgacactccaaccttcagctatgcagccctggcaggacccactgtacccccaaggccagagccagggccaagtatggagcccagcctcaccccacctgcagttcccccccgtgctcctatcctgagcaaaggcccaagcccccctcttaatggtaacatcctgagctgcagcccagataggaggtccccatcccccaaggaatcaggccggagtcactgggatgacagcactagtgactcagaactggagaagggggctcgggaacagccagaaaaagaggcccaatccccaagtcctcctcaccccattcctatggggtcccccacattatggccagaaactgaggcacatgttagccctcccttggactcacacctggggcctgcccgacccagtctggacttccctgcttcagcctttggcttctcctcattgcagccagctcccccacagctgccctctccagctgaaccccgctcggcaccctgtggctcccttgccttctctggggatcgagctctggctctggctccaggaccccccaccagaacccggcatgatgaatacctggaagtgaccaaggcccccagcctggattcctcactgccccagctcccatcacccagttctcctggggcccctctcctctccaatctgccacgacctgcctcaccagccctgtctgagggctcctcctctgaggctaccacgcctgtgatttcaagtgtggcggagcgcttctctccaagccttgaggctgcagaacaggagtctggagagctggacccaggaatggaaccagctgcccacagcctctgggacctcactcctctgagcccagcacccccagcttcactggacttggccctagctccagctccaagcctgcctggagacatgggtgatggcatcctgccgtgccacctggagtgctcagaggcagccacggagaagccaagccccttccaggttccctctgaggattgtgcagccaatggcccaactgaaaccagccctaaccccccaggccctgccccagccaaggctgaaaatgaagaggctgcggcttgccctgcctgggaacgtggggcctggcctgaaggagctgagaggagctcccggcctgacacattgctctcccctgagcagccagtgtgtcctgcagggggctccgggggcccacccagcagtgcctctcctgaggtcgaagctgggccccagggatgtgccactgagcctcggccccatcgtggggagctctccccatccttcctgaacccacctctgcccccatccatagatgatagggacctctcaactgaggaagttcggctagtaggaagaggggggcggcgccgggtaggggggccagggaccactgggggcccatgccctgtgactgatgagacaccccctacatcagccagtgactcaggctcctcacagtcagattctgatgtcccgccagaaactgaggagtgtccgtccatcacagctgaggcagccctcgactcagatgaagatggagacttcctacctgtggacaaagctgggggtgtcagtggtactcaccaccccaggcctggccatgacccacctcctctcccacagccagacccccgcccatcccctccccgccctgatgtgtgcatggctgaccccgaggggctcagctcagagtctgggagagtagagaggctacgggagaaggaaaaggttcaggggcgagtagggcgcagggccccaggcaaggccaagccagcgtcccctgcacggcgtctggatcttcggggaaaacgctcacccacccctggtaaagggcctgcagatcgagcatcccgggccccacctcgaccacgcagcaccacaagccaggtcaccccagcagaggaaaaggatggacacagccccatgtccaaaggcctagtcaatggactcaaggcaggaccaatggccttgagttccaagggcagctctggtgcccctgtatatgtggatctcgcctacatcccgaatcattgcagtggcaagactgctgaccttgacttcttccgtcgagtgcgtgcatcctactatgtggtcagtgggaatgaccctgccaatggcgagccaagccgggctgtgctggatgccctgctggagggcaaggcccagtggggggagaatcttcaggtgactctgatccctactcatgacacggaggtgactcgtgagtggtaccaacaaactcatgagcagcagcaacaactgaatgtcctggtcctggctagcagcagcaccgtggtgatgcaggatgagtccttccctgcctgcaagattgagttctgaaagagccgccctcccttccccaaggatccactcccccagctcctttagagaatggctactgctgagtcctttggggttgagggagatgggagctagggggaggggagggagatgtcttgttgtggggacttgggctgggctaaatgggaggggttgtccctccccatcatccattcctgtgaggtgtctcaaaccaaagttaacagggagaggatgggggaggggacaaattagaataggatagcatctgatgcctgagaaccctctcctagcactgtcaaatgctggtattgaatggggactgaggatgggtctcagagagcaacctcctccctcgtagagggagattatatccccaactccagggacctctttatctcaatctatttatttggcatcctgggagggatttccaatagtaatttatgtgacctggggcaggataccgtcagtgaggtgcccagagctgcaccctttcctccatttcccatcccccatctcctcaaccaccagggtctgagttctagcagggtcctgggggtatcccactgctatactgttctactgcttccctcagtatctgaatgtctcaatttaaaacttgaagctctttagaccaatagactggtgagaggagaaaggagcttatcccccagaccctgctttataccattcacatcccagggctgtgtccagacagcacaaaacggcaaggagagcccaagccccaatgccagaattcttccaaactccctgactctttgaagtttttactcaccccatttcaattatcctgatcccttctcatcccctgcttggcttctctgcatgtggtcatctgctgtggcttggtgtttaatgggttaaaaataagccactgcctgacatcccaacatttgacaccccagcaatgtgtgactcccccaacattccactatgccatcctgcagctgaaatgggaacactggctgcctctccaaacccgctcttggacagaggatctgggaggtggaagccaggccagaggacttggggaaaatgagatggaggaaggaaaaagggagaagctgagccacagcttaactcctacagagtgaaatgaaaacgggctgaaaataccaccccaggagaggacctcgccccaagcaagccagtgagcagccctgccagactactgccagactgagaaacccagaagctggtagtcatgtgggcttgccttctctgccaaacgactgggaaaccaaaatgagcccaccttgtgttcttcctagctccaccctccccgtgctgctgtgttctgctcctccccacgcttccctgctatagttcccagctgctgtaacggagccacctccaactctaacaataaaccaagttcattgca

SEQ ID NO: 29 - RNA, 8494 nt, Homo sapiens
  source 1..8494: mol_type = mRNA
agcagagaggagttgagggcgatgagagcgggtactgcgaactgccgggcgatgctgtcgctgccgccgtgatacggagagcaacagttccccagcaacacccctccccgacacaggcacacaccccccgacaggcacgcacacccaccccacagtgcccggctcggctgcgcctcctctattggcccaggaagcccacccagccccgccacgcagagcccagaaggaaagaaagcctcatgcctgagccgaggggagcaccatggatctgacaaaaatgggcatgatccagctgcagaaccctagccaccccacggggctactgtgcaaggccaaccagatgcggctggccgggactttgtgcgatgtggtcatcatggtggacagccaggagttccacgcccaccggacggtgctggcctgcaccagcaagatgtttgagatcctcttccaccgcaatagtcaacactatactttggacttcctctcgccaaagaccttccagcagattctggagtatgcatatacagccacgctgcaagccaaggcggaggacctggatgacctgctgtatgcggccgagatcctggagatcgagtacctggaggaacagtgcctgaagatgctggagaccatccaggcctcagacgacaatgacacggaggccaccatggccgatggcggggccgaggaagaagaggaccgcaaggctcggtacctcaagaacatcttcatctcgaagcattccagcgaggagagtgggtatgccagtgtggctggacagagcctccctgggcccatggtggaccagagcccttcagtctccacttcatttggtctttcagccatgagtcccaccaaggctgcagtggacagtttgatgaccataggacagtctctcctgcagggaactcttcagccacctgcagggcccgaggagccaactctggctgggggtgggcggcaccctggggtggctgaggtgaagacggagatgatgcaggtggatgaggtgcccagccaggacagccctggggcagccgagtccagcatctcaggagggatgggggacaaggttgaggaaagaggcaaagaggggcctgggaccccgactcgaagcagcgtcatcaccagtgctagggagctacactatgggcgagaggagagtgccgagcaggtgccacccccagctgaggctggccaggcccccactggccgacctgagcacccagcacccccgcctgagaagcatctgggcatctactccgtgttgcccaaccacaaggctgacgctgtattgagcatgccgtcttccgtgacctctggcctccacgtgcagcctgccctggctgtctccatggacttcagcacctatggggggctgctgccccagggcttcatccagagggagctgttcagcaagctgggggagctggctgtgggcatgaagtcagagagccggaccatcggagagcagtgcagcgtgtgtggggtcgagcttcctgataacgaggctgtggagcagcacaggaagctgcacagtgggatgaagacgtacgggtgcgagctctgcgggaagcggttcctggatagtttgcggctgagaatgcacttactggctcattcagcgggtgccaaagcctttgtctgtgatcagtgcggtgcacagttttcgaaggaggatgccctggagacacacaggcagacccatactggcactgacatggccgtcttctgtctgctgtgtgggaagcgcttccaggcgcagagcgcactgcagcagcacatggaggtccacgcgggcgtgcgcagctacatctgcagtgagtgcaaccgcaccttccccagccacacggctctcaaacgccacctgcgctcacatacaggcgaccacccctacgagtgtgagttctgtggcagctgcttccgggatgagagcacactcaagagccacaaacgcatccacacgggtgagaaaccctacgagtgcaatggctgtggcaagaagttcagcctcaagcatcagctggagacgcactatagggtgcacacaggtgagaagccctttgagtgtaagctctgccaccagcgctcccgggactactcggccatgatcaagcacctgagaacgcacaacggcgcctcgccctaccagtgcaccatctgcacagagtactgccccagcctctcctccatgcagaagcacatgaagggccacaagcccgaggagatcccgcccgactggaggatagagaagacgtacctctacctgtgctatgtgtgaagggaggcccgcggcggtggagccgagcggggagccaggaaagaagagttggagtgagatgaaggaaggactatgacaaataaaaaaggaaaagaaaaaaaaaaacagaaggaaaaggaaacctggtagctttttggccttggattctctctgggctccagatgacctggatgccaagccactgcccctcctctgggggcctccaccctcctctcccggctggaggtttgcctgattttctgggatggggttgggtattttgttcactcaaatggtggcacatttttctccttccttcacccagaccttcttttatgtgtccagaaatggaggctagaaagcaggtgagaggtcctctggtcagagccacacggtctgtgccggccttcctccaccaagacccccaggagatgaagggagggaggaggtgagccagaagggcgctcccctgctgatgggtctgggctgggtcactagctgctcaaaatggcagctctagtttgctggcggctgactggggaggagaagggctctgtttctcttcccaccactcagcccacctgctgctttcctctgctttgccacatctgggtgtcccccggtggtctctgagagcctcaggacccctgcccctcctccagctctttgttcccagcctccccttgactcctgtcctccaagtcccaggggagtcccagcccctcagggacctggcggtgtctccatccttctccggttccctagtgggatagctgcctctgacttcagggtccctcctaccctcagccttctgagaacacaaaacaaatccaataccccaccctagtccagcaccatcgtgagcaagattcctgctgcgctgcttccaaaatggaaaagcatcacaactaaatacctaatatcctaccaaacaaaccacagtccctacgtagccctacttcagtcccaggagaaggaatccatgaatgggctgaggttccgagggtaggttgtggatgtctttctctagaggggtcccacacctggaaaagaggacacccagcccgtgggatgagggaagctgggcaagggagaaagttgttgagtcacactggggaccccagatgtagtgagctcagcaagaaaagccaggtccagagagagtcgcacagaattcctgactcacagcgcccctcggtccacagtggagaggaggaggaggaggagcagaaggagggggaggagctgcaggaggaggaggatttgaaagcgctttggccttgtgttatgttttgcttcttttctgtgtcccctgttagcacattgtacttgaattacctcagttttttgtgacctcatgagctttcttaacctctgtatctctttttcggttggggcttggaggaatggggagggtgttcttttctgtttcttgtgtaaattaatagttgtttttatagacttcagctggtcaagaccctccccgtgcccctggagaccagcctcccagctggcaggaactgtgcaggaggagttgatactcaggatctgaatgtgagggccgaggagggcgaagagcgtgggtggggaggggatgttgctttggggtctcatggtccccagagggcactagggagtcacttttggctccgctggtgcatgaagtcacctgtggccaccatccgttccgcctaaaacactctggagagaatcccacctttcttacaatttgctgggccattgaggtttgagggcctgtgtttggatccttgcaactgtgtggtctcacctctgtgcgtgcattctcattgccagaattggtctattttcacggctggtctttggggaggggggcgggatccagcctttgttttgttgtgttggggtgggggtgttgtttttctaaaagctacctcttatgtttgtccagttgttcttttgttcctttcccgcctcccattctgctgctcttcctccctcttttccccaacctcccccgaccctcctgaattttggaaagcacatttgcaatattcgtgtttgctttgggacggaccctccgtttcatctcatgctttatgtgtaagagttttttattattattttttctttcctttctctctctgagaaagttgtggctgcgttttgatcttaggttttacaaagtggtttagggaagcggttttggggagaaggatcacgaggaatgtagggaagccggagggatgggtgctgctgcgacgacccccccgtccctcggccccagccctcctgccctccccttcaatctcatccaccaaatctgaaggccttaaaattgtgtgttgggaggatgtgaattgggaggacggtgtcactagactgtggattagggatggtaaagtagggaggatgctattttgcaactatagtaacgacttagtgttttggaaaggaaaagaagttaaacttgaaatacgtgactagaacagttgtcatgtttataatgtgaaaagggtgaaatcatttgggggaggggccgtctgtaagaaatcattatgcactatggcttcctcctctggtctgggaagaagcggggactggctggccctcaggggatctgtaaatcccagaaaacagtatttttaacagcaagatgtcattcaacattggtggggaaggaagagaaaaaaatcaaactattccatagaactagctggccccctcactcccatgcccttcccactcagcctgggcccctccccgctccattcataaaagctgagagggttgagctaatcttcacaaattgtaatatttttgtagtatctgttagttccttcgtcagttctgcagaaccttgccctttccttttgtaatgtgaataggaagacaaaagacaaaaaaaaatccaccaccaccaaaatatccctttgtacatgtatgtgcgtgtgcgcgtgtgctttgtgtgtgtggttgtgtgttaaatcatgcagtattgtcgtaatctggtgttgcagcaatggatggtactaaatcagcacctggatgccccacccaaccccgtgggccctgcagaccccagtagggaggtatggggagagctcaggggagtgtggtttctgagggctactgtctggggacacctctgaacttactgtaccttcctctccccatgaagacacctgaatagagtctaacatgcctcttctccaacttcctacctacaacaacagaacagttctaatgttgcacggcctagtggccagggggcaagctaagaggctgtctggaggctttatatgtgtctggagttaaggggagaggaggagggtagacaggggtctctccccaggtgggatctgaatatctgtcctcccctcttcttcatgccacctgactccttcggccccctggctgcctttagctgtggtactgctgacaaccctgcttgctactgccttatccagcacagtgaaaaacttctccagcctggcaaggccacgttggttaatagtccctttcccatgtccagctcctacaaatatgtcccttaatgcatttggtgacatttacacctcatgtgctctttccctattcactccttcactcattcaaagcattaaaatcctatgtatatataggatagacaaatatatagatatatagatatatatatatatagcaagagattgatataaaatagtaaatatcattgctgctttgggctgctttggaggaggaggccatgaatatggggaaggcagatctggggtgcaggggtaggtagggaggctgggggacccagtgattcagtacaatccaagggatgcaacgcgggcttgtttaatctttgtgcctgaacagtttttccatgttgagaaaaaaaagaaaaaaaaactgctgcaatttttcacaagtgtatggtacctttctggatgctattggtacaattgctgtggatggaagagggccattgagcttacctccctataggggagagagcagaggtggggcagcctttcgactctgtccatgacggctggcagggtcagggtagtttctgggcctgcttcccggcaagccgagctagggtgaaaactgggggcgcaccaggatgtgagacagaaaagcagaagatgagactctgttcattcacttttcctaggcccatcctgtggtcatctttccccctcccatcatacctcctccttcctggagcctctgccggcttggctgtaatggtggcacttacctggatatttcagtgggaggatgaaaggcgagactcaccctacgcggtgggacagatggggagaggaaaaaggcagagatggccaggagaggggtgcaggacaaaccagagaggttgggtcaggggaaaagggtggggagaaagaggggtgcaggccctgcaggccggttagccagcagctgcggcctccccgggcccttggcatccaacttcgcagacagggtaccagcctcctggtgtgtatcataggatttgttcacatagtgttatgcatgatcttcgtaaggttaagaagccgtggtggtgcaccatgacatccaacccgtatatataaagataaatatatatatatatgtatgtaaattatagcactgagggccctgctgccctgctggaccaagcaaaactaagccttttggtttgggtattatgtttcgttttgttatttgtttgtttttgtggcttgtcttatgtcgtgatagcacaagtgccagtcggattgctctgtattacagaatagtgtttttaattcatcaatgttctagttaatgtctacctcagcacctcctcttagcctaattttaggaggttgcccaattttgtttcttcaattttactggttacttttttgtacaaatcaatctctttctctctttctctcctccccacctctcacccttgccctctccatctccctctcccgccctcccctcctccctctggctccccgtctcatttctgtccactccattctctctccctctctcctgcctcctgctgccccctccccagcccacttccccgagttgtgcttgccgctccttatctgttctagttccgaagcagtttcactcgaagttgtgcagtcctggttgcagctttccgcatctgccttcgtttcgtgtagattgacgcgtttctttgtaatttcagtgtttctgacaagatttaaaaaaaaaaaaaaaggaaaaaaaaagaaaaaatgaatttactgctgcaggtttttttctctctccatgtgtcactaagtgaagtttgtgccttctatagcaaagagaatattttttacatcctactaacagtagatttttttgtagtgaacattttttgtatttttatttataagtctcataagaaaaatagcaatgttcagttgtataccttgaatctgcagttagaagagaataaagttaattcagttgtctctcgcttgaagcgtcccacctttttattgaagtacttggttttgttttgttttttttttttgttttttttgccttttcttgtgtggggaacatggtagaggaattaagatttttgtgtggggactgggaaaaagaaagctctgtattacacatatttagacttatctatgtgtcacttttatgccacatttacaaggcacagatgcactgaataacatttttctaatactttttagttaaaaaatgttaaatacgttaatatcgtatgatccttggtacaatgtgctaggtaggcacttgttcacttattcagcaagaccaccatgtaccagttactgttgtcggcgctgggaattacagcaaaggacaaacagacaaaccctggccgccctggggctaccatgctagcgggccgctgagtcggaatccgtggctgtgttaggataacttgctcaggattgcacggctggtgagcagcagtcagaactccatccacctctcctgataccaggccaggttcctttactccagagttctcaaagcaggggtctcacgtcttctttagtctttagagagacattttcaactgactccttagtggctaagcaagcttcagaaatttctcaacaagaagcttccacacaatcaaaggtccctgcctgcgtctgtagcagccaagagctgttaagaaaggagattggagcaggtggccttgtgcaggggaggggatgggtgggaggtggccgtgcaagctctgcattgtcatggacggaataaaggatttccacaaca

SEQ ID NO: 30 - RNA, 4464 nt, Homo sapiens
  source 1..4464: mol_type = mRNA
gcgcactccagccctgcagcctccggagtcagtgccgcgcgcccgccgccccgcgccttcctgctcgccgcacctccgggagccggggcgcacccagcccgcagcgccgcctccccgcccgcgccgcctccgaccgcaggccgagggccgccactggccggggggaccgggcagcagcttgcggccgcggagccgggcaacgctggggactgcgccttttgtccccggaggtccctggaagtttgcggcaggacgcgcgcggggaggcggcggaggcagccccgacgtcgcggagaacagggcgcagagccggcatgggcatcgggcgcagcgaggggggccgccgcggggcagccctgggcgtgctgctggcgctgggcgcggcgcttctggccgtgggctcggccagcgagtacgactacgtgagcttccagtcggacatcggcccgtaccagagcgggcgcttctacaccaagccacctcagtgcgtggacatccccgcggacctgcggctgtgccacaacgtgggctacaagaagatggtgctgcccaacctgctggagcacgagaccatggcggaggtgaagcagcaggccagcagctgggtgcccctgctcaacaagaactgccacgccggcacccaggtcttcctctgctcgctcttcgcgcccgtctgcctggaccggcccatctacccgtgtcgctggctctgcgaggccgtgcgcgactcgtgcgagccggtcatgcagttcttcggcttctactggcccgagatgcttaagtgtgacaagttccccgagggggacgtctgcatcgccatgacgccgcccaatgccaccgaagcctccaagccccaaggcacaacggtgtgtcctccctgtgacaacgagttgaaatctgaggccatcattgaacatctctgtgccagcgagtttgcactgaggatgaaaataaaagaagtgaaaaaagaaaatggcgacaagaagattgtccccaagaagaagaagcccctgaagttggggcccatcaagaagaaggacctgaagaagcttgtgctgtacctgaagaatggggctgactgtccctgccaccagctggacaacctcagccaccacttcctcatcatgggccgcaaggtgaagagccagtacttgctgacggccatccacaagtgggacaagaaaaacaaggagttcaaaaacttcatgaagaaaatgaaaaaccatgagtgccccacctttcagtccgtgtttaagtgattctcccgggggcagggtggggagggagcctcgggtggggtgggagcgggggggacagtgccccgggaacccggtgggtcacacacacgcactgcgcctgtcagtagtggacattgtaatccagtcggcttgttcttgcagcattcccgctcccttccctccatagccacgctccaaaccccagggtagccatggccgggtaaagcaagggccatttagattaggaaggtttttaagatccgcaatgtggagcagcagccactgcacaggaggaggtgacaaaccatttccaacagcaacacagccactaaaacacaaaaagggggattgggcggaaagtgagagccagcagcaaaaactacattttgcaacttgttggtgtggatctattggctgatctatgcctttcaactagaaaattctaatgattggcaagtcacgttgttttcaggtccagagtagtttctttctgtctgctttaaatggaaacagactcataccacacttacaattaaggtcaagcccagaaagtgataagtgcagggaggaaaagtgcaagtccattatgtaatagtgacagcaaagggaccaggggagaggcattgccttctctgcccacagtctttccgtgtgattgtctttgaatctgaatcagccagtctcagatgccccaaagtttcggttcctatgagcccggggcatgatctgatccccaagacatgtggaggggcagcctgtgcctgcctttgtgtcagaaaaaggaaaccacagtgagcctgagagagacggcgattttcgggctgagaaggcagtagttttcaaaacacatagttaaaaaagaaacaaatgaaaaaaattttagaacagtccagcaaattgctagtcagggtgaattgtgaaattgggtgaagagcttaggattctaatctcatgttttttccttttcacatttttaaaagaacaatgacaaacacccacttatttttcaaggttttaaaacagtctacattgagcatttgaaaggtgtgctagaacaaggtctcctgatccgtccgaggctgcttcccagaggagcagctctccccaggcatttgccaagggaggcggatttccctggtagtgtagctgtgtggctttccttcctgaagagtccgtggttgccctagaacctaacaccccctagcaaaactcacagagctttccgtttttttctttcctgtaaagaaacatttcctttgaacttgattgcctatggatcaaagaaattcagaacagcctgcctgtccccccgcactttttacatatatttgtttcatttctgcagatggaaagttgacatgggtggggtgtccccatccagcgagagagtttcaaaagcaaaacatctctgcagtttttcccaagtaccctgagatacttcccaaagcccttatgtttaatcagcgatgtatataagccagttcacttagacaactttacccttcttgtccaatgtacaggaagtagttctaaaaaaaatgcatattaatttcttcccccaaagccggattcttaattctctgcaacactttgaggacatttatgattgtccctctgggccaatgcttatacccagtgaggatgctgcagtgaggctgtaaagtggccccctgcggccctagcctgacccggaggaaaggatggtagattctgttaactcttgaagactccagtatgaaaatcagcatgcccgcctagttacctaccggagagttatcctgataaattaacctctcacagttagtgatcctgtccttttaacaccttttttgtggggttctctctgacctttcatcgtaaagtgctggggaccttaagtgatttgcctgtaattttggatgattaaaaaatgtgtatatatattagctaattagaaatattctacttctctgttgtcaaactgaaattcagagcaagttcctgagtgcgtggatctgggtcttagttctggttgattcactcaagagttcagtgctcatacgtatctgctcattttgacaaagtgcctcatgcaaccgggccctctctctgcggcagagtccttagtggaggggtttacctggaacattagtagttaccacagaatacggaagagcaggtgactgtgctgtgcagctctctaaatgggaattctcaggtaggaagcaacagcttcagaaagagctcaaaataaattggaaatgtgaatcgcagctgtgggttttaccaccgtctgtctcagagtcccaggaccttgagtgtcattagttactttattgaaggttttagacccatagcagctttgtctctgtcacatcagcaatttcagaaccaaaagggaggctctctgtaggcacagagctgcactatcacgagcctttgtttttctccacaaagtatctaacaaaaccaatgtgcagactgattggcctggtcattggtctccgagagaggaggtttgcctgtgatttcctaattatcgctagggccaaggtgggatttgtaaagctttacaataatcattctggatagagtcctgggaggtccttggcagaactcagttaaatctttgaagaatatttgtagttatcttagaagatagcatgggaggtgaggattccaaaaacattttatttttaaaatatcctgtgtaacacttggctcttggtacctgtgggttagcatcaagttctccccagggtagaattcaatcagagctccagtttgcatttggatgtgtaaattacagtaatcccatttcccaaacctaaaatctgtttttctcatcagactctgagtaactggttgctgtgtcataacttcatagatgcaggaggctcaggtgatctgtttgaggagagcaccctaggcagcctgcagggaataacatactggccgttctgacctgttgccagcagatacacaggacatggatgaaattcccgtttcctctagtttcttcctgtagtactcctcttttagatcctaagtctcttacaaaagctttgaatactgtgaaaatgttttacattccatttcatttgtgttgtttttttaactgcattttaccagatgttttgatgttatcgcttatgttaatagtaattcccgtacgtgttcattttattttcatgctttttcagccatgtatcaatattcacttgactaaaatcactcaattaatcaa

SEQ ID NO: 31 - RNA, 2925 nt, Homo sapiens
  source 1..2925: mol_type = mRNA
gactctcccctggagcagcgtgactgacaccggctcctattcagctgggaggagggagaggggaggagaaggggagggccgcgggaggagggtacgagtggccgaccacggatttgcattgccgaggacgggaccccagggcagcgaagcagaatggccaacatgcagggactggtggaaagactggaacgagctgtcagccgcctggagtcgctgtctgcagagtcccacaggccccctgggaactgcggggaagtcaatggtgtcattgcaggtgtggcaccctccgtggaagcctttgacaagctgatggacagtatggtggccgagtttttaaagaacagtaggatccttgctggggacgtggagacccatgcagaaatggtgcacagtgctttccaggcccagcgggctttccttctgatggcctctcagtaccaacaaccccacgagaatgacgtggccgcacttctgaaacccatatcggaaaagattcaggaaatccaaactttcagagagagaaaccgggggagtaacatgtttaatcatctttcggccgtcagcgaaagcatccctgcccttggatggatagctgtgtctcccaaacctggtccttatgtcaaggagatgaatgacgctgccaccttttacactaacagggtcttaaaggactacaaacacagtgatttgcgtcatgtggattgggtgaagtcatatttgaacatttggagtgaacttcaagcatacatcaaggaacaccacaccacgggcctcacatggagcaaaacaggtcctgtagcatccacagtatcagcgttttctgtcctctcctctgggcctggccttcctccaccccctcctcctctgcctcctccagggccacctccacttttcgagaatgaaggcaaaaaagaggaatcttctccttcacgctcagctttatttgcccaacttaaccagggagaagcaattacaaaagggctccgccatgtcacagatgaccagaagacatacaaaaatcccagcctgcgggctcaaggagggcaaactcaatctcccaccaaaagtcacactccaagtcccacatctcctaaatcttatccttctcaaaaacatgccccagtgttggagttggaaggaaagaaatggagagtggagtaccaagaggacaggaatgaccttgtgatttcagagactgagctgaaacaagtggcttacattttcaaatgcgaaaaatcaactattcagataaaagggaaagtaaactccattataattgacaactgtaaaaaactcggcctggtgtttgacaatgtggtgggcattgtggaagtgatcaactcccaggacattcaaatccaggtaatggggagagtgccaacaatttccattaataagacagaaggttgccacatatacctcagtgaagatgcattagactgtgagatcgtgagcgccaagtcatctgaaatgaacatacttatccctcaggatggtgattatagagaatttcccattcctgaacagttcaagacagcatgggatggatccaagttaatcactgaacctgcagaaattatggcctaacttcctgagagaccgaaccccctcacctgaatccccctctatcaaacaaacaaaaaagcagcagtaaagagctagaagttgcagtagcccctactgctttagctttggcctccaacgattctgtgctatagatacagcactgtttctggcacgcctcgtgggcattttgaaatatttaacgtttcctcatgatttgcctttgtgtgtgattttagttccacatgatgacttgtgaacattagggatttaaaggaaaaaaaaaaagaattctgttcccctcatatcatgaacacagtaactgataggtaaaaagactgcatgattcacttttacacttatatttcattgctagttaaaaaataaaacctttgagaatctaagatgtacatttttaccttttaggcaatttcaatataatgtagaagtagtagtgtgccctgaaaaatgtacacgttttttcttattgttaccacatgttcacctttatcagcgtggatactgtcagcatgagtacatatttcaacccacgcttgtaaaagacataagagtttataaaggaccaaattcagttccttggtccttggaagacctatattctctgtagttactgaaaaccgaaagtcaattctaattattcatcttacatatttttccaccatgtcatttgaaaacttgcttttcttctgcataagagattcttatgccaaaaacattaaacagaagaaatcattttttttgctatgtaatacctcgcaactttgctctaaaatcaagctcagttattattttccaagtttgaacatgttaaatatcagatgccttgtaaattatgtctttaacgttttcttatagactaatttcctcttttccacctgccagacttgctaaccaagctcgaaaatgaacatgaaaaagccatacatgtattatttctcctaaaacctaaggcattatctgttggtttggcttgctgctcctattttgtagtcttgatagtagatgcttcttcagcgtaagagtagctatgatattcctttttatcttttcagtacatagtgctgaaaaatctgcaacttcttggatcatatttaatgaattatagtataatgcttgcaggcccagtacaagcatatatattgtgcctcttacagcctttggaatacattgtttccattttttaaatatcttctatatccatatagtattcaaattattaatgctcatgtaccaaggttttgctataaaagttttgtctgtatgaataatgtggctttagtaaataatcatttttcaactgtaaacttattctgaaataaagtaaaattctaattgtttaaa

SEQ ID NO: 32 - RNA, 9905 nt, Homo sapiens
  source 1..9905: mol_type = mRNA
gggctccccgcgccgcccggtcggcagcagggcgctgagcgagctcggagcccgcgctgtgcgcctgcggccggggcgccccgccgagcgccggtgccccggctcccgggccgccttcgccgcgcgggaaggattcttcaaaattaacagaaaccaattcgggccagctgaagagaaaaaataaaggtggctcccggctgcctctgctgcagttcagagcaacttcaggagcttcccagccgagagcttcaggacgcctttcctgtcccactggcccagttgccacaacaaacaacagagaagacggtgaccatgggggatgtgaagctggttgcctcgtcacacatttccaaaacctccctcagtgtggatccctcaagagttgactccatgcccctgacagaggcccctgctttcattttgccccctcggaacctctgcatcaaagaaggagccaccgccaagttcgaagggcgggaagttttgcgaagcagcttggtcagcctgttgtttccaaaaccttaggggatagattttcagctccagcagtggagacccgtcctagcatctggggggagtgcccaccaaagtttgctaccaagctgggccgagttgtggtcaaagaaggacagatgggacgattctcctgcaagatcactggccggccccaaccgcaggtcacctggctcaagggaaatgttccactgcagccgagtgcccgtgtgtctgtgtctgagaagaacggcatgcaggttctggaaatccatggagtcaaccaagatgacgtgggagtgtacacgtgcctggtggtgaacgggtcggggaaggcctcgatgtcagctgaactttccatccaaggtttggacagtgccaataggtcatttgtgagagaaacaaaagccaccaattcagatgtcaggaaagaggtgaccaatgtaatctcaaaggagtcgaagctggacagtctggaggctgcagccaaaagcaagaactgctccagcccccagagaggtggctccccaccctgggctgcaaacagccagcctcagcccccaagggagtccaagctggagtcatgcaaggactcgcccagaacggccccgcagaccccggtccttcagaagacttccagctccatcaccctgcaggccgcaagagttcagccggaaccaagagcaccaggcctgggggtcctatcaccttctggagaagagaggaagaggccagctcctccccgtccagccaccttccccaccaggcagcctggcctggggagccaagatgttgtgagcaaggctgctaacaggagaatccccatggagggccagagggattcagcattccccaaatttgagagcaagccccaaagccaggaggtcaaggaaaatcaaactgtcaagttcagatgtgaagtttccgggattccaaagcctgaagtggcctggttcctggaaggcacccccgtgaggagacaggaaggcagcattgaggtttatgaagatgctggctcccattacctctgcctgctgaaagcccggaccagggacagtgggacatacagctgcactgcttccaacgcccaaggccagctgtcctgtagctggaccctccaagtggaaaggcttgccgtgatggaggtggccccctccttctccagtgtcctgaaggactgcgctgttattgagggccaggattttgtgctgcagtgctccgtacgggggaccccagtgccccggatcacttggctgctgaatgggcagcccatccagtacgctcgctccacctgcgaggccggcgtggctgagctccacatccaggatgccctgccggaggaccatggcacctacacctgcctagctgagaatgccttggggcaggtgtcctgcagcgcctgggtcaccgtccatgaaaagaagagtagcaggaagagtgagtaccttctgcctgtggctcccagcaagcccactgcacccatcttcctgcagggcctctctgatctcaaagtcatggatggaagccaggtcactatgactgtccaagtgtcagggaatccaccccctgaagtcatctggctgcacaatgggaatgagatccaagagtcagaggacttccactttgaacagagaggaactcagcacagcctttgtatccaggaagtgttcccggaggacacgggcacgtacacctgcgaggcctggaacagcgctggagaggtccgcacccaggccgtgctcacggtacaagagcctcacgatggcacccagccctggttcatcagtaagcctcgctcagtgacagcctccctgggccagagtgtcctcatctcctgcgccatagctggtgacccctttcctaccgtgcactggctcagagatggcaaagccctctgcaaagacactggccacttcgaggtgcttcagaatgaggacgtgttcaccctggttctaaagaaggtgcagccctggcatgccggccagtatgagatcctgctcaagaaccgggttggcgaatgcagttgccaggtgtcactgatgctacagaacagctctgccagagcccttccacgggggagggagcctgccagctgcgaggacctctgtggtggaggagttggtgctgatggtggtggtagtgaccgctatgggtccctgaggcctggctggccagcaagagggcagggttggctagaggaggaagacggcgaggacgtgcgaggggtgctgaagaggcgcgtggagacgaggcagcacactgaggaggcgatccgccagcaggaggtggagcagctggacttccgagacctcctggggaagaaggtgagtacaaagaccctatcggaagacgacctgaaggagatcccagccgagcagatggatttccgtgccaacctgcagcggcaagtgaagccaaagactgtgtctgaggaagagaggaaggtgcacagcccccagcaggtcgattttcgctctgtcctggccaagaaggggacttccaagacccccgtgcctgagaaggtgccaccgccaaaacctgccaccccggattttcgctcagtgctgggtggcaagaagaaattaccagcagagaatggcagcagcagtgccgagaccctgaatgccaaggcagtggagagttccaagcccctgagcaatgcacagccttcagggcccttgaaacccgtgggcaacgccaagcctgctgagaccctgaagccaatgggcaacgccaagcctgccgagaccctgaagcccatgggcaatgccaagcctgatgagaacctgaaatccgctagcaaagaagaactcaagaaagacgttaagaatgatgtgaactgcaagagaggccatgcagggaccacagataatgaaaagagatcagagagccaggggacagccccagccttcaagcagaagctgcaagatgttcatgtggcagagggcaagaagctgctgctccagtgccaggtgtcttctgaccccccagccaccatcatctggacgctgaacggaaagaccctcaagaccaccaagttcatcatcctctcccaggaaggctcactctgctccgtctccatcgagaaggcactgcctgaggacagaggcttatacaagtgtgtagccaagaatgacgctggccaggcggagtgctcctgccaagtcaccgtggatgatgctccagccagtgagaacaccaaggccccagagatgaaatcccggaggcccaagagctctcttcctcccgtgctaggaactgagagtgatgcgactgtgaaaaagaaacctgcccccaagacacctccgaaggcagcaatgccccctcagatcatccagttccctgaggaccagaaggtacgcgcaggagagtcagtggagctgtttggcaaagtgacaggcactcagcccatcacctgtacctggatgaagttccgaaagcagatccaggaaagcgagcacatgaaggtggagaacagcgagaatggcagcaagctcaccatcctggccgcgcgccaggagcactgcggctgctacacactgctggtggagaacaagctgggcagcaggcaggcccaggtcaacctcactgtcgtggataagccagaccccccagctggcacaccttgtgcctctgacattcggagctcctcactgaccctgtcctggtatggctcctcatatgatgggggcagtgctgtacagtcctacagcatcgagatctgggactcagccaacaagacgtggaaggaactagccacatgccgcagcacctctttcaacgtccaggacctgctgcctgaccacgaatataagttccgtgtacgtgcaatcaacgtgtatggaaccagtgagccaagccaggagtctgaactcacaacggtaggagagaaacctgaagagccgaaggatgaagtggaggtgtcagatgatgatgagaaggagcccgaggttgattaccggacagtgacaatcaatactgaacaaaaagtatctgacttctacgacattgaggagagattaggatctgggaaatttggacaggtctttcgacttgtagaaaagaaaactcgaaaagtctgggcagggaagttcttcaaggcatattcagcaaaagagaaagagaatatccggcaggagattagcatcatgaactgcctccaccaccctaagctggtccagtgtgtggatgcctttgaagaaaaggccaacatcgtcatggtcctggagatcgtgtcaggaggggagctgtttgagcgcatcattgacgaggactttgagctgacggagcgtgagtgcatcaagtacatgcggcagatctcggagggagtggagtacatccacaagcagggcatcgtgcacctggacctcaagccggagaacatcatgtgtgtcaacaagacgggcaccaggatcaagctcatcgactttggtctggccaggaggctggagaatgcggggtctctgaaggtcctctttggcaccccagaatttgtggctcctgaagtgatcaactatgagcccatcggctacgccacagacatgtggagcatcggggtcatctgctacatcctagtcagtggcctttcccccttcatgggagacaacgataacgaaaccttggccaacgttacctcagccacctgggacttcgacgacgaggcattcgatgagatctccgacgatgccaaggatttcatcagcaatctgctgaagaaagatatgaaaaaccgcctggactgcacgcagtgccttcagcatccatggctaatgaaagataccaagaacatggaggccaagaaactctccaaggaccggatgaagaagtacatggcaagaaggaaatggcagaaaacgggcaatgctgtgagagccattggaagactgtcctctatggcaatgatctcagggctcagtggcaggaaatcctcaacagggtcaccaaccagcccgctcaatgcagaaaaactagaatctgaagaagatgtgtcccaagctttccttgaggctgttgctgaggaaaagcctcatgtaaaaccctatttctctaagaccattcgcgatttagaagttgtggagggaagtgctgctagatttgactgcaagattgaaggatacccagaccccgaggttgtctggttcaaagatgaccagtcaatcagggagtcccgccacttccagatagactacgatgaggacgggaactgctctttaattattagtgatgtttgcggggatgacgatgccaagtacacctgcaaggctgtcaacagtcttggagaagccacctgcacagcagagctcattgtggaaacgatggaggaaggtgaaggggaaggggaagaggaagaagagtgaaacaaagccagagaaaagcagtttctaagtcatattaaaaggactatttctctaaaactcaaaaaaaaaaaaaaaactcaagatagtaaaagcacctagtgtgatagattatcggttaggtcatttgtgggttgattcttcagaaacagcagttgatacctagcagcgttattgatgggcattaatctatgttagttggcaccttaagatactagtgcagctagatttcatttagggaaatcaccagtaacttgactgaccaattgattttagagagaaagtaaccaaaccaaatatttatctgggcaaagtcataaattctccacttgaatgcgctcatgaaaaataaggccaaaacaagagttctgggccacagctcagcccagagggttcctggggatgggaggcctctctctccccaccccctgactctagagaactgggttttctcccagtactccagcaattcatttctgaaagcagttgagccactttattccaaagtacactgcagatgttcaaactctccatttctctttccccttccacctgccagttttgctgactctcaacttgtcatgagtgtaagcattaaggacattatgcttcttcgattctgaagacaggtccctgctcatggatgactctggcttccttaggaaaatatttttcttccaaaatcagtaggaaatctaaacttatcccctctttgcagatgtctagcagcttcagacatttggttaagaacccatgggaaaaaaaaaatccttgctaatgtggtttcctttgtaaaccaggattcttatttgtgctgttatagaatatcagctctgaacgtgtggtaaagatttttgtgtttgaatataggagaaatcagtttgctgaaaagttagtcttaattatctattggccacgatgaaacagatttcaactgataaagagctggagaactccatgtactttggaatctcctccaagatagccagagtttaatacatcttcattctcaacactctccaaagaacttgacctaccttatgggttccatatttttcttcttaaatgtgcatcaatcatgccttgcccccaacctttaaatatattcttagacctggtaaatgcactcagacttgcgtctttaggaatttttaactttctttcactacattggcacttaaattttttctttataaagctttttgaaggtcataaacaaagaccataattgatgatagacctaatacatttcctctgtgtgtgtgtgtaacattccaaatactttttttttcttttccactgtttgtaaggtgcaacaatttaatatttttaagggactttttaagagttccttaagaaccaatttaaaattacttcagtgcaatcctacacagtatcaacattagaattttgatattagtcttatgttatcttccattctatttttatctgctttttgctgctagtttcaaactgccagtatttttccttttgcttttaaaatagttacaatatttttcatgatagccacagtattgccacagtttattataataaagggtttttatttgatttagcgcattcaaagcttttttctatcacttttgtgttcagaatataacctttgtgtgcgtgtatgttgtgtgtgtgcatgtgtggcgtatatgtgtgttacaggttaatgccttcttggaattgtgttaatgttctcttggtttattatgccatcagaatggtaaatgagaacactacaactgtagtcagctcacaatttttaaataaaggataccacagtgcatgctgtttgttcaatctttgcagacttctctttctttccatgctaccagttgtaaaggacacagctatatcctggaaatgaaaaacaaacactgtggtgcctagatgtgaagaactggcttatgtggttgtgttttgctatggaacagaatgatttaggaagttcttgtttatataggtagccgaatttacacatttagttcaaaatttctcttgagcatcagcttagtactatatcaatcattctagaaggatatcttatagagcaggtgtccccaacccccggtaagtagcctgttaggaaccaggtcacacataaggaggttagcagtgggcaagtgagcaaagcatcatctatatttacagccgatccccattgctcgcattaccgcctgagctctgcctcctgtcagatcagcggcagcatcaggttctctcaggaacgaactctattgtgaactgctcatgtgagggatctaggtttcacgctccttatgagaatctaacacctgatgatctgtcactgtctcccatcacccctagatgggacagtctagttgcaggaaaacaagctcagggcttccactgattctacattatgatgagttgtatacttattttatattataataaaatatattattacaatgtaataataatagaaataaaatgcacaatacatgtaatgtgcttgaataatcccaaaaccaccccctctcctggtccatggaaaaactgtcttccatgaaagtggtccctggtgccaaaaaggttagggaccactgttacagagtatcaggtcctcaagatgctaaaatctatatgacatttttaacatgtgacattatcatcatcatcatcatcatcatcactgatgatactatttaccagggcatggtttgaattggtgactttggtgcagttcattattggcagccaaatgctttatccataccttcatattgaagaatttgttatcaggaaactaccagtcctgctttacaggaagtctgttatcagatatcagatggcaagttccccatgtcttcagatgttcaaacaatattgtggatggtctagaaagagtttaagacatgctgttaaatgtagggctagataattctctgattctttgatgtagtctggaaagaaacaatccattgtccagttaataaatatttagtgttttcatttttaagacactcacaatccacaaatgtccctaacaatttattatttttaaagaaaatgactttttattccttgctagtgaaaaatgtacaatttatatgctgcactgagaaaaataacagatatactttcttccattcattttcatcccaaacatataaaaaataatccattgattgttccttgcattgcatatcttattaaaagatatttcctacatgcaactaataagacatgctgactgttgtcagctctaaatttatgtaaagattttttatttttgttaaaatgtttgaaatttgctttttgctccacacctcacctgtttttgataaatctgtgctaataagtacataggaggtaataaataattgagttgtgagaaacccaattctccatttttcaagaaaacacaagtagcactactctctttatcccttgggactccttcctgtaatttgaaagggggggctaatgttggtggcagttgttgctaaggatctctgcacagagttagggcttcactctcggcttcctggttagatggggccatgtgactagtcctagtcagtgagctgtgaccagaagtgatgtatgtaccctcgggaccagagcatttatgtgctggtacaagcctctccataatgacgggcaacacatgagatggtggctgctgcagccatctgggtctctagccaacccaaaatggggacataacacaagcaagaaataaacatttgttcttataaatcaccaagattttggggttctcagtggctgcaacataacctagactatcctgatacaggcttatcaccatgttctggatgtgtggtgaccaggatggtagccactactcacaagtggctatttaaatttaagttactttaaaaaataaaataaaaaattcagttcctcagttgtatgagttacatttcaaatgctcgacagtcacatgtacatcacttttcaaattatgtgaaattaaaactgaaaagcttgtgtgaaagtctagagagtatggtctatagtttcatcaattgtattggataatatagtctcgatactcaa

SEQ ID NO: 33 - RNA, 5419 nt, Homo sapiens
  source 1..5419: mol_type = mRNA
gactgcctgaccacatgcattatttttgaactggcccccagggtcctgtctttagccctgcctcttaacattgtcttggattcaacctaggtggagtcttcattctctcatccagctcctcggcctcatcggaacatttccaccaccattactcctttggaaactggtggcccggttccttcaaggggcacaggatgtctttgcctttttatcagaggtgccaccagcactatgatctcagctaccgcaacaaggacgtgcgcagcaccgtgagtcactaccagcgggagaagaaacgctccgccgtctacacccagggctccacggcctacagcagccgctcctccgccgcgcaccgccgggagtccgaggccttccgtcgggcgtccgcctcctcctcccagcagcaggcctcgcagcacgccctgagctctgaagtcagtcggaaggcagcctcagcctacgattatggctcctcccatggacttacagattccagtctgctgttagatgattattcatccaagttgagccccaaaccaaagagagccaagcacagcctactgtctggagaagagaaagaaaatttgcccagtgactacatggtacccattttctcaggacgtcaaaagcatgtcagtggaattactgatacggaagaagaaagaattaaagaagctgctgcttatatagcccagaggaatcttcttgctagtgaggaaggaatcacaacatctaaacagtccacggcatccaagcagaccacggcatctaagcagtccacggcatccaagcagtccacagcatccaagcagtccacggcatccaggcagtccacggcatccaggcagtctgtggtttccaaacaggccacatccgctcttcaacaggaagaaacttctgaaaagaagtcaaggaaagttgtgattcgagaaaaggcagaacgcctgtccctgaggaaaacattagaagaaaccgagacatatcatgccaagctgaatgaagaccatcttctccatgctcctgagtttatcattaaacctcgctcccacacggtttgggagaaggagaatgtaaaattgcattgctccatagcaggctggccagaacctcgtgtcacgtggtataaaaaccaggtgccaataaatgtccatgcaaaccctggaaagtatattattgagagtcgatatgggatgcacactctggagattaatggatgtgattttgaagatacagctcagtaccgggcctcggcgatgaatgttaaaggagagctttcggcatatgcttcagttgtggtaaaaaggtataagggagagtttgatgagactcgcttccacgctggggcttccaccatgcccctcagctttggtgtgaccccatatggttatgcatcccggtttgagatccactttgatgacaaatttgatgtgtcttttgggagagagggagagacaatgagtctaggctgtcgtgttgtcatcactcctgaaattaaacatttccagccagagatccagtggtacagaaacggagtacctctttctccatcaaaatgggtgcaaacactttggagtggagagcgggcaacgctgacattttcccatctcaacaaagaagatgaaggcctctatacaatccgtgtacggatgggagaatattatgaacaatatagtgcttatgtctttgttcgagatgctgatgcagagattgaaggagccccagctgctcccttggatgtgaagtgcttggaggccaacaaagattatatcatcatctcctggaaacagccagctgtcgatggagggagtcctattctcggatattttattgataagtgtgaggtgggcacagatagctggtcgcagtgcaatgacacacctgtgaagtttgctcgttttcctgtcactggattgatcgaaggtcgttcctatatcttccgagttcgagctgtgaataaaatgggaataggtttcccatctcgagtttccgagcccgtggctgctctggatccggctgagaaagctagacttaaaagtcgcccctcagcaccctggactggacagatcattgttactgaagaggaaccttcagagggtattgtgcctggccccccgacagacctctctgtcactgaggccacccggagctatgtggtgctcagctggaagccccctggccagcgtggtcatgagggcattatgtactttgtggaaaagtgtgaggcaggaacagaaaactggcagcgagtgaacacggagctccctgtgaagtctccccgctttgctctgtttgacttggccgaggggaaatcctactgtttccgtgtccgctgttctaattctgcaggagttggtgagccctcagaggcaacggaggtgactgtggtaggggacaaacttgatatccccaaggctcctggcaaaatcatcccaagcagaaacacagacacctcagtggtagtttcgtgggaggagtccaaagatgccaaagagctggtcgggtactacatagaggcgagcgttgctggctctggcaagtgggagccctgtaacaacaaccccgtgaagggctcacgattcacttgtcatggattagtgactggtcagagttatattttccgggtcagagcagtcaatgcagctggacttagtgaatattcccaggattcagaagctattgaagtcaaagctgctattgcaccaccatctccaccctgtgatatcacctgtcttgaaagttttcgtgactcaatggttcttggatggaagcaaccagataagattggaggggcagaaattactggctattatgtgaactatcgcgaggtcattgatggggtaccaggaaaatggagagaagccaatgtcaaggctgtcagtgaggaggcatacaagattagcaacttgaaggaaaacatggtgtatcagttccaagtggcagccatgaacatggctgggctgggcgcgccctccgcagtaagcgaatgcttcaaatgtgaagagtggaccatcgccgtcccaggaccaccgcacagtctcaagtgtagtgaagtcaggaaagactcactggttctccagtggaagccgccagtccactccgggcggactccggtcactggttacttcgtggacttgaaggaggccaaggccaaagaagaccagtggcgagggctcaatgaggcggctattaaaaacgtatacctgaaggttcgaggcctcaaggagggcgtcagctacgtgttccgtgttcgagccataaaccaggcgggagttgggaagccatctgaccttgctggccctgttgtggcagagacccgtccaggaaccaaagaggttgttgtaaatgtggatgatgatggagtcatttcattgaacttcgagtgtgataagatgactccaaagtccgagttctcctggtccaaagattatgtatccactgaggactctccacgattggaagtcgaaagcaagggcaacaagacgaaaatgaccttcaaagaccttgggatggatgacttgggtatttactcttgcgatgtaacagacactgatggaatagcatcaagctacttaatagatgaggaagaattgaaacgtttacttgctctcagccatgaacacaagttcccaactgtcccagttaaatcagagttggcagttgaaattttggagaaaggccaggtccggttttggatgcaggctgagaaactgtctggcaatgccaaagtcaactacatatttaacgagaaggaaatttttgaaggcccgaaatataaaatgcatattgaccgaaacactggcatcatcgaaatgttcatggaaaagctacaggatgaggatgagggaacgtacactttccagcttcaagatggaaaagcaactaaccattctactgttgttctcgttggagatgttttcaaaaagctccagaaagaagctgaattccagcggcaagaatggatcaggaaacaaggtcctcactttgttgagtatttgagctgggaagtgactggtgaatgtaatgtactattgaaatgcaaggtggcaaatattaagaaggagactcatattgtgtggtacaaagatgagagggagatatcagtggatgaaaagcatgactttaaggatggtatatgtaccctgcttataacagagttttccaagaaagatgctgggatttatgaagttatcctgaaagatgaccgaggaaaagataagagcagactgaagcttgtggatgaagcctttaaggaactgatgatggaagtatgcaaaaaaatagctttgtctgctacagacctgaaaatccagagcacagccgagggcatccaactgtactcttttgtaacttactatgtggaggatttgaaagttaactggtcccacaatgggtccgccattaggtactcagacagagttaagaccggggtcactggagagcagatctggctacaaatcaacgagcccaccccgaatgacaaagggaagtatgtcatggagctctttgatggcaaaactggacatcagaagacagtggatctctctggacaagcatacgatgaggcctatgctgaattccagaggttgaaacaagctgccattgccgagaaaaatcgtgcccgggtgttgggaggtctcccagacgtggtcaccatccaggaggggaaggcccttaatctcacttgcaacgtgtggggagacccgcctccggaggtgtcgtggttgaagaacgagaaggccctggcctcagacgaccactgcaacctcaagttcgaggctgggaggaccgcgtacttcaccatcaacggcgtgagcaccgctgactcgggcaaatacgggctggttgtgaagaacaagtatggctcggagaccagcgacttcaccgtcagcgtgttcatcccagaggaggaggcgaggatggccgccttggagtccctgaaaggtggcaagaaggccaagtgaccggaggtgcgaggagagccagccggcctgtgtgacttgggtgtgaatggtttgggttaaggatgagacgtcttcatgctttctcctccctattattttctggcttgaggggaaaataatgtcaggtctttcactcatataaaaaagcaccaactaatgacactttaattgtttttctttatctacaaaattatgtgttaagaaaataccattcatagcatgaagattaggaaacagttttaaggagaagacttgaatgaagttggagggacattgaatgatggtcagagggcagacgaatgtgtcgtggggcgaattgggatttgctgcagctgtgaagccatggccgtgtctcgtgtgttgttacagaggtgatgtgcttttcgacgggcgcctcgtggcttggaacctcctctgtatgaataaacagttttcacgtctgtcctcttccccga

SEQ ID NO: 34 - RNA, 4361 nt, Homo sapiens
  source 1..4361: mol_type = mRNA
atgctccgcagcgcggcgggtccacagatgaggggagtcgagactcccgcgccccaccacccccggcggagctgctgctgagccactcaatctgagccctggctactaataaaatttgagagggaagatctgatctcctagaattagagttggtacagaaaccatttcagctccaaaaatgttggaggaagatatggaagtcgccataaagatggtggttgtagggaatggagcagttggaaaatcaagtatgattcagcgatattgcaaaggcatttttacaaaagactacaagaaaaccattggagttgattttttggagcgacaaattcaagttaatgatgaagatgtcagactaatgttatgggacactgcaggtcaggaggaatttgatgcaattacaaaggcctactatcgaggagcccaggcttgtgtgctcgtgttctctaccacagatagggaatcttttgaagcagtttccagttggagagagaaagtagtagccgaagtgggagatataccaactgtacttgtgcaaaacaagattgatcttctggatgattcttgtataaagaatgaggaagctgaggcactggcaaaaaggttaaagttaagattctacagaacatcagtgaaagaagatctaaatgtgaatgaagtttttaagtatttggctgaaaaataccttcagaaactcaaacaacaaatagctgaggatccagaactaacgcattcaagtagtaacaagattggtgtctttaatacatctggtggaagtcactccggtcagaattcaggtaccctcaatggtggagatgtcatcaatcttagacccaacaaacaaaggaccaagaaaaacagaaatccttttagcagctgtagcataccctaagatgttttgggaggaaaacaattgaattacattgtgcaatgcattaagaaacccatccagctgtcatggtatgttacaaggttttcagcagactttgctcctaatggctctctgaaagtgacagacttaaatattgctctgcagtgcttttcagaatgtagagtgagacctctggtggaaaaattattgccctgtggactcctttaattttttttacattagacgaagcttctcctgtttgtaaaggaatgctataagaaatttcaaacacaggttttgcggaattttaaatgctggaaaacataaatgaaatgcctaaatatattgttacagattttaatactgtggatcaaggaaagatagcaagcattcttttcctgaaattggtcatgtagcttttctgcgaaatagtattgaatctgaatactttcacaaaataatactgaaaggtaaaccctaaatcttgccagactgcattagtattttggcattgaaacttgtgcaatatctgtgtaatgtagaatgtggggtgtgcatgcagatgtctggtactggagtaagctgaaggtatgtgcagtatttaagaaaatgtacattctaattaattcacttataaaaccatttacatattgtgtatatgtttttattttcaaatgataaactctagacatatattttgcaaaatgagcttgggtttaaaaagtgctttgtgccaaaaatatcatacctaatttttatagtgctttactatcagaatttatattgtttattatatcttttaaaagcagtaagcagttttcatctgacagcgtagataaaagaggagtataggaatttgaatgctagagcatctcccaggtgagccttattgcagatctttttgatatagtcacccataagcatggtgagctcctgctctcataaggtcagccaaagccccttaagaaggtacacagcacatctgcagtcattcaggaggtcctgtgaagtgtggtgatgcatctaacaccttttgctgctcactgagaacccagctttgaacttacaagattacactaaccatttttaaagtgcacaaaaatattattattagtcttaactaaaattacatattttataatgccctgcaactctaaaccatccttttgtttacacatttttgtatggtattttaagattatcaatcacttcaacatttctataaccttgtttgtatagcactttctcaagagctgtcagtcccacatacagaatcatttcttttacaaaatgatttaatatgtaatcatgtgtcaggacataaattttgtcacttgggacagtagctttccagctaagataattgcgtgaactctgttaaaactgattatcactcatcaatggctttatttttaacctataaataacccctttcaatatacctggtttttacagcattgcaaaatctgtaaaaataacttttattggaaaatgtcatgaagtcatttttcattatttgtactaaacaatgttttatgtactccttttgtgttttatcttttgtttttccatctgtactcccctcatcctcctaatgttgagaaaatcaaatttcctgggtgtgtccttgttaagtgatcaaaagtaaatgttctctttgccattttagatggaaaaataaaaaaaattaaaaagtaaatttttgcttttcattatattgaaatgatctggcattatctatttcacagtaatgtaaaatgcttatttttatgtcaccagttgtcaccactcccattgctgatagtgacataggttttgggggcaaaattcagttcctaacaaacagtggatactgctaatgagtcatcttttctactctcttcaattttctactctctactctcctctttaatttttgcacaaaataatactttgcaacaaatagtcttttgtctttattggcagaaaaatcacttgttatatgtgttctagttagttctttttcatgttagctgtgtggctaaaagcgtgttacctttctatatttaaaaaaagtaatctctgaggatagttacagttcctgtaatataattttatgtacctagttttatctttttttaaataagaactgaagagagagctttgttacatatttgaatttttaatttgcactgctgtattttaaacctaaccataattagtcatttaaaataattaagtaggcctgaaagtcagccatgttaatttctcaatttaatcaattcttaaagccttcaaaaattgacattttttttccaagacccttcattctcttaaataactttaattttatgaaaccatgtatactaaagaaaaacttttccaagattccaggtgattgtgcatttgtgctctaatctacttttttaacattacggctaatcttttgcgtagacatatcgctgtggaataactgccatatttcagagttcctcaggtttccttttccttttccagtctctgtctatgaattaaatagtatatagaatgacccatataaggcaatatagttaaataaaaccaggttaaatgatttcctttgtatctgcccaaagttgatagcacacgttactttttcaaaataaagctaaaactaccaaaaagaggatgaaaactttttcctcattatggagtgaagttctaggtggttgctttagaagttggcagtgcagtgctcagaaggaactctcaataaataacatgtactccttggacctgtgagttttaggaaactggaccttttctgaagaccttagaatagggagttggccttaggacctaatgtcccaacttagtgttggacccttttaatataagatattgttaattattagcatacttttcaaaacctttgaaatagttactgctaacctgataaaatgttcccattaatctatcattagtctgtttctctgaaaacaaaatgcattgatgaggtgaaagcttgttccacatggcacctacctaatgaacaggacttactcagtttttaactgttaagaatgtcacatgtactattgtcactccttaggttttcagctataaaacatgtaagtctctcatcatacagatgaattcatttgctaacaaaatatttaaaacccgcagtagactctgaaatatccagtcatcaaactcctggctaactggatgatttggctataataatctttattattattattttcatctgtctctcgaaatatctacagtaggatgttagtaaatggtcttttaaaagcaaaaaattggggataaaaggaaaactgaattccttctatatttttattactaataaataatgcttttgtaaatttgaatggaaaaccacttgtatgtattgctatttggttgcagttacactctggagcttaatttaaaacactactctaaaaatttcatgaaggatgaattccaataatcagaaaataaatgcatttcaaagctaaaa

SEQ ID NO: 35 - DNA, 5358 bp, Homo sapiens
  source 1..5358: mol_type = genomic DNA
agaaagccgcgcacctcctcccgccaggcgctttctcggacgccttgcccagcgggccgcccgaccccctgcaccatggaccccgctcgccccctggggctgtcgattctgctgcttttcctgacggaggctgcactgggcgatgctgctcaggagccaacaggtatctggccgctccaggagcttctctccccaaccggcggagagggcgcagcgggccatggggccccgtgtaggcgccctccaagcctcgctttctccaggtccctgccgcgcgctccgctggcaggggggactcgctcccaagtttgcactttctctgcagaggcccctccgctcggaaggggacagaactccccgggatgttctttcctcctaggagctacgcctgaccactttccctctcttttgctctccttctgccccttcttcaggaaataacgcggagatctgtctcctgcccctagactacggaccctgccgggccctacttctccgttactactacgacaggtacacgcagagctgccgccagttcctgtacgggggctgcgagggcaacgccaacaatttctacacctgggaggcttgcgacgatgcttgctggaggatagaaagtaagtgccctgcgcgcacccaggactctcgcgctccttgcgccggcggctggtagcagcttcgccagtttcccacgtctcgctttctacaggaagttttagcctgggttttctcaagtgttaagcaaacctcatggttttcagtttcttaaaagtaatcacaaatttacaaccactaacacatttcctgtctcccaactgacattgatcataattcagtgcctgtgcggactcagggaaagatttgttccctcaccatggggtataataaatgcaagagaataacgtgttaggtacaacgtaagtgcttctctgtatttttcattaattccaaacctatgatttttatctctcctggagtacatcatttccttctgtcgattatccatcaatctgaaatatttttagtggattttattattgaagtgtgacttagctcattatataactctacttttgtcccgatacccaaacatgtgttggattagttgcgggacatggtggagattcataatactgttatattttaatttatttttaatttttaaattatatcggttaaggcctgtaagagaacatggggcttttccattcaaggaactgagccaggggaaaatgcgtattcatgtgaataagctttgattcactgcatatgtacaatcagagaacacccagagaaaacagagagtctttctactgaacttgaaagatacatcacagctgagtcagctctgaatacactgttagaaaaaaaaaaagtaaatatctggattcatgggagtattctgggtatttactatcccaacactaatacaacttctctccccccacaaaatgttgctgaaaatacagtgatggtttaataagaaggctacttttgactaacattgttctattaccctccttttcctagaagttcccaaagtttgccggctgcaagtgagtgtggacgaccagtgtgaggggtccacagaaaagtatttctttaatctaagttccatgacatgtgaaaaattcttttccggtgggtgtcaccggaaccggattgagaacaggtttccagatgaagctacttgtatgggcttctgcgcaccaaagaaaagtaaatacgatttttatggtatttctatttcacttttttgaaaagacatttgggtggaaaaaactcaatttgatgcgaaattaacatgtgcattttcatgatttcacattacttgacaagttagtgacttgtcaagttcttaggactggaaagtgacaaagccatgattcaaatttttgctttctgcctcttctgatttgttgtttttgagacggactctcgccctgttgcccaggctggagtgcagtggcacaatctcggctctctgcaacctctgcctcccgggttcaagcgattctcctgcctcagcctcctgagtagctgggactacaggcgcccgccaccatgcccagctaatttttttttttttcttctttctctttctctttctttctctccttccttcctttctctcctttctttttctctttctttctttctttctctttccttccttccttccttccttccttccttccttccttccttctttccttccttccttccttctttctttcttttctttctttctttcttttttctttcgacggggtgtcaccgtgtaagccaggatggtcttgatctcctgacctcatgatctgcccacctcggcctcccaaaatgctgggattacaggtgtaagccaccacgcccagccctgaattgtttctttagaactatttctcagctactcaatttatgcataaaagattaaagtattcattaatgaatgttatgacctcagatttgtacacaataagttatacatgtgagatagtggaatatatacagaattaagatggtgaaacttgaaaatttctttctaaagttttcggttagatttctgtattcttcagtaattgcaaattgcagcacaaacatctccacacgtttctgtcctatccatttgttacctctcccaccaccacccctgaatccttgaaatgatagtctcttgagtagtatttaatgtttgcagagggagacaatacaggcatttcccccagacacagagatttttgaaaagttcaacaaacaaggaaaacttgctttggcagagaatttgataaagctttatagctgtactgtgttgaatatgcaaaatcttgagttaatgtggtgatggttactgtggatgttctcttgtttgtgtacatataaatgtttgctccagtggttacctggaaattagtatgcatatattattgattaataatggaatgagagctgttaaaaacattaaagcaaaactaccaacacgacaaaatttaccaaatcatgccacatattgtccttgaaacttaccccatttttacctaaccatatctggtatttgggtttaacttctttttacatttaaaggatacaaagatgtagcttcagaagaaattctatccagtttacaaaaatttagaattaccaaaatatagcatgtaagcttacctgcaatttgaagcacatctttttaaaggtttagtatgatattttggattcagactgaggcttctatgggattagattttcttcagttacttcagtaatcaccataatttaaaaattctggtattataacatttctaattttcttctcttttttataaagttccatcattttgctacagtccaaaagatgagggactgtgctctgccaatgtgactcgctattattttaatccaagatacagaacctgtgatgctttcacctatactggctgtggagggaatgacaataactttgttagcagggaggattgcaaacgtgcatgtgcaaaaggtagtgaatgttttcttattccacctttagataaactttataaataacttatcagaaaaattatatttttatttatccattttactaatagcaaattgctgtttctagactacttctacataagtatctccgtagtgttaatcagttttgtcaaaatgcttttactggctagctgcagtagacggtagctgtatcttcatatcttaaaggtaaaatattattaactgagtgtataatgagttttgacttcacagtccttaaaaataagatgaagtgagctcaataaccttatcagaaatagtgatttatagtgagcctacagactggagatgtatgattttcattgtcgttttattgattttagctttgaaaaagaaaaagaagatgccaaagcttcgctttgccagtagaatccggaaaattcggaagaagcaattttaaacattcttaatatgtcatcttgtttgtctttatggcttatttgcctttatggttgtatctgaagaataatatgacagcatgaggaaacaaatcattggtgatttattcaccagtttttattaatacaagtcactttttaaaaaatttggatttttttatatataactagctgctattcaaatgtgagtctaccatttttaatttatggttcaactgtttgtgagactgaattcttgcaatgcataagatataaaagcaaatatgactcactcatttcttggggtcgtattcctgatttcagaagaggatcataactgaaacaacataagacaatataatcatgtgcttttaacatatttgagaataaaaaggactagcaaataaaactcattttgcatttaaaagttggattatattttagtcccaagaagacaaagtcgcagattaacaacactttaaaaatattactcccattttattgtgttagattgcagtacaatgaatgaataaggggatttatttaaaagatcttaactttcttgactgatttaaaaagctaatcaatttattaaagccagaaatgttctcctctgggaaagcaatttctatctatttatctaccaatccccactcacatgtatatgtttgtgtttacatagagatagatggttttaagggttttcctattgttaaattatttcctaagacattgtgggttggagaccactaaacttataaaaaaccaaggaaagtaaagtttttcaaatgtttatactgtttaaggtgtttatttatataaaccatgcatgagaaaccatgcataaatttaataatttaaatttcaccagtaaattatcattgattaaatatggtcataccaatgaaataggttttttctttctctgtaataaaacaatttttctaaattcttatgttttcatagcaagattaacatatttaattacaaattaaatatgcaaaatgacaaatgcgtttaccttttgcttgaacaatctttcatttaaaaatttatcccagttattttgacaaataggtatatgcctgagaactttgaatgatgctgaaagctagaagcaaaccaggtactcttcagtcagggactggttgaagattttatggatgaggagttagcaaaatatctatatatgcatatcttctgactcccaggatacataagaaacacagggcctagaacagtatgaataaacacacatatacacaaacatcacagaagatactaaagatattaaaaatgtttacctatagaggtttggagagaacagaggggtggacagttgtggagataatatttgtgtaaatataactgtgatatagtttttatcttggaccatgtaaatatttgacataattaataatcaaaattaaataaaaaagaaaaagca

SEQ ID NO: 36 - RNA, 1642 nt, Homo sapiens
  source 1..1642: mol_type = mRNA
acaaactttcagagacagcagagcacacaagcttctaggacaagagccaggaagaaaccaccggaaggaaccatctcactgtgtgtaaacatgacttccaagctggccgtggctctcttggcagccttcctgatttctgcagctctgtgtgaaggtgcagttttgccaaggagtgctaaagaacttagatgtcagtgcataaagacatactccaaacctttccaccccaaatttatcaaagaactgagagtgattgagagtggaccacactgcgccaacacagaaattattgtaaagctttctgatggaagagagctctgtctggaccccaaggaaaactgggtgcagagggttgtggagaagtttttgaagagggctgagaattcataaaaaaattcattctctgtggtatccaagaatcagtgaagatgccagtgaaacttcaagcaaatctacttcaacacttcatgtattgtgtgggtctgttgtagggttgccagatgcaatacaagattcctggttaaatttgaatttcagtaaacaatgaatagtttttcattgtaccatgaaatatccagaacatacttatatgtaaagtattatttatttgaatctacaaaaaacaacaaataatttttaaatataaggattttcctagatattgcacgggagaatatacaaatagcaaaattgaggccaagggccaagagaatatccgaactttaatttcaggaattgaatgggtttgctagaatgtgatatttgaagcatcacataaaaatgatgggacaataaattttgccataaagtcaaatttagctggaaatcctggatttttttctgttaaatctggcaaccctagtctgctagccaggatccacaagtccttgttccactgtgccttggtttctcctttatttctaagtggaaaaagtattagccaccatcttacctcacagtgatgttgtgaggacatgtggaagcactttaagttttttcatcataacataaattattttcaagtgtaacttattaacctatttattatttatgtatttatttaagcatcaaatatttgtgcaagaatttggaaaaatagaagatgaatcattgattgaatagttataaagatgttatagtaaatttattttattttagatattaaatgatgttttattagataaatttcaatcagggtttttagattaaacaaacaaacaattgggtacccagttaaattttcatttcagataaacaacaaataattttttagtataagtacattattgtttatctgaaattttaattgaactaacaatcctagtttgatactcccagtcttgtcattgccagctgtgttggtagtgctgtgttgaattacggaataatgagttagaactattaaaacagccaaaactccacagtcaatattagtaatttcttgctggttgaaacttgtttattatgtacaaatagattcttataatattatttaaatgactgcatttttaaatacaaggctttatatttttaactttaagatgtttttatgtgctctccaaattttttttactgtttctgattgtatggaaatataaaagtaaatatgaaacatttaaaatataatttgttgtcaaagtaa

SEQ ID NO: 37 - protein, 99 aa, Homo sapiens
MTSKLAVALLAAFLISAALCEGAVLPRSAKELRCQCIKTYSKPFHPKFIKELRVIESGPHCANTEIIVKLSDGRELCLDPKENWVQRVVEKFLKRAENS

SEQ ID NO: 38 - protein, 95 aa, Homo sapiens
MTSKLAVALLAAFLISAALCEGAVLPRSAKELRCQCIKTYSKPFHPKFIKELRVIESGPHCANTEIIVKLSDGRELCLDPKENWVQRVVEKFLKR

SEQ ID NO: 39 - RNA, 3875 nt, Homo sapiens
  source 1..3875: mol_type = mRNA
agctgttcttggctgacttcacatcaaaactcctatactgacctgagacagaggcagcagtgatacccacctgagagatcctgtgtttgaacaactgcttcccaaaacggaaagtatttcaagcctaaacctttgggtgaaaagaactcttgaagtcatgattgcttcacagtttctctcagctctcactttggtgcttctcattaaagagagtggagcctggtcttacaacacctccacggaagctatgacttatgatgaggccagtgcttattgtcagcaaaggtacacacacctggttgcaattcaaaacaaagaagagattgagtacctaaactccatattgagctattcaccaagttattactggattggaatcagaaaagtcaacaatgtgtgggtctgggtaggaacccagaaacctctgacagaagaagccaagaactgggctccaggtgaacccaacaataggcaaaaagatgaggactgcgtggagatctacatcaagagagaaaaagatgtgggcatgtggaatgatgagaggtgcagcaagaagaagcttgccctatgctacacagctgcctgtaccaatacatcctgcagtggccacggtgaatgtgtagagaccatcaataattacacttgcaagtgtgaccctggcttcagtggactcaagtgtgagcaaattgtgaactgtacagccctggaatcccctgagcatggaagcctggtttgcagtcacccactgggaaacttcagctacaattcttcctgctctatcagctgtgataggggttacctgccaagcagcatggagaccatgcagtgtatgtcctctggagaatggagtgctcctattccagcctgcaatgtggttgagtgtgatgctgtgacaaatccagccaatgggttcgtggaatgtttccaaaaccctggaagcttcccatggaacacaacctgtacatttgactgtgaagaaggatttgaactaatgggagcccagagccttcagtgtacctcatctgggaattgggacaacgagaagccaacgtgtaaagctgtgacatgcagggccgtccgccagcctcagaatggctctgtgaggtgcagccattcccctgctggagagttcaccttcaaatcatcctgcaacttcacctgtgaggaaggcttcatgttgcagggaccagcccaggttgaatgcaccactcaagggcagtggacacagcaaatcccagtttgtgaagctttccagtgcacagccttgtccaaccccgagcgaggctacatgaattgtcttcctagtgcttctggcagtttccgttatgggtccagctgtgagttctcctgtgagcagggttttgtgttgaagggatccaaaaggctccaatgtggccccacaggggagtgggacaacgagaagcccacatgtgaagctgtgagatgcgatgctgtccaccagcccccgaagggtttggtgaggtgtgctcattcccctattggagaattcacctacaagtcctcttgtgccttcagctgtgaggagggatttgaattacatggatcaactcaacttgagtgcacatctcagggacaatggacagaagaggttccttcctgccaagtggtaaaatgttcaagcctggcagttccgggaaagatcaacatgagctgcagtggggagcccgtgtttggcactgtgtgcaagttcgcctgtcctgaaggatggacgctcaatggctctgcagctcggacatgtggagccacaggacactggtctggcctgctacctacctgtgaagctcccactgagtccaacattcccttggtagctggactttctgctgctggactctccctcctgacattagcaccatttctcctctggcttcggaaatgcttacggaaagcaaagaaatttgttcctgccagcagctgccaaagccttgaatcagatggaagctaccaaaagccttcttacatcctttaagttcaaaagaatcagaaacaggtgcatctggggaactagagggatacactgaagttaacagagacagataactctcctcgggtctctggcccttcttgcctactatgccagatgcctttatggctgaaaccgcaacacccatcaccacttcaatagatcaaagtccagcaggcaaggacggccttcaactgaaaagactcagtgttccctttcctactctcaggatcaagaaagtgttggctaatgaagggaaaggatattttcttccaagcaaaggtgaagagaccaagactctgaaatctcagaattccttttctaactctcccttgctcgctgtaaaatcttggcacagaaacacaatattttgtggctttctttcttttgcccttcacagtgtttcgacagctgattacacagttgctgtcataagaatgaataataattatccagagtttagaggaaaaaaatgactaaaaatattataacttaaaaaaatgacagatgttgaatgcccacaggcaaatgcatggagggttgttaatggtgcaaatcctactgaatgctctgtgcgagggttactatgcacaatttaatcactttcatccctatgggattcagtgcttcttaaagagttcttaaggattgtgatatttttacttgcattgaatatattataatcttccatacttcttcattcaatacaagtgtggtagggacttaaaaaacttgtaaatgctgtcaactatgatatggtaaaagttacttattctagattaccccctcattgtttattaacaaattatgttacatctgttttaaatttatttcaaaaagggaaactattgtcccctagcaaggcatgatgttaaccagaataaagttctgagtgtttttactacagttgttttttgaaaacatggtagaattggagagtaaaaactgaatggaaggtttgtatattgtcagatattttttcagaaatatgtggtttccacgatgaaaaacttccatgaggccaaacgttttgaactaataaaagcataaatgcaaacacacaaaggtataattttatgaatgtctttgttggaaaagaatacagaaagatggatgtgctttgcattcctacaaagatgtttgtcagatatgatatgtaaacataattcttgtatattatggaagattttaaattcacaatagaaactcaccatgtaaaagagtcatctggtagatttttaacgaatgaagatgtctaatagttattccctatttgttttcttctgtatgttagggtgctctggaagagaggaatgcctgtgtgagcaagcatttatgtttatttataagcagatttaacaattccaaaggaatctccagttttcagttgatcactggcaatgaaaaattctcagtcagtaattgccaaagctgctctagccttgaggagtgtgagaatcaaaactctcctacacttccattaacttagcatgtgttgaaaaaaaagtttcagagaagttctggctgaacactggcaacaacaaagccaacagtcaaaacagagatgtgataaggatcagaacagcagaggttcttttaaaggggcagaaaaactctgggaaataagagagaacaactactgtgatcaggctatgtatggaatacagtgttattttctttgaaattgtttaagtgttgtaaatatttatgtaaactgcattagaaattagctgtgtgaaataccagtgtggtttgtgtttgagttttattgagaattttaaattataacttaaaatattttataatttttaaagtatatatttatttaagcttatgtcagacctatttgacataacactataaaggttgacaataaatgtgcttatgttta

SEQ ID NO: 40 - protein, 610 aa, Homo sapiens
MIASQFLSALTLVLLIKESGAWSYNTSTEAMTYDEASAYCQQRYTHLVAIQNKEEIEYLNSILSYSPSYYWIGIRKVNNVWVWVGTQKPLTEEAKNWAPGEPNNRQKDEDCVEIYIKREKDVGMWNDERCSKKKLALCYTAACTNTSCSGHGECVETINNYTCKCDPGFSGLKCEQIVNCTALESPEHGSLVCSHPLGNFSYNSSCSISCDRGYLPSSMETMQCMSSGEWSAPIPACNVVECDAVTNPANGFVECFQNPGSFPWNTTCTFDCEEGFELMGAQSLQCTSSGNWDNEKPTCKAVTCRAVRQPQNGSVRCSHSPAGEFTFKSSCNFTCEEGFMLQGPAQVECTTQGQWTQQIPVCEAFQCTALSNPERGYMNCLPSASGSFRYGSSCEFSCEQGFVLKGSKRLQCGPTGEWDNEKPTCEAVRCDAVHQPPKGLVRCAHSPIGEFTYKSSCAFSCEEGFELHGSTQLECTSQGQWTEEVPSCQVVKCSSLAVPGKINMSCSGEPVFGTVCKFACPEGWTLNGSAARTCGATGHWSGLLPTCEAPTESNIPLVAGLSAAGLSLLTLAPFLLWLRKCLRKAKKFVPASSCQSLESDGSYQKPSYIL

SEQ ID NO: 41 - RNA, 4510 nt, Homo sapiens
  source 1..4510: mol_type = mRNA
aattgtcatacgacttgcagtgagcgtcaggagcacgtccaggaactcctcagcagcgcctccttcagctccacagccagacgccctcagacagcaaagcctacccccgcgccgcgccctgcccgccgctgcgatgctcgcccgcgccctgctgctgtgcgcggtcctggcgctcagccatacagcaaatccttgctgttcccacccatgtcaaaaccgaggtgtatgtatgagtgtgggatttgaccagtataagtgcgattgtacccggacaggattctatggagaaaactgctcaacaccggaatttttgacaagaataaaattatttctgaaacccactccaaacacagtgcactacatacttacccacttcaagggattttggaacgttgtgaataacattcccttccttcgaaatgcaattatgagttatgtgttgacatccagatcacatttgattgacagtccaccaacttacaatgctgactatggctacaaaagctgggaagccttctctaacctctcctattatactagagcccttcctcctgtgcctgatgattgcccgactcccttgggtgtcaaaggtaaaaagcagcttcctgattcaaatgagattgtggaaaaattgcttctaagaagaaagttcatccctgatccccagggctcaaacatgatgtttgcattctttgcccagcacttcacgcatcagtttttcaagacagatcataagcgagggccagctttcaccaacgggctgggccatggggtggacttaaatcatatttacggtgaaactctggctagacagcgtaaactgcgccttttcaaggatggaaaaatgaaatatcagataattgatggagagatgtatcctcccacagtcaaagatactcaggcagagatgatctaccctcctcaagtccctgagcatctacggtttgctgtggggcaggaggtctttggtctggtgcctggtctgatgatgtatgccacaatctggctgcgggaacacaacagagtatgcgatgtgcttaaacaggagcatcctgaatggggtgatgagcagttgttccagacaagcaggctaatactgataggagagactattaagattgtgattgaagattatgtgcaacacttgagtggctatcacttcaaactgaaatttgacccagaactacttttcaacaaacaattccagtaccaaaatcgtattgctgctgaatttaacaccctctatcactggcatccccttctgcctgacacctttcaaattcatgaccagaaatacaactatcaacagtttatctacaacaactctatattgctggaacatggaattacccagtttgttgaatcattcaccaggcaaattgctggcagggttgctggtggtaggaatgttccacccgcagtacagaaagtatcacaggcttccattgaccagagcaggcagatgaaataccagtcttttaatgagtaccgcaaacgctttatgctgaagccctatgaatcatttgaagaacttacaggagaaaaggaaatgtctgcagagttggaagcactctatggtgacatcgatgctgtggagctgtatcctgcccttctggtagaaaagcctcggccagatgccatctttggtgaaaccatggtagaagttggagcaccattctccttgaaaggacttatgggtaatgttatatgttctcctgcctactggaagccaagcacttttggtggagaagtgggttttcaaatcatcaacactgcctcaattcagtctctcatctgcaataacgtgaagggctgtccctttacttcattcagtgttccagatccagagctcattaaaacagtcaccatcaatgcaagttcttcccgctccggactagatgatatcaatcccacagtactactaaaagaacgttcgactgaactgtagaagtctaatgatcatatttatttatttatatgaaccatgtctattaatttaattatttaataatatttatattaaactccttatgttacttaacatcttctgtaacagaagtcagtactcctgttgcggagaaaggagtcatacttgtgaagacttttatgtcactactctaaagattttgctgttgctgttaagtttggaaaacagtttttattctgttttataaaccagagagaaatgagttttgacgtctttttacttgaatttcaacttatattataagaacgaaagtaaagatgtttgaatacttaaacactgtcacaagatggcaaaatgctgaaagtttttacactgtcgatgtttccaatgcatcttccatgatgcattagaagtaactaatgtttgaaattttaaagtacttttggttatttttctgtcatcaaacaaaaacaggtatcagtgcattattaaatgaatatttaaattagacattaccagtaatttcatgtctactttttaaaatcagcaatgaaacaataatttgaaatttctaaattcatagggtagaatcacctgtaaaagcttgtttgatttcttaaagttattaaacttgtacatataccaaaaagaagctgtcttggatttaaatctgtaaaatcagtagaaattttactacaattgcttgttaaaatattttataagtgatgttcctttttcaccaagagtataaacctttttagtgtgactgttaaaacttccttttaaatcaaaatgccaaatttattaaggtggtggagccactgcagtgttatcttaaaataagaatattttgttgagatattccagaatttgtttatatggctggtaacatgtaaaatctatatcagcaaaagggtctacctttaaaataagcaataacaaagaagaaaaccaaattattgttcaaatttaggtttaaacttttgaagcaaacttttttttatccttgtgcactgcaggcctggtactcagattttgctatgaggttaatgaagtaccaagctgtgcttgaataatgatatgttttctcagattttctgttgtacagtttaatttagcagtccatatcacattgcaaaagtagcaatgacctcataaaatacctcttcaaaatgcttaaattcatttcacacattaattttatctcagtcttgaagccaattcagtaggtgcattggaatcaagcctggctacctgcatgctgttccttttcttttcttcttttagccattttgctaagagacacagtcttctcatcacttcgtttctcctattttgttttactagttttaagatcagagttcactttctttggactctgcctatattttcttacctgaacttttgcaagttttcaggtaaacctcagctcaggactgctatttagctcctcttaagaagattaaaagagaaaaaaaaaggcccttttaaaaatagtatacacttattttaagtgaaaagcagagaattttatttatagctaattttagctatctgtaaccaagatggatgcaaagaggctagtgcctcagagagaactgtacggggtttgtgactggaaaaagttacgttcccattctaattaatgccctttcttatttaaaaacaaaaccaaatgatatctaagtagttctcagcaataataataatgacgataatacttcttttccacatctcattgtcactgacatttaatggtactgtatattacttaatttattgaagattattatttatgtcttattaggacactatggttataaactgtgtttaagcctacaatcattgatttttttttgttatgtcacaatcagtatattttctttggggttacctctctgaatattatgtaaacaatccaaagaaatgattgtattaagatttgtgaataaatttttagaaatctgattggcatattgagatatttaaggttgaatgtttgtccttaggataggcctatgtgctagcccacaaagaatattgtctcattagcctgaatgtgccataagactgaccttttaaaatgttttgagggatctgtggatgcttcgttaatttgttcagccacaatttattgagaaaatattctgtgtcaagcactgtgggttttaatatttttaaatcaaacgctgattacagataatagtatttatataaataattgaaaaaaattttcttttgggaagagggagaaaatgaaataaatatcattaaagataactcaggagaatcttctttacaattttacgtttagaatgtttaaggttaagaaagaaatagtcaatatgcttgtataaaacactgttcactgttttttttaaaaaaaaaacttgatttgttattaacattgatctgctgacaaaacctgggaatttgggttgtgtatgcgaatgtttcagtgcctcagacaaatgtgtatttaacttatgtaaaagataagtctggaaataaatgtctgtttatttttgtactatttaaaaattgacagatcttttctgaagataaactttgattgtttctata

SEQ ID NO: 42 - protein, 604 aa, Homo sapiens
MLARALLLCAVLALSHTANPCCSHPCQNRGVCMSVGFDQYKCDCTRTGFYGENCSTPEFLTRIKLFLKPTPNTVHYILTHFKGFWNVVNNIPFLRNAIMSYVLTSRSHLIDSPPTYNADYGYKSWEAFSNLSYYTRALPPVPDDCPTPLGVKGKKQLPDSNEIVEKLLLRRKFIPDPQGSNMMFAFFAQHFTHQFFKTDHKRGPAFTNGLGHGVDLNHIYGETLARQRKLRLFKDGKMKYQIIDGEMYPPTVKDTQAEMIYPPQVPEHLRFAVGQEVFGLVPGLMMYATIWLREHNRVCDVLKQEHPEWGDEQLFQTSRLILIGETIKIVIEDYVQHLSGYHFKLKFDPELLFNKQFQYQNRIAAEFNTLYHWHPLLPDTFQIHDQKYNYQQFIYNNSILLEHGITQFVESFTRQIAGRVAGGRNVPPAVQKVSQASIDQSRQMKYQSFNEYRKRFMLKPYESFEELTGEKEMSAELEALYGDIDAVELYPALLVEKPRPDAIFGETMVEVGAPFSLKGLMGNVICSPAYWKPSTFGGEVGFQIINTASIQSLICNNVKGCPFTSFSVPDPELIKTVTINASSSRSGLDDINPTVLLKERSTEL

SEQ ID NO: 43 - RNA, 2204 nt, Homo sapiens
  source 1..2204: mol_type = mRNA
ggagccccggctcctaggctgacagaccagcccagatccagtggcccggaggggcctgagctaaatccgcaggacctgggtaacacgaggaagtcggtttggtccctttagggctccggatatctttggtgacttgtccactccagtgtggcatcatgtggcagctgctcctcccaactgctctgctacttctagtttcagctggcatgcggactgaagatctcccaaaggctgtggtgttcctggagcctcaatggtacagggtgctcgagaaggacagtgtgactctgaagtgccagggagcctactcccctgaggacaattccacacagtggtttcacaatgagagcctcatctcaagccaggcctcgagctacttcattgacgctgccacagtcgacgacagtggagagtacaggtgccagacaaacctctccaccctcagtgacccggtgcagctagaagtccatatcggctggctgttgctccaggcccctcggtgggtgttcaaggaggaagaccctattcacctgaggtgtcacagctggaagaacactgctctgcataaggtcacatatttacagaatggcaaaggcaggaagtattttcatcataattctgacttctacattccaaaagccacactcaaagacagcggctcctacttctgcagggggctttttgggagtaaaaatgtgtcttcagagactgtgaacatcaccatcactcaaggtttggcagtgtcaaccatctcatcattctttccacctgggtaccaagtctctttctgcttggtgatggtactcctttttgcagtggacacaggactatatttctctgtgaagacaaacattcgaagctcaacaagagactggaaggaccataaatttaaatggagaaaggaccctcaagacaaatgacccccatcccatgggggtaataagagcagtagcagcagcatctctgaacatttctctggatttgcaaccccatcatcctcaggcctctctacaagcagcaggaaacatagaactcagagccagatcccttatccaactctcgacttttccttggtctccagtggaagggaaaagcccatgatcttcaagcagggaagccccagtgagtagctgcattcctagaaattgaagtttcagagctacacaaacactttttctgtcccaaccgttccctcacagcaaagcaacaatacaggctagggatggtaatcctttaaacatacaaaaattgctcgtgttataaattacccagtttagaggggaaaaaaaaacaattattcctaaataaatggataagtagaattaatggttgaggcaggaccatacagagtgtgggaactgctggggatctagggaattcagtgggaccaatgaaagcatggctgagaaatagcaggtagtccaggatagtctaagggaggtgttcccatctgagcccagagataagggtgtcttcctagaacattagccgtagtggaattaacaggaaatcatgagggtgacgtagaattgagtcttccaggggactctatcagaactggaccatctccaagtatataacgatgagtcctcttaatgctaggagtagaaaatggtcctaggaaggggactgaggattgcggtggggggtggggtggaaaagaaagtacagaacaaaccctgtgtcactgtcccaagttgctaagtgaacagaactatctcagcatcagaatgagaaagcctgagaagaaagaaccaaccacaagcacacaggaaggaaagcgcaggaggtgaaaatgctttcttggccagggtagtaagaattagaggttaatgcagggactgtaaaaccaccttttctgcttcaatatctaattcctgtgtagctttgttcattgcatttattaaacaaatgttgtataaccaatactaaatgtactactgagcttcgctgagttaagttatgaaactttcaaatccttcatcatgtcagttccaatgaggtggggatggagaagacaattgttgcttatgaaagaaagctttagctgtctctgttttgtaagctttaagcgcaacatttcttggttccaataaagcattttacaagatcttgcatgctactcttagatagaagatgggaaaaccatggtaataaaatatgaatgataaaaaaaaaaaaaaaaaaaaaaaaaaaaaaaaaaa

SEQ ID NO: 44 - protein, 254 aa, Homo sapiens
MWQLLLPTALLLLVSAGMRTEDLPKAVVFLEPQWYRVLEKDSVTLKCQGAYSPEDNSTQWFHNESLISSQASSYFIDAATVDDSGEYRCQTNLSTLSDPVQLEVHIGWLLLQAPRWVFKEEDPIHLRCHSWKNTALHKVTYLQNGKGRKYFHHNSDFYIPKATLKDSGSYFCRGLFGSKNVSSETVNITITQGLAVSTISSFFPPGYQVSFCLVMVLLFAVDTGLYFSVKTNIRSSTRDWKDHKFKWRKDPQDK

SEQ ID NO: 45 - protein, 358 aa, Homo sapiens
MAEGTLWQILCVSSDAQPQTFEGVKGADPPTLPPGSFLPGPVLWWGSLARLQTEKSDEVSRKGNWWVTEMGGGAGERLFTSSCLVGLVPLGLRISLVTCPLQCGIMWQLLLPTALLLLVSAGMRTDLPKAVVFLEPQWYRVLEKDSVTLKCQGAYSPEDNSTQWFHNESLISSQASSYFIDAATVDDSGEYRCQTNLSTLSDPVQLEVHIGWLLLQAPRWVFKEEDPIHLRCHSWKNTALHKVTYLQNGKGRKYFHHNSDFYIPKATLKDSGSYFCRGLFGSKNVSSETVNITITQGLAVSTISSFFPPGYQVSFCLVMVLLFAVDTGLYFSVKTNIRSSTRDWKDHKFKWRKDPQDK

SEQ ID NO: 46 - protein, 253 aa, Homo sapiens
MWQLLLPTALLLLVSAGMRTDLPKAVVFLEPQWYRVLEKDSVTLKCQGAYSPEDNSTQWFHNESLISSQASSYFIDAATVDDSGEYRCQTNLSTLSDPVQLEVHIGWLLLQAPRWVFKEEDPIHLRCHSWKNTALHKVTYLQNGKGRKYFHHNSDFYIPKATLKDSGSYFCRGLFGSKNVSSETVNITITQGLAVSTISSFFPPGYQVSFCLVMVLLFAVDTGLYFSVKTNIRSSTRDWKDHKFKWRKDPQDK

SEQ ID NO: 47 - protein, 273 aa, Homo sapiens
MAEGTLWQILCVSSDAQPQTFEGVKGADPPTLPPGSFLPGPVLWWGSLARLQTEKSDEVSRKGNWWVTEMGGGAGERLFTSSCLVGLVPLGLRISLVTCPLQCGIMWQLLLPTALLLLVSAGMRTEDLPKAVVFLEPQWYRVLEKDSVTLKCQGAYSPEDNSTQWFHNESLISSQASSYFIDAATVDDSGEYRCQTNLSTLSDPVQLEVHIGLAVSTISSFFPPGYQVSFCLVMVLLFAVDTGLYFSVKTNIRSSTRDWKDHKFKWRKDPQDK

SEQ ID NO: 48 - protein, 283 aa, Homo sapiens
MKFQEKEIVGLVPLGLRISLVTCPLQCGIMWQLLLPTALLLLVSAGMRTEDLPKAVVFLEPQWYRVLEKDSVTLKCQGAYSPEDNSTQWFHNESLISSQASSYFIDAATVDDSGEYRCQTNLSTLSDPVQLEVHIGWLLLQAPRWVFKEEDPIHLRCHSWKNTALHKVTYLQNGKGRKYFHHNSDFYIPKATLKDSGSYFCRGLFGSKNVSSETVNITITQGLAVSTISSFFPPGYQVSFCLVMVLLFAVDTGLYFSVKTNIRSSTRDWKDHKFKWRKDPQDK

SEQ ID NO: 49 - protein, 277 aa, Homo sapiens
MKFQEKEIGLRISLVTCPLQCGIMWQLLLPTALLLLVSAGMRTEDLPKAVVFLEPQWYRVLEKDSVTLKCQGAYSPEDNSTQWFHNESLISSQASSYFIDAATVDDSGEYRCQTNLSTLSDPVQLEVHIGWLLLQAPRWVFKEEDPIHLRCHSWKNTALHKVTYLQNGKGRKYFHHNSDFYIPKATLKDSGSYFCRGLFGSKNVSSETVNITITQGLAVSTISSFFPPGYQVSFCLVMVLLFAVDTGLYFSVKTNIRSSTRDWKDHKFKWRKDPQDK

SEQ ID NO: 50 - RNA, 2174 nt, Homo sapiens
  source 1..2174: mol_type = mRNA
agaaagccgcgcacctcctcccgccaggcgctttctcggacgccttgcccagcgggccgcccgaccccctgcaccatggaccccgctcgccccctggggctgtcgattctgctgcttttcctgacggaggctgcactgggcgatgctgctcaggagccaacagactacggaccctgccgggccctacttctccgttactactacgacaggtacacgcagagctgccgccagttcctgtacgggggctgcgagggcaacgccaacaatttctacacctgggaggcttgcgacgatgcttgctggaggatagaaaaagttcccaaagtttgccggctgcaagtgagtgtggacgaccagtgtgaggggtccacagaaaagtatttctttaatctaagttccatgacatgtgaaaaattcttttccggtgggtgtcaccggaaccggattgagaacaggtttccagatgaagctacttgtatgggcttctgcgcaccaaagaaaattccatcattttgctacagtccaaaagatgagggactgtgctctgccaatgtgactcgctattattttaatccaagatacagaacctgtgatgctttcacctatactggctgtggagggaatgacaataactttgttagcagggaggattgcaaacgtgcatgtgcaaaagctttgaaaaagaaaaagaagatgccaaagcttcgctttgccagtagaatccggaaaattcggaagaagcaattttaaacattcttaatatgtcatcttgtttgtctttatggcttatttgcctttatggttgtatctgaagaataatatgacagcatgaggaaacaaatcattggtgatttattcaccagtttttattaatacaagtcactttttaaaaaatttggatttttttatatataactagctgctattcaaatgtgagtctaccatttttaatttatggttcaactgtttgtgagactgaattcttgcaatgcataagatataaaagcaaatatgactcactcatttcttggggtcgtattcctgatttcagaagaggatcataactgaaacaacataagacaatataatcatgtgcttttaacatatttgagaataaaaaggactagcaaataaaactcattttgcatttaaaagttggattatattttagtcccaagaagacaaagtcgcagattaacaacactttaaaaatattactcccattttattgtgttagattgcagtacaatgaatgaataaggggatttatttaaaagatcttaactttcttgactgatttaaaaagctaatcaatttattaaagccagaaatgttctcctctgggaaagcaatttctatctatttatctaccaatccccactcacatgtatatgtttgtgtttacatagagatagatggttttaagggttttcctattgttaaattatttcctaagacattgtgggttggagaccactaaacttataaaaaaccaaggaaagtaaagtttttcaaatgtttatactgtttaaggtgtttatttatataaaccatgcatgagaaaccatgcataaatttaataatttaaatttcaccagtaaattatcattgattaaatatggtcataccaatgaaataggttttttctttctctgtaataaaacaatttttctaaattcttatgttttcatagcaagattaacatatttaattacaaattaaatatgcaaaatgacaaatgcgtttaccttttgcttgaacaatctttcatttaaaaatttatcccagttattttgacaaataggtatatgcctgagaactttgaatgatgctgaaagctagaagcaaaccaggtactcttcagtcagggactggttgaagattttatggatgaggagttagcaaaatatctatatatgcatatcttctgactcccaggatacataagaaacacagggcctagaacagtatgaataaacacacatatacacaaacatcacagaagatactaaagatattaaaaatgtttacctatagaggtttggagagaacagaggggtggacagttgtggagataatatttgtgtaaatataactgtgatatagtttttatcttggaccatgtaaatatttgacataattaataatcaaaattaaataaaaaagaaaaagca

SEQ ID NO: 51 - protein, 235 aa, Homo sapiens
MDPARPLGLSILLLFLTEAALGDAAQEPTGNNAEICLLPLDYGPCRALLLRYYYDRYTQSCRQFLYGGCEGNANNFYTWEACDDACWRIEKVPKVCRLQVSVDDQCEGSTEKYFFNLSSMTCEKFFSGGCHRNRIENRFPDEATCMGFCAPKKIPSFCYSPKDEGLCSANVTRYYFNPRYRTCDAFTYTGCGGNDNNFVSREDCKRACAKALKKKKKMPKLRFASRIRKIRKKQF

SEQ ID NO: 52 - protein, 224 aa, Homo sapiens
MDPARPLGLSILLLFLTEAALGDAAQEPTDYGPCRALLLRYYYDRYTQSCRQFLYGGCEGNANNFYTWEACDDACWRIEKVPKVCRLQVSVDDQCEGSTEKYFFNLSSMTCEKFFSGGCHRNRIENRFPDEATCMGFCAPKKIPSFCYSPKDEGLCSANVTRYYFNPRYRTCDAFTYTGCGGNDNNFVSREDCKRACAKALKKKKKMPKLRFASRIRKIRKKQF

SEQ ID NO: 53 - protein, 186 aa, Homo sapiens
MDPARPLGLSILLLFLTEAALGDAAQEPTGNNAEICLLPLDYGPCRALLLRYYYDRYTQSCRQFLYGGCEGNANNFYTWEACDDACWRIEKVPKVCRLQVSVDDQCEGSTEKYFFNLSSMTCEKFFSGGCHRNRIENRFPDEATCMGFCAPKKNTEPVMLSPILAVEGMTITLLAGRIANVHVQKL